European Patent Specification EP 3 458 056 B1, published October 15, 2025. Title: METHODS AND COMPOSITIONS FOR TREATING NON-ERK MAPK PATHWAY INHIBITOR-RESISTANT CANCERS. Applicant: SAHA, Saurabh. The sequence listing filed with the application follows.

SEQUENCE LISTING (82 sequences)

SEQ ID NO: 1 - DNA, 2949 bp, Homo sapiens
cgcctcccttccccctccccgcccgacagcggccgctcgggccccggctctcggttataagatggcggcgctgagcggtggcggtggtggcggcgcggagccgggccaggctctgttcaacggggacatggagcccgaggccggcgccggcgccggcgccgcggcctcttcggctgcggaccctgccattccggaggaggtgtggaatatcaaacaaatgattaagttgacacaggaacatatagaggccctattggacaaatttggtggggagcataatccaccatcaatatatctggaggcctatgaagaatacaccagcaagctagatgcactccaacaaagagaacaacagttattggaatctctggggaacggaactgatttttctgtttctagctctgcatcaatggataccgttacatcttcttcctcttctagcctttcagtgctaccttcatctctttcagtttttcaaaatcccacagatgtggcacggagcaaccccaagtcaccacaaaaacctatcgttagagtcttcctgcccaacaaacagaggacagtggtacctgcaaggtgtggagttacagtccgagacagtctaaagaaagcactgatgatgagaggtctaatcccagagtgctgtgctgtttacagaattcaggatggagagaagaaaccaattggttgggacactgatatttcctggcttactggagaagaattgcatgtggaagtgttggagaatgttccacttacaacacacaactttgtacgaaaaacgtttttcaccttagcattttgtgacttttgtcgaaagctgcttttccagggtttccgctgtcaaacatgtggttataaatttcaccagcgttgtagtacagaagttccactgatgtgtgttaattatgaccaacttgatttgctgtttgtctccaagttctttgaacaccacccaataccacaggaagaggcgtccttagcagagactgccctaacatctggatcatccccttccgcacccgcctcggactctattgggccccaaattctcaccagtccgtctccttcaaaatccattccaattccacagcccttccgaccagcagatgaagatcatcgaaatcaatttgggcaacgagaccgatcctcatcagctcccaatgtgcatataaacacaatagaacctgtcaatattgatgacttgattagagaccaaggatttcgtggtgatggaggatcaaccacaggtttgtctgctaccccccctgcctcattacctggctcactaactaacgtgaaagccttacagaaatctccaggacctcagcgagaaaggaagtcatcttcatcctcagaagacaggaatcgaatgaaaacacttggtagacgggactcgagtgatgattgggagattcctgatgggcagattacagtgggacaaagaattggatctggatcatttggaacagtctacaagggaaagtggcatggtgatgtggcagtgaaaatgttgaatgtgacagcacctacacctcagcagttacaagccttcaaaaatgaagtaggagtactcaggaaaacacgacatgtgaatatcctactcttcatgggctattccacaaagccacaactggctattgttacccagtggtgtgagggctccagcttgtatcaccatctccatatcattgagaccaaatttgagatgatcaaacttatagatattgcacgacagactgcacagggcatggattacttacacgccaagtcaatcatccacagagacctcaagagtaataatatatttcttcatgaagacctcacagtaaaaataggtgattttggtctagctacagtgaaatctcgatggagtgggtcccatcagtttgaacagttgtctggatccattttgtggatggcaccagaagtcatcagaatgcaagataaaaatccatacagctttcagtcagatgtatatgcatttggaattgttctgtatgaattgatgactggacagttaccttattcaaacatcaacaacagggaccagataatttttatggtgggacgaggatacctgtctccagatctcagtaaggtacggagtaactgtccaaaagccatgaagagattaatggcagagtgcctcaaaaagaaaagagatgagagaccactctttccccaaattctcgcctctattgagctgctggcccgctcattgccaaaaattcaccgcagtgcatcagaaccctccttgaatcgggctggtttccaaacagaggattttagtctatatgcttgtgcttctccaaaaacacccatccaggcagggggatatggtgcgtttcctgtccactgaaacaaatgagtgagagagttcaggagagtagcaacaaaaggaaaataaatgaacatatgtttgcttatatgttaaattgaataaaatactctctttttttttaaggtgaaccaaagaacacttgtgtggttaaagactagatataatttttccccaaactaaaatttatacttaacattggatttttaacatccaagggttaaaatacatagacattgctaaaaattggcagagcctcttctagaggctttactttctgttccgggtttgtatcattcacttggttattttaagtagtaaacttcagtttctcatgcaacttttgttgccagctatcacatgtccactagggactccagaagaagaccctacctatgcctgtgtttgcaggtgagaagttggcagtcggttagcctgggttagataaggcaaactgaacagatctaatttaggaagtcagtagaatttaataattctattattattcttaataatttttctataactatttctttttataacaatttggaaaatgtggatgtcttttatttccttgaagcaataaactaagtttctttttataaaaa

SEQ ID NO: 2 - protein, 765 aa, Homo sapiens
AALSGGGGGGAEPGQALFNGDMEPEAGAGAGAAASSAADPAIPEEVWNIKQMIKLTQEHIEALLDKFGGEHNPPSIYLEAYEEYTSKLDALQQREQQLLESLGNGTDFSVSSSASMDTVTSSSSSSLSVLPSSLSVFQNPTDVARSNPKSPQKPIVRVFLPNKQRTVVPARCGVTVRDSLKKALMMRGLIPECCAVYRIQDGEKKPIGWDTDISWLTGEELHVEVLENVPLTTHNFVRKTFFTLAFCDFCRKLLFQGFRCQTCGYKFHQRCSTEVPLMCVNYDQLDLLFVSKFFEHHPIPQEEASLAETALTSGSSPSAPASDSIGPQILTSPSPSKSIPIPQPFRPADEDHRNQFGQRDRSSSAPNVHINTIEPVNIDDLIRDQGFRGDGGSTTGLSATPPASLPGSLTNVKALQKSPGPQRERKSSSSSEDRNRMKTLGRRDSSDDWEIPDGQITVGQRIGSGSFGTVYKGKWHGDVAVKMLNVTAPTPQQLQAFKNEVGVLRKTRHVNILLFMGYSTKPQLAIVTQWCEGSSLYHHLHIIETKFEMIKLIDIARQTAQGMDYLHAKSIIHRDLKSNNIFLHEDLTVKIGDFGLATVKSRWSGSHQFEQLSGSILWMAPEVIRMQDKNPYSFQSDVYAFGIVLYELMTGQLPYSNINNRDQIIFMVGRGYLSPDLSKVRSNCPKAMKRLMAECLKKKRDERPLFPQILASIELLARSLPKIHRSASEPSLNRAGFQTEDFSLYACASPKTPIQAGGYGAFPVH

SEQ ID NO: 3 - DNA, 3906 bp, Rattus norvegicus
atggcggcgctgagtggcggcggtggcagcagcagcggtggcggtggcggcggcggcggcggcggtggtggcggcggcggcggcggcgccgaacagggacaggctctgttcaatggcgacatggagccggaggccggcgctggcgccgcggcctcttcggccgcggacccggccattcctgaagaggtgtggaatatcaagcaaatgattaagttgacacaggaacatatagaggccctattggacaagtttggtggggagcataacccaccgtcaatatacctggaggcctatgaagagtacaccagcaagctagatgcccttcagcagagagagcagcagctgttggaatccctggtttttcaaactcccacagatgtatcacggaacaaccccaagtcaccacagaaacctatcgttcgtgtcttcctgcccaacaaacagaggacagtggtgcccgcaagatgtggtgtaacggtccgagacagtctaaagaaagcactaatgatgaggggtctcatcccagagtgctgtgctgtttacagaattcaggacggagagaagaaaccaattggctgggacactgacatttcctggcttactggagaggagctacatgttgaagtactagagaatgttcctctgacaacccacaacttcgtacggaaaacttttttcaccttagcattttgtgacttttgccgaaagctgcttttccagggtttccgctgtcaaacatgtggttataagtttcaccagcgttgtagtacagaggttccactgatgtgtgttaattatgaccaacttgatttgctgtttgtctccaagttctttgagcatcacccagtaccacaggaggaggccttctcagcagagactacccttccatctggatgctcttccgcacccccctcagactctattgggccccaaatcctcaccagtccatctccttcaaaatccattccaattccacagcccttccggccagcagatgaagatcatcgcaatcagtttgggcaacgagaccgctcctcctccgctcccaatgttcatataaacacaatcgaacctgtcaatattgatgaaaaattcccagaagtggaattacaggatcaaagggatttgattagagaccaggggtttcgtggggatggagcccctttgaaccagctgatgcgctgtcttcggaaataccaatcccggactcccagccccctcctccattctgtccccagtgaaatagtgtttgattttgagcctggcccagtgttcagagggtcaaccacaggcttgtcggccaccccacctgcctcattacctggctcactcactaacgtgaaagccttacagaaatctccaggacctcagcgggaaaggaagtcctcctcctcctcctcctccacggaagacagaagtcggatgaaaacacttggtagaagagattcaagtgatgattgggagattcctgatggacagattacagtgggacagagaattggatctgggtcctttggaactgtctacaagggaaagtggcatggcgacgtggcagtgaaaatgctgaatgtgacagcacccacacctcagcagttacaggccttcaaaaacgaagtcggagtactcaggaaaactcgacatgtgaacatcctccttttcatgggctattctacaaagccacagctggctattgttacacagtggtgtgaaggctccagcttatatcaccatctccacatcattgagaccaaatttgagatgatcaaacttatagatattgcacggcagactgcacagggcatggattacttacacgccaagtcaatcatccacagagacctcaagagtaataatatatttcttcatgaagacctcacggtaaaaataggtgactttggtttagccacagtgaagtcccgatggagtgggtcccatcagtttgaacagttgtctggatctattttgtggatggcacccgaagtaatcagaatgcaagataaaaacccatatagctttcagtcagacgtgtatgcatttgggattgttctgtatgaactgatgactggtcagctaccttattcaaacatcaacaacagggatcagataatttttatggtgggacgaggatacctatctccagatctcagtaaggtacggagtaactgtccaaaagccatgaagagattaatggcagagtgcctcaaaaagaaaagagacgagagaccactctttccccaaattctcgcctctattgagctgctggcccgctcattgccaaaaattcaccgcagtgcatcagaaccctccttgaatcgggctggtttccaaacagaagattttagtctgtatgcttgtgcttctccaaaaacacccatccaagcagggggatatggagaatttgcagccttcaagtagccactccatcatggcagcatctactctttatttcttaagtcttgtgttcatacaatttgttaacatcaaaacacagttctgttcctcaaattttttttaaagatacaaaattttcaatgcataagctcgtgtggaacagaatggaatttcctattcaacaaaagagggaagaatgttttaggaaccagaattctctgctgcccgtgtttcttcttcaacacaaatatcatgtgcatacaactctgcccattcccaagaagaaagaggagagaccccgaattctgcccttttggtggtcaggcatgatggaaagaatttgctgctgcagcttgggaaaaattgctatggaaagtctgccagtcaactttgcccttctaaccaccagatccatttgtggctggtcatctgatggggcgatttcaatcaccaagcatcgttcttgcctgttgtgggattatgtcgtggagcactttccctatccaccaccgttaatttccgagggatggagtaaatgcagcataccctttgtgtagcacctgtccagtcctcaaccaatgctatcacagtgaagctctttaaatttaagtggtgggtgagtgttgaggagagactgccttgggggcagagaaaaggggatgctgcatcttcttcctcacctccagctctctcacctcgggttgccttgcacactgggctccgcctaaccactcgggctgggcagtgctggcacacattgccgccttttctcattgggtccagcaattgagcagagggttgggggattgtttcctccacaatgtagcaaattctcaggaaaatacagtccatatcttcctctcagctcttccagtcaccaaatacttacgtggctcctttgtccaggacataaaacaccgtggacaacacctaattaaaagcctacaaaactgcttactgacagttttgaatgtgagacatttgtgtaatttaaatgtaaggtacaggtcttaatttcttctattaagtttcttctatttttatttaaacgaagaaaataattttcaggtttaattggaataaacgaatacttcccaaaagactatataccctgaaaattatatttttgttaattgtaaacaacttttaaaaaatggttattatccttttctctacctaaaattatgggaaatcttagcataatgacaattatttatactttttaaataaatggtacttgctggatccacactaacatctttgctaacattcccattgtttcttccaacttcactcctacactacatcctccatcctctttctagtcttttatctataatatgcaacctaaaataaaagtggtggtgtctccattcattcttcttcttccttttttccccaagcctggtcttcaaaaggttgggtaatttagtagctgagttccctaggtagaaatagaactattagggacattggggttgtaggaaagcgtgaggcctgtcaccagttgttctt

SEQ ID NO: 4 - protein, 804 aa, Rattus norvegicus
MAALSGGGGSSSGGGGGGGGGGGGGGGGGAEQGQALFNGDMEPEAGAGAAASSAADPAIPEEVWNIKQMIKLTQEHIEALLDKFGGEHNPPSIYLEAYEEYTSKLDALQQREQQLLESLVFQTPTDVSRNNPKSPQKPIVRVFLPNKQRTVVPARCGVTVRDSLKKALMMRGLIPECCAVYRIQDGEKKPIGWDTDISWLTGEELHVEVLENVPLTTHNFVRKTFFTLAFCDFCRKLLFQGFRCQTCGYKFHQRCSTEVPLMCVNYDQLDLLFVSKFFEHHPVPQEEAFSAETTLPSGCSSAPPSDSIGPQILTSPSPSKSIPIPQPFRPADEDHRNQFGQRDRSSSAPNVHINTIEPVNIDEKFPEVELQDQRDLIRDQGFRGDGAPLNQLMRCLRKYQSRTPSPLLHSVPSEIVFDFEPGPVFRGSTTGLSATPPASLPGSLTNVKALQKSPGPQRERKSSSSSSSTEDRSRMKTLGRRDSSDDWEIPDGQITVGQRIGSGSFGTVYKGKWHGDVAVKMLNVTAPTPQQLQAFKNEVGVLRKTRHVNILLFMGYSTKPQLAIVTQWCEGSSLYHHLHIIETKFEMIKLIDIARQTAQGMDYLHAKSIIHRDLKSNNIFLHEDLTVKIGDFGLATVKSRWSGSHQFEQLSGSILWMAPEVIRMQDKNPYSFQSDVYAFGIVLYELMTGQLPYSNINNRDQIIFMVGRGYLSPDLSKVRSNCPKAMKRLMAECLKKKRDERPLFPQILASIELLARSLPKIHRSASEPSLNRAGFQTEDFSLYACASPKTPIQAGGYGEFAAFK

SEQ ID NO: 5 - DNA, 9728 bp, Mus musculus
ccctcaggctcggctgcgccggggccgccggcgggttccagaggtggcctccgccccggccgctccgcccacgccccccgcgcctccgcgcccgcctccgcccgccctgcgcctcccttccccctccccgccccgcggcggccgctcggcccggctcgcgcttcgaagatggcggcgctgagtggcggcggtggcagcagcagcggtggcggcggcggcggtggcggcggcggtggcggtggcgacggcggcggcggcgccgagcagggccaggctctgttcaatggcgacatggagccggaggccggcgctggcgccgcggcctcttcggctgcggacccggccattcctgaagaggtatggaatatcaagcaaatgattaagttgacacaggaacatatagaggccctattggacaaatttggtggagagcataacccaccatcaatatacctggaggcctatgaagagtacaccagcaagctagatgcccttcagcaaagagaacagcagcttttggaatccctggtttttcaaactcccacagatgcatcacggaacaaccccaagtcaccacagaaacctatcgttagagtcttcctgcccaacaaacagaggacagtggtacccgcaagatgtggtgttacagttcgagacagtctaaagaaagcactgatgatgagaggtctcatcccagaatgctgtgctgtttacagaattcaggatggagagaagaaaccaattggctgggacacggacatttcctggcttactggagaggagttacatgttgaagtactggagaatgtcccacttacaacacacaactttgtacggaaaacttttttcaccttagcattttgtgacttttgccgaaagctgcttttccagggtttccgttgtcaaacatgtggttataaatttcaccagcgttgtagtacagaggttccactgatgtgtgtaaattatgaccaacttgatttgctgtttgtctccaagttctttgagcatcacccagtaccacaggaggaggcctccttcccagagactgcccttccatctggatcctcttccgcacccccctcagactctactgggccccaaatcctcaccagtccatctccttcaaaatccattccaattccacagcccttccgaccagcagatgaagatcatcgcaatcagtttgggcaacgagaccggtcctcctcagctcccaatgttcatataaacacaattgagcctgtgaatatcgatgaaaaattcccagaagtggaattacaggatcaaagggatttgattagagaccaggggtttcgtggtgatggagcccccttgaaccaactgatgcgctgtcttcggaaataccaatcccggactcccagccccctcctccattctgtccccagtgaaatagtgtttgattttgagcctggcccagtgttcagagggtcaaccacaggcttgtccgccaccccgcctgcctcattacctggctcactcactaacgtgaaagccttacagaaatctccaggtcctcagcgggaaaggaagtcatcttcttcctcatcctcggaggacagaagtcggatgaaaacacttggtagaagagattcaagtgatgactgggagattcctgatggacagattacagtgggacagagaattggatctgggtcatttggaactgtctacaagggaaagtggcatggtgatgtggcagtgaaaatgttgaatgtgacagcacccacacctcaacagctacaggccttcaaaaatgaagtaggagtgctcaggaaaactcgacatgtgaatatcctccttttcatgggctattctacaaagccacaactggcaattgttacacagtggtgtgagggctccagcttatatcaccatctccacatcattgagaccaaatttgagatgatcaaacttatagatattgctcggcagactgcacagggcatggattacttacacgccaagtcaatcatccacagagacctcaagagtaataatatatttcttcatgaagacctcacggtaaaaataggtgactttggtctagccacagtgaaatctcggtggagtgggtcccatcagtttgaacagttgtctggatctattttgtggatggcaccagaagtaatcagaatgcaagataaaaacccgtatagctttcagtcagacgtgtatgcgtttgggattgttctgtacgaactgatgaccggccagctaccttattcaaacatcaacaacagggatcagataatttttatggtgggacgaggatacctatctccagatctcagtaaggtacggagtaactgtccaaaagccatgaagagattaatggcagagtgcctcaaaaagaaaagagacgagagaccactctttccccaaattctcgcctccattgagctgctggcccgctcattgccaaaaattcaccgcagtgcatcagaaccttccttgaatcgggctggtttccaaacagaagattttagtctgtatgcttgtgcttctccgaaaacacccatccaagcagggggatatggagaatttgcagccttcaagtagccagtccatcatggcagcatctactctttatttcttaagtcttgtgttcatacagtttgttaacatcaaaacacagttctgttcctcaaaaaattttttaaagatacaaaattttcaatgcataagttcatgtggaacagaatggaatttcctattcaacaaaagagggaagaatgttttaggaaccagaattctctgctgcccgtgtttcttcttcaacataactatcacgtgcatacaagtctgcccattcccaagaagaaagaggagagaccctgaattctgcccttttggtggtcaggcatgatggaaagaatttgctgctgcagcttgggaaaattgctatggaaagtctgccagtcgactttgcccttctaaccaccagatcagcctgtggctggtcatctgatggggcgatttccatcaccaagcatcgttcttgcctattctgggattatgttgtggagcactttccctgtccagcaccgttcatttctgagggatggagtaaatgcagcattcccttgtgtagcgcctgttcagtcctcagcagctgctgtcacagcgaagctttttacagttaagtggtgggggagagttgaggagagcctgcctcggggcagagaaaagggggtgctgcatcttcttcctcacctccagctctctcacctcgggttgccttgctcactgggctccgcctaaccactcaggctgctcagtgctggcacacattgccttcttttctcattgggtccagcaattgaggagagggttgggggattgtttcctcctcaatgtagcaaattctcaggaaaatacagtccatatcttcctctcagctcttccagtcaccaaatacttacgtggctcctttgtccaggacataaaacaccgtggacaacacctaattaaaagcctacaaaactgcttactgacagttttgaatgtgagacacttgtgtaatttaaatgtaaggtacaggttttaatttctgagtttcttctatttttatttaaaagaagaaaataattttcagttttaattggaataaatgagtacttcccacaagactatataccctgaaaattatatttttgttaattgtaaacaacttttaaagaataattattatccttttctctacctaaaaattatggggaatcttagcataatgacaattatttatactttttaaataaatggtacttgctggatccacactaacatctttgctaacaatcccattgtttcttccaacttaactcctacactacatcctacatcctctttctagtcttttatctataatatgcaacctaaaataaacgtggtggcgtctccattcattctccctcttcctgttttccccaagcctggtcttcaaaaggttgggtaatcggtccctgagctccctagctggcaatgcaactattagggacattggagttgcaggagagcaggaagcctgtccccagctgttcttctagaaccctaaatcttatctttgcacagatcaaaagtatcacctcgtcacagttctccttagcctttacttacaggtaatataaataaaaatcaccatagtagtaaagaaaacaactggatggattgatgaccagtacctctcagagccaggaatcttgaatctccaggatttatacgtgcaaatttaaggagatgtacttagcaacttcaagccaagaacttccaaaatactagcgaatctaaaataaaatggaattttgagttatttttaaagttcaaattataattgataccactatgtatttaagcctactcacagcaagttagatggattttgctaaactcattgccagactgtggtggtggtggtggtagtgtgcacctttaatccaagcaactcagcaatcagaatgaggtaaatctctgtgaatacaaggcctgcctagtctgcagcgctagttccaggatagccagggctacacacacaaaaaccctctctcaaaaaaaacaaaattaattagttgataataaaaaataactaaagtatcatcaaaggaaggcctactggaagttttatatattcccagtaaattgaaaaatattctgaagttattaaccagttagcaacaatgtgtttttaagtcttacataaacagagcaaagtcttcaaatgtttcagagctgagaagataattgtgcttgatatgaaaaatagcctctccatatgatgtgccacattgaaaggcgtcattacccttttaaatacttcttaatgtggctttgttccctttacccaggattagctagaaagagctaggtaggcttcggccacagttgcacatttcgggcctgctgaagaatgggagctttgaaggctggccttggtggaggagcccctcagtgctggagggtggggcgtgtacgcagcatggaagtggtctagacagagtgcaaagggacagacttctttctcattttagtatagggtgatgtctcacttgaaatgagaaagtagagttgatattaaacgaagctgtgcccagaaaccaggctcagggtattgtgagattttctttttaaatagagaatataaaagatagaaataaatatttaaaccttccttcttattttctatcaaatagattttttttatcatttgcaaacaacataaaaaaaggtttcttttgtggggttttctttccttcttttttttttttttttttttttaagactgcagataatcttgttgagctcctcggaaaatacaaggaagtccgtgtttgtgcagagcgctttatgagtaactgtatagacagtgtggctgcttcactcatcccagagggctgcagctgtcggcccatgaagtggctgcagtgcctcgtgagatctgctttgttttgtttggagtgaagtctttgaaaggtttgagtgcaactatataggactgtttttaaataagtagtattcctcatgaactttctcattgttaagctacaggacccaaactctaccactaagatattattaacctcaaaatgtagtttatagaaggaatttgcaaatagaatatccagttcgtacttatatgcatcttcaacaaagattctctgtgacttgttggatttggttcctgaacagcccatttctgtatttgaggttaggagggcataatgaggcatcctaaaagacaatctgatataaactgtatgctagatgtatgctggtaggggagaaagcattctgtaaagacatgatttaagacttcagctctgtcaaccagaaaccttgtaaatacttcctgtcttggtgcagccccgcccctttgatcacacgatgttgtcttgtgcttgtcagacactgtcagagctgctgttcgtccctctgcagatctcacctgtccccactgcacacccacctcctgcctcttgcagacctcagcatctagctttagttggaaacagttcagggttcaggtgacttcttaaaaaaaaaaaaaaaccctacctcctcagaatgaggtaatgaatagttatttatttaaagtatgaagagtcaggagcgctcgaacatgaaggtgatttaagatggttcctttcgtgtgtattgtagctgagcacttgtttttgtcctaaagggcattatacatttaagcagtgattctgtttaaagatgtttttctttaaaggtgtagctcagagtatctgttgttggaattggtgccagagtctgcttaatagatttcagaatcctaagcttaagtcagtcgcatgaagttaagtagttatggtaacactttgctagccatgatataattctactttttaggagtaggtttggcaaaactgtatgccttcaaagtgagttggccacagctttgtcacatgcacagatactcatctgaagagactgcccagctaagagggcggaaggatacccttttttcctacgattcgcttctttgtccacgttggcattgttagtactagtttatcagcaccttgaccagcagatgtcaaccaataagctatttttaaaaccatagccagagatggagaggtcactgtgagtagaaacagcaggacgcttacaggagtgaaatggtgtagggaggctctagaaaaatatcttgacaatttgccaaatgatcttactgtgccttcatgatgcaataaaaaagctaacattttagcagaaatcagtgatttacgaagagagtggccagtctggtttaactcagctgggataatatttttagagtgcaatttagactgcgaagataaatgcactaaagagtttatagccaattcacatttgaaaaataagaaaatggtaaattttcagtgaaatatttttttaaagcacataatccctagtgtagccagaaatatttaccacatagagcagctaggctgagatacagtccagtgacatttctagagaaaccttttctactcccacgggctcctcaaagcatggaaattttatacaaaatgtttgacattttaagatactgctgtagtttagttttgaaatagtatgtgctgagcagcaatcatgtactaactcagagagagaaaacaacaacaaattgtgcatctgatttgttttcagagaaatgctgccaacttagatactgagttctcagagcttcaagtgtaaacttgcctcccaagtcctgtttgcaaatgaagttggctagtgctactgactgctccagcacatgatggaaggcagggggctgtctctgaagtgtcttctataaagggacaatagaatagtgagagacctggtcagtgtgtgtcagctggacactccatgctatgggacttgcatcttctgtcctcaccatccccaagacattgtgctttcctcagttgtcctctagctgtttcactcagacaccaagatgaattactgatgccagaaggggccaaaatggccagtgtgttttgggggttgtatcagttgactggacaataactttaatagtttcagatcatttatttttacttccattttgacagacatttaaatggaaatttagtcctaacttttgtcatttgaaaggaaaaattaacagttcctataagatacttttgaggtggaatctgacatcctaattttttttcttttcagtgggtttgcagcgagggtcttgtatgcactaggcaagggttctaccactaagccacatttcccaggaaataaaatgttaacagttaaaacatacacacaaatacacaaacaccttattaccactttagtaaagtgagagatgtgcgtcctttgtctcagtctccacgatttcagctgccccttgtatgaataactcagtctcgctaaactgtttacttttatttacctggtttgactagttgcagctatataaccagttgtgcatgaggacaacagccagtgtgtttgttttgtttttggttttttgtggtacattttttgtaaagaattctgtagattgaagtgctctttgaaaacagaactgagatatatttattcttgttagcatcaaaaaacattttgtgcaaatgatttgcttttcctggcaggctgagtaccatatccagcgcccacaattgcgggttcccatctaccatgtccacaggggagacagacgggaagcacatgaggggtgtgtttacagagttgtaggagttatgtagttctcttgttgccttggaaatcactgttgttttaagactgttgaacccgtgtgtttggctgggctgtgagttacatgaagaaactgcaaactagcatatgcagacaaagctcacagactaggcgtaaatggaggaaaatggaccaaaataaggcagggtgacacataaaccttgggcttcggagaaaactaagggtggagatgaactataatcacctgaatacaatgtaagagtgcaataagtgtgcttattctaagctgtgaacttcttttaaatcattcctttctaatacatttatgtatgttccattgctgactaaaaccagctatgagaacatatgcctttttattcatgttaactaccagtttaagtggctaaccttaatgtcttatttatcttcattttgtattagtttacataccaggtatgtgtgtgtgctgtactcttcttccctttatttgaaaacacttttcactgggtcatctccttggccattccacaacacaactttggtttggctttcaatgtcaccttatttgatggcctgtgtcccagtagcagaatttatggtattcccattgctggctgctcttccgaccctttgcttctacagcacttgtctctcctaagatagtcagaaactaactgatcaggggatggacttcaccattcatcgtgtctcttcaattctattaaatagaccactcttgggctttagaccaggaaaaaggagacagctctagccatctaccaagcctcaccctaaaaggtcacccgtacttcttggtctgaggacaagtctccactccagtaagggagaggggaggaaatgcttcctgtttgaaatgcagtgaattcctatggctcctgtttcaccacccgcacctatggcaacccatatacattcctcttgtctgtaactgccaaaggttgggtttatgtcacttcagttccactcaagcattgaaaaggttctcatggagtctggggtgtgcccagtgaaaagatggggactttttcattatccacagacctctctatacctgctttgcaaaaattataatggagtaactatttttaaagcttatttttcaattcataagaaaaagacatttattttcaatcaaatggatgatgtctcttatcccttatccctcaatgtttgcttgaattttgtttgttccctatacctactccctaattctttagttccttcctgctcaggtcccttcatttgtactttggagtttttctcatgtaaatttgtataatggaaaatattgttcagtttggatagaaagcatggagaaataaataaaaaaagatagctgaaaatcaaattgaagaaatttatttctgtgtaaagttatttaaaaactctgtattatatttaaagaaaaaagcccaaccccccaaaaagtgctatgtaattgatgtgaatatgcgaatactgctataataaagattgactgcatggagaaa

SEQ ID NO: 6 - protein, 804 aa, Mus musculus
MAALSGGGGSSSGGGGGGGGGGGGGDGGGGAEQGQALFNGDMEPEAGAGAAASSAADPAIPEEVWNIKQMIKLTQEHIEALLDKFGGEHNPPSIYLEAYEEYTSKLDALQQREQQLLESLVFQTPTDASRNNPKSPQKPIVRVFLPNKQRTVVPARCGVTVRDSLKKALMMRGLIPECCAVYRIQDGEKKPIGWDTDISWLTGEELHVEVLENVPLTTHNFVRKTFFTLAFCDFCRKLLFQGFRCQTCGYKFHQRCSTEVPLMCVNYDQLDLLFVSKFFEHHPVPQEEASFPETALPSGSSSAPPSDSTGPQILTSPSPSKSIPIPQPFRPADEDHRNQFGQRDRSSSAPNVHINTIEPVNIDEKFPEVELQDQRDLIRDQGFRGDGAPLNQLMRCLRKYQSRTPSPLLHSVPSEIVFDFEPGPVFRGSTTGLSATPPASLPGSLTNVKALQKSPGPQRERKSSSSSSSEDRSRMKTLGRRDSSDDWEIPDGQITVGQRIGSGSFGTVYKGKWHGDVAVKMLNVTAPTPQQLQAFKNEVGVLRKTRHVNILLFMGYSTKPQLAIVTQWCEGSSLYHHLHIIETKFEMIKLIDIARQTAQGMDYLHAKSIIHRDLKSNNIFLHEDLTVKIGDFGLATVKSRWSGSHQFEQLSGSILWMAPEVIRMQDKNPYSFQSDVYAFGIVLYELMTGQLPYSNINNRDQIIFMVGRGYLSPDLSKVRSNCPKAMKRLMAECLKKKRDERPLFPQILASIELLARSLPKIHRSASEPSLNRAGFQTEDFSLYACASPKTPIQAGGYGEFAAFK

SEQ ID NO: 7 - DNA, 2232 bp, Oryctolagus cuniculus
atggggaatgtgtggaatatcaaacaaatgattaagttgacacaggagcatatagaggccctattggacaaatttggtggggagcataatccaccatcaatatatctggaggcctacgaagaatacaccagcaagctagatgccctccaacaaagagaacagcagttattggaatccctagtttttcaaaatcccacagatgtgtcacggagcaaccccaagtcaccacaaaaacctattgttagagtcttcctgcccaacaaacagaggacagtggtacctgcaagatgtggagttacggttcgagacagtctaaagaaagcgctgatgatgagaggtctgatcccagaatgctgtgctgtttacagaattcaggatggagagaagaagccaattggctgggacactgatatttcctggctcactggagaagagctgcatgtggaagtgttagagaatgtcccactcaccacacataactttgtacggaaaacttttttcaccttagcattttgtgacttctgtagaaagctgcttttccagggtttccgctgtcaaacatgtggctacaaatttcaccagcgttgtagtacggaagttccactgatgtgtgttaattatgaccaacttgatttgctgtttgtctccaagttctttgaacaccacccagtaccacaggaggaggcctccttagcagagactgccctcacatctgggtcatcgccttccgcacctccctcagactctattgggcaccaaattctcaccagtccgtccccttcaaaatccattccgattccacagtccttccgaccagcagatgaagatcatcgaaatcagtttgggcaacgagaccggtcttcatcagcgcctaatgttcacattaacacaatagaacctgtcaatattgatgaaaaattcccagaagtggaattacaggatcaaagggacttgattagagaccaagggtttcgtggtgatggagcccctttgaaccagctgatgcgctgtcttcggaaataccaatcccggactcccagtcccctcctaccttctgtccccagtgacatagtgtttgattttgagcctggcccagtgttcagaggatcgaccacgggtttgtctgccactccccctgcctcattacctggctcactcactagtgtgaaagctgtacagagatccccaggacctcagcgagagaggaagtcgtcttcctcctcagaagacaggaatcgaatgaaaactcttggtagacgggattcaagtgatgattgggagattcctgatgggcagatcaccgtgggacagagaattggatctggatcatttggaaccgtctacaagggaaaatggcacggtgatgtggcagtaaaaatgttgaatgtgacagcacctacacctcagcagttacaggccttcaaaaatgaagtaggagtactcaggaaaacacgacatgtgaatatcctacttttcatgggctattccacaaagccacagctggctattgttacccagtggtgtgagggctccagtttatatcaccatctccacatcattgagaccaaattcgagatgatcaaacttatagatattgcacggcagactgcacagggcatggattacttacacgccaagtcaatcatccacagagacctcaagagtaataatatatttcttcatgaagacctcacagtaaaaataggtgattttggtctagccacagtgaaatctcgatggagtgggtcccatcagtttgaacaattgtctggatccattttgtggatggcaccagaagtaatcagaatgcaagacaaaaacccatatagctttcagtcagatgtatatgcatttgggattgttctgtatgaattgatgactgggcagttaccttactcaaacatcaacaacagggaccagatcatttttatggtgggacgtggctacctgtctccagacctcagtaaggtacggagtaactgtccgaaagccatgaagagattaatggcagagtgcctcaaaaagaaaagagatgagagaccactctttccccaaattctcgcctccattgagctgctggcccgctcattgccaaaaatccaccgcagtgcatcagaaccctccttgaatcgggctggtttccagacagaggattttagtctatatgcttgtgcttctccaaaaacacccatccaggcagggggatatggagaatttgcagccttcaagtag

SEQ ID NO: 8 - protein, 743 aa, Oryctolagus cuniculus
MGNVWNIKQMIKLTQEHIEALLDKFGGEHNPPSIYLEAYEEYTSKLDALQQREQQLLESLVFQNPTDVSRSNPKSPQKPIVRVFLPNKQRTVVPARCGVTVRDSLKKALMMRGLIPECCAVYRIQDGEKKPIGWDTDISWLTGEELHVEVLENVPLTTHNFVRKTFFTLAFCDFCRKLLFQGFRCQTCGYKFHQRCSTEVPLMCVNYDQLDLLFVSKFFEHHPVPQEEASLAETALTSGSSPSAPPSDSIGHQILTSPSPSKSIPIPQSFRPADEDHRNQFGQRDRSSSAPNVHINTIEPVNIDEKFPEVELQDQRDLIRDQGFRGDGAPLNQLMRCLRKYQSRTPSPLLPSVPSDIVFDFEPGPVFRGSTTGLSATPPASLPGSLTSVKAVQRSPGPQRERKSSSSSEDRNRMKTLGRRDSSDDWEIPDGQITVGQRIGSGSFGTVYKGKWHGDVAVKMLNVTAPTPQQLQAFKNEVGVLRKTRHVNILLFMGYSTKPQLAIVTQWCEGSSLYHHLHIIETKFEMIKLIDIARQTAQGMDYLHAKSIIHRDLKSNNIFLHEDLTVKIGDFGLATVKSRWSGSHQFEQLSGSILWMAPEVIRMQDKNPYSFQSDVYAFGIVLYELMTGQLPYSNINNRDQIIFMVGRGYLSPDLSKVRSNCPKAMKRLMAECLKKKRDERPLFPQILASIELLARSLPKIHRSASEPSLNRAGFQTEDFSLYACASPKTPIQAGGYGEFAAFK

SEQ ID NO: 9 - DNA, 2186 bp, Cavia porcellus
atggcggcgctcagcggcggcggtggcgcggagcagggccaggctctgttcaacggggacatggagctcgaggccggcgccggcgccgcagcctcttcggctgcagaccctgccattcccgaggaggtatggaatatcaaacaaatgattaagttgacgcaggaacacatagaggccctattggacaaatttggtggagagcataatccaccatcaatatacctggaggcctatgaagaatacaccagcaaactagatgccctccaacaaagagaacagcagttactggaatccctcgggaatggaactgatttttctgtttctagctctgcatcactggacaccgttacatcttcttcttcttctagcctttcagtactaccttcatctctttcagtttttcaaaatcctacagatgtgtcacggagcaaccccaaatcaccacaaaaacctattgttagagtcttcctgcccaacaaacagaggacagtggtacctgcaaggtgtggagttacagtccgagacagtctgaagaaagcactcatgatgagaggtcttatcccagagtgctgtgctgtgtacagaattcaggatggagaaaagaaaccaattggctgggacactgacatttcctggcttactggggaagaattacatgtagaagtattggagaatgttccacttacaacacacaattttgtatgtatctttatattttttttgctgtttgtctccaagttctttgaacaccacccaataccacaggaggaggcttccttagcagagaccacccttacatctggatcatccccttctgcacccccctcagagtccattgggcccccaattctcaccagcccatctccttcaaaatccattccaattccacagcctttccggccaggagaggaagatcatcgaaatcaatttgggcagcgagaccggtcctcatctgctcccaatgtgcatataaacacaatagaacctgtcaatattgatgatttgattagagaccaagggtttcgtagtgatggaggatcaactacaggtttgtctgccaccccacctgcctcattacctggctcactcactaatgtgaaagccttacagaaatctccaggacctcagcgagaaaggaagtcatcttcatcctcagaagacagaaatcgaatgaaaacgcttggtagacgggactcaagtgatgattgggagattcctgatgggcagattacagtgggacaaagaattggatctgggtcatttggaacagtctacaaggggaagtggcatggtgacgtggcagtgaaaatgttgaatgtgacagcacccacacctcaacagttacaggccttcaaaaatgaagtaggagtactcaggaaaacacgacatgtgaatatcctactcttcatgggctattccacaaagccacagctagctattgttacccagtggtgtgagggctccagcttataccaccatctccacatcatcgagaccaaatttgagatgatcaaacttatagatattgcacgacagactgcccagggcatggattacttacacgccaagtcaatcatccacagagacctcaagagtaataatatatttcttcacgaagacctcacggttaaaataggtgattttggtctagccacagtgaaatctcgatggagtgggtcccatcagtttgaacagttgtctggatccattttgtggatggcaccagaagtaatcagaatgcgagataaaaacccatacagttttcagtccgatgtatatgcatttgggattgttctatatgaattgatgactgggcagttaccctattcaaatatcaacaacagggaccagataatttttatggtgggacgaggatatctatctccagatctcagcaaggtacggagtaactgtccaaaagccatgaagaggttaatggcggagtgcctcaaaaagaaaagagatgagagaccactctttccccaaattctcgcctctattgagctgctggcccgctcattgccaaaaattcaccgcagtgcatcagaaccctccttgaatcgggctggtttccaaacagaggattttagtctctatgcttgtgcttctccaaaaacacccatccaggcagggggatatggtgcgtttcctgtccactgatgcaaattaaatgagtgagaaataaa

SEQ ID NO: 10 - protein, 719 aa, Cavia porcellus
MAALSGGGGAEQGQALFNGDMELEAGAGAAASSAADPAIPEEVWNIKQMIKLTQEHIEALLDKFGGEHNPPSIYLEAYEEYTSKLDALQQREQQLLESLGNGTDFSVSSSASLDTVTSSSSSSLSVLPSSLSVFQNPTDVSRSNPKSPQKPIVRVFLPNKQRTVVPARCGVTVRDSLKKALMMRGLIPECCAVYRIQDGEKKPIGWDTDISWLTGEELHVEVLENVPLTTHNFVCIFIFFLLFVSKFFEHHPIPQEEASLAETTLTSGSSPSAPPSESIGPPILTSPSPSKSIPIPQPFRPGEEDHRNQFGQRDRSSSAPNVHINTIEPVNIDDLIRDQGFRSDGGSTTGLSATPPASLPGSLTNVKALQKSPGPQRERKSSSSSEDRNRMKTLGRRDSSDDWEIPDGQITVGQRIGSGSFGTVYKGKWHGDVAVKMLNVTAPTPQQLQAFKNEVGVLRKTRHVNILLFMGYSTKPQLAIVTQWCEGSSLYHHLHIIETKFEMIKLIDIARQTAQGMDYLHAKSIIHRDLKSNNIFLHEDLTVKIGDFGLATVKSRWSGSHQFEQLSGSILWMAPEVIRMRDKNPYSFQSDVYAFGIVLYELMTGQLPYSNINNRDQIIFMVGRGYLSPDLSKVRSNCPKAMKRLMAECLKKKRDERPLFPQILASIELLARSLPKIHRSASEPSLNRAGFQTEDFSLYACASPKTPIQAGGYGAFPVH

SEQ ID NO: 11 - DNA, 3229 bp, Canis familiaris
gtaatgctggattttcatggaataagtttgacctgtgctgcagtggcctccagcaaggtacccgcaagatgtggagttacagtccgggacagtctaaagaaagctctgatgatgagaggtctaatcccagagtgctgtgctgtttacagaattcaggatggagagaagaaaccgattggctgggacactgatatttcctggctcactggagaggaattgcatgtagaagtgttggaaaatgttccgcttaccacacacaactttgtacggaaaacttttttcaccttagcattttgtgacttttgtcgaaagctgcttttccagggttttcgctgtcaaacatgtggttataaatttcaccagcgttgtagtacagaggttccactgatgtgtgttaattatgaccaacttgatttgctgtttgtctccaagttctttgaacaccacccaataccacaggaggaggcctccatagcagagactgcccttacgtctggatcatccccttctgctcccccctccgattctcctgggcccccaattctgaccagtccgtctccttcaaaatccattccaattccacagcctttccgaccagcagatgaagatcatcgaaatcagtttggacaacgagaccggtcctcatcagctccaaatgtgcatataaacacaatagaacccgtcaacattgatgacttgattagagaccaagggtttcgtagtgatggaggatcaaccacaggtttgtctgccaccccccctgcctcattgcctggctcactcactaatgtaaaagcattacagaaatctccaggacctcagcgggaaagaaaatcatcttcatcctcagaagataggaatcgaatgaaaacacttggtagacgggattcaagtgatgattgggagatacctgatgggcagatcacagtgggacagagaattggatccgggtcatttgggacagtctacaagggaaagtggcatggtgacgtggcagtgaaaatgttgaatgtgacagcacccacacctcagcagttacaggccttcaaaaatgaagtaggagtactcaggaaaactcgacatgtgaatatcctactctttatgggctattcaacaaagccccaactggctattgttacccagtggtgtgagggctccagcttatatcaccatctccacatcattgagaccaaatttgagatgataaagcttatagatattgcacggcagactgcacagggcatggattacttacacgccaagtcaatcatccacagagacctcaagagtaataatatttttcttcatgaagacctcacagtaaaaataggtgattttggtctagccacagtgaaatctcgatggagtgggtcccatcagtttgaacagttgtctggatccattttgtggatggcaccagaagtgatccgaatgcaagacaaaaacccatatagcttccagtcagatgtatacgcatttgggattgttctatatgaattgatgacagggcagttaccttattcaaacatcaacaacagggaccagataatttttatggtgggacgaggatatctttctccagatctcagtaaggtacggagtaactgtccaaaagccatgaagagattgatggcagagtgcctaaaaaagaaaagagatgagaggccactctttccccaaattctcgcctctattgagctgctggcccgctcattgccaaaaattcaccgcagtgcatcagaaccctccttgaatcgggctggcttccaaacagaggattttagtctctatgcttgcgcttctccaaaaacacccatccaggcagggggatacggagaatttgcagccttcaagtagccacaccatcatggcaacaactactcttatttcttaagtcttgtgttcgtacaatttgttaacatcaaaacacagttctgttcctcaaatctttttttaaagatacagaattttcaatgcataagctggtgtggaacagaatggaatttcccatccaacaaaagagggaagaatgttttaggaaccagaattctctgctgccagtgtttcttcttcaacacaaataccacgtgcatacaagtctgcccactcccaggaaggaagaggagagcctgagttctgaccttttgatggtcaggcatgatggaaagaaactgctgctacagcttgggagattggctgtggagagcctgcccgtcagctctgcccttctaaccgccagatgagtgtgtggctggtcacctgacagggcagctgcaatcgccaagcatcgttctctttcctgtcctgggattttgtcgtggagctctttccccctagtcaccaccggttcatttctgagggatggaacaaaaatgcagcatggcctttctgtgtggtgcatgtccggtctttgacaaatttttatcaagtgaagctcttgtatttaaatggagaatgagaggcgagggggggggatcacgttttggtgtaggggcaaagggaatgctgcatctttttcctgacccactgggtttctggcctttgtttccttgctcactgagggtgtctgcctataaccacgcaggctggaaagtgctggcacacattgccttctcttctcactgggtccagcaatgaagacaagtgttggggatttttttttttgccctccacaatgtagcaagttctcaggaaaatacagttaatatcttcctcctaagctcttccagtcatcaagtacttatgtggctactttgtccagggcacaaaatgccatggcggtatccaattaaaagcctacaaaactgcttgataacagttttgaatgtgtgagacatttatgtaatttaaatgtaaggtacaagttttaatttctgagtttctctattatatttttattaaaaagaaaataattttcagatttaattgaattggaataaaataatacttcccaccagaattatatatcctggaaaattgtatttttgttatataaacaacttttaaagaaagatcattatccttttctctacctaaatatggggagtcttagcataatgacagatatttataatttttaaattaatggtacttgctggatccacactaacatctttgctaatatctcatgttttcctccaacttactcctacactacatcctccatcctctttccagtcttttatctagaatatgcaacctaaaataaaaatggtggtgtctccattca

SEQ ID NO: 12 - protein, 617 aa, Canis familiaris
MLDFHGISLTCAAVASSKVPARCGVTVRDSLKKALMMRGLIPECCAVYRIQDGEKKPIGWDTDISWLTGEELHVEVLENVPLTTHNFVRKTFFTLAFCDFCRKLLFQGFRCQTCGYKFHQRCSTEVPLMCVNYDQLDLLFVSKFFEHHPIPQEEASIAETALTSGSSPSAPPSDSPGPPILTSPSPSKSIPIPQPFRPADEDHRNQFGQRDRSSSAPNVHINTIEPVNIDDLIRDQGFRSDGGSTTGLSATPPASLPGSLTNVKALQKSPGPQRERKSSSSSEDRNRMKTLGRRDSSDDWEIPDGQITVGQRIGSGSFGTVYKGKWHGDVAVKMLNVTAPTPQQLQAFKNEVGVLRKTRHVNILLFMGYSTKPQLAIVTQWCEGSSLYHHLHIIETKFEMIKLIDIARQTAQGMDYLHAKSIIHRDLKSNNIFLHEDLTVKIGDFGLATVKSRWSGSHQFEQLSGSILWMAPEVIRMQDKNPYSFQSDVYAFGIVLYELMTGQLPYSNINNRDQIIFMVGRGYLSPDLSKVRSNCPKAMKRLMAECLKKKRDERPLFPQILASIELLARSLPKIHRSASEPSLNRAGFQTEDFSLYACASPKTPIQAGGYGEFAAFK

SEQ ID NO: 13 - DNA, 1889 bp, Canis familiaris
ggaatatcaaacaaatgattaagttgacacaggaacatatagaagccctattggacaagtttggtggggagcataatccaccatcaatatatctggaggcctatgaagaatacaccagcaaactagatgccctccaacagcgagaacaacagttattggaatccctggggaatggaactgatttttctgtttctagctctgcatcaacggacaccgttacatcttcttcctcttctagcctttcagtgctaccttcatctctttcagtttttcaaaatcccacagatatatcacggagcaatcccaagtcaccacaaaaacctatcgttagagtcttcctgcccaataaacagaggacggtggtacccgcaagatgtggagttacagtccgggacagtctaaagaaagctctgatgatgagaggtctaatcccagagtgctgtgctgtttacagaattcaggatggagagaagaaaccgattggctgggacactgatatttcctggctcactggagaggaattgcatgtagaagtgttggaaaatgttccgcttaccacacacaactttgtacggaaaacttttttcaccttagcattttgtgacttttgtcgaaagctgcttttccagggttttcgctgtcaaacatgtggttataaatttcaccagcgttgtagtacagaggttccactgatgtgtgttaattatgaccaacttgatttgctgtttgtctccaagttctttgaacaccacccaataccacaggaggaggcctccatagcagagactgcccttacgtctggatcatccccttctgctcccccctccgattctcctgggcccccaattctgaccagtccgtctccttcaaaatccattccaattccacagcctttccgaccagcagatgaagatcatcgaaatcagtttggacaacgagaccggtcctcatcagctccaaatgtgcatataaacacaatagaacccgtcaacattgatgacttgattagagaccaagggtttcgtagtgatggaggatcaaccacaggtttgtctgccaccccccctgcctcattgcctggctcactcactaatgtaaaagcattacagaaatctccaggacctcagcgggaaagaaaatcatcttcatcctcagaagataggaatcgaatgaaaacacttggtagacgggattcaagtgatgattgggagatacctgatgggcagatcacagtgggacagagaattggatccgggtcatttgggacagtctacaagggaaagtggcatggtgacgtggcagtgaaaatgttgaatgtgacagcacccacacctcagcagttacaggccttcaaaaatgaagtaggagtactcaggaaaactcgacatgtgaatatcctactctttatgggctattcaacaaagccccaactggctattgttacccagtggtgtgagggctccagcttatatcaccatctccacatcattgagaccaaatttgagatgataaagcttatagatattgcacggcagactgcacagggcatggattacttacacgccaagtcaatcatccacagagacctcaagagtaataatatttttcttcatgaagacctcacagtaaaaataggtgattttggtctagccacagtgaaatctcgatggagtgggtcccatcagtttgaacagttgtctggatccattttgtggatggcaccagaagtgatccgaatgcaagacaaaaacccatatagcttccagtcagatgtatacgcatttgggattgttctatatgaattgatgacagggcagttaccttattcaaacatcaacaacagggaccagctcagatcatgatcacggtgtcatgagatcaagccccac

SEQ ID NO: 14 - protein, 615 aa, Canis familiaris
MIKLTQEHIEALLDKFGGEHNPPSIYLEAYEEYTSKLDALQQREQQLLESLGNGTDFSVSSSASTDTVTSSSSSSLSVLPSSLSVFQNPTDISRSNPKSPQKPIVRVFLPNKQRTVVPARCGVTVRDSLKKALMMRGLIPECCAVYRIQDGEKKPIGWDTDISWLTGEELHVEVLENVPLTTHNFVRKTFFTLAFCDFCRKLLFQGFRCQTCGYKFHQRCSTEVPLMCVNYDQLDLLFVSKFFEHHPIPQEEASIAETALTSGSSPSAPPSDSPGPPILTSPSPSKSIPIPQPFRPADEDHRNQFGQRDRSSSAPNVHINTIEPVNIDDLIRDQGFRSDGGSTTGLSATPPASLPGSLTNVKALQKSPGPQRERKSSSSSEDRNRMKTLGRRDSSDDWEIPDGQITVGQRIGSGSFGTVYKGKWHGDVAVKMLNVTAPTPQQLQAFKNEVGVLRKTRHVNILLFMGYSTKPQLAIVTQWCEGSSLYHHLHIIETKFEMIKLIDIARQTAQGMDYLHAKSIIHRDLKSNNIFLHEDLTVKIGDFGLATVKSRWSGSHQFEQLSGSILWMAPEVIRMQDKNPYSFQSDVYAFGIVLYELMTGQLPYSNINNRDQLRS

SEQ ID NO: 15 - DNA, 3521 bp, Felis catus
  misc_feature (630)..(649): n is a, c, g, or t
atgcctaacctcagtctctgccaccacggccaatttgctcatgtgcccactgtgtcggcactgggatattttgtgatttgccttggccattgtccactgtccttgacattgcctgaaggagaaccactgatgctaatgttgaaggtgacctttgcaggctctccactactcataccaaagatgcggccccctgataatcccagagccactgtctgcacatgggcaaaacaggctacattctgtgcagactggggagaaaggttccaagaacacagtgccatagttttgggcagagagtttcaacacagcatagtgtctatggcagtatctggatttggccgggggaagtgcccaagaggagacagtcaggctgtgtcctacggccaaggacctgcacttatttttgcatgcagtggtttagcacagggaagagaacgaagtaggaaatcggagccatggaaacggcagagcggaggaaacgtgcacgcgcgagggtgggcacgaaaggaaagaaccctccccagaagactgcgcgagggcgctcctaggattacgtcacgcaccccgcgaaaactgaaatgtactgtgtgtggtcttttaattgaactatcttccttatgtgcacttaannnnnnnnnnnnnnnnnnnngcggcggcggcggtggcgcggagcagggccaggctctgttcaacggggacatggagcccgaagccggcgccgcggcctcttcggctgcggaccctgccattcccgaggaggtgtggaatatcaaacaaatgattaagttgacacaggaacatatagaggccctattggacaaatttggtggggagcataatccaccatcaatatatctagaggcctatgaagaatacaccagcaagctagatgccctccaacagagagaacaacagttattggaatccctggggaatggaactgatttttctgtttctagctctgcatcaacagacaccgttacatcttcctcctcttctagcctttcagtgctaccttcatctctttcagtttttcaaaaccccacagatgtgtcacggagcaatcccaagtcaccacagaaacctatcgttagagtcttcctgcctaataaacagaggacagtggtacctgcaagatgtggagttacagtccgggacagtctaaagaaagctctgatgatgagaggtctaatccctgagtgctgtgctgtttacagaattcaggatggagagaagaaaccaattggctgggacactgatatctcctggctcaccggagaggaattgcatgtagaagtgttggaaaatgttccacttacaactcacaactttgtatgtacggaaaacgttttcaccttagcattttgtgacttttgtcgaaagctgcttttccaaggttttcgctgtcaaacgtgtggttataaatttcaccagcgttgtagtacagaggttccactgatgtgtgttaattatgaccaacttgatttgctgtttgtctccaagttctttgaacaccacccaataccacaggaggaggcctccatagcagagactgccctaacgtctggatcgtccccttctgcccccccctccgattctactgggccccaaattctcaccagtccgtctccttcaaaatccattccaattccacagcctttccgaccagcagatgaagatcatcgaaatcaatttggacagcgagaccggtcctcatcagctccaaatgtgcatataaatacaatagaacctgtcaatattgatgacttgattagagaccaggggtttcgtagtgatggaggatcaaccacaggcttgtctgccaccccccctgcctcattgccgggctctctcactaatgtaaaagcattacagaaatctccagggcctcagcgggaaaggaaatcttcttcatcctcagaagataggaatcgaatgaaaacacttggtagaagggattcaagtgatgattgggagattcctgatgggcagatcacagtgggacagagaattggatccgggtcatttgggacagtctacaagggaaagtggcatggtgatgtggcagtgaaaatgttgaatgtgacagcacccacacctcagcagttacaggccttcaaaaatgaagtaggagtactcaggaaaactcggcatgtgaacatcctgctcttcatgggctattcaacaaagccccagctggctattgtcacccagtggtgtgagggctccagcttataccaccatctccacatcatcgagaccaaattcgagatgatcaagctgatagatattgctcggcagactgcgcagggcatggattacttacacgccaagtcaatcatccacagagacctcaagagtaataatatttttcttcacgaagacctcacagtaaaaataggtgattttggtctagccacagtgaaatctcgatggagtgggtcccatcagtttgaacagttgtctggatccattttgtggatggcaccagaagtaattcgaatgcaagataaaaacccatatagctttcagtcagatgtatatgcatttgggattgttctatatgaattgatgactggacagttaccttattcaaacatcaacaacagggaccagataatttttatggtgggacgaggatatctttctccagatctcagtaaggtacgaagtaactgtccaaaagccatgaagagattgatggcagagtgcctaaaaaagaaaagagatgagaggccactgtttccccaaattcttgcctctattgagctgctggcccgctcattgccaaaaattcaccgcagtgcatcagaaccctccttgaatcgggctggcttccagacagaggattttagtctctatgcttgtgcttctccaaaaacacccatccaggcagggggatatggtgcgtttcccgtccactgagataagttagatgagtgcgcgagtgcagggggccggggccaaggaggtggaaatgtgcgtgcttctgtactaagttggatagcatcttcttttttaaaaaaagatgaaccaaagaatgtgtatgtttttaaagactagatataattatttcctgatctaaaatgtatacttagctttggattttcaatatccaagggttttcaaaatgcacagacattgctgaacatttgcagtacctcttctggaggctttacttcctgttacaaattggttttgtttactggcttatcctaattattaaacttcaattaaacttttctcctgcaccttttgttatgagctatcacatgtcccttagggactcgcaagagcagtactgcccccgtgtacgggcttgcaggtagaaaggggatgacgggttttaacacctgtgtgaggcaaggcagtccgaacagatctcatttaggaagccacgagagttgaataagttatttttattcttagtattttttctgtaactactttttattataacttggaaaatatggatgtcctttatacaccttagcaatagactgaatttctttttataaatt

SEQ ID NO: 16 - protein, 974 aa, Felis catus
  misc_feature (210)..(217): Xaa can be any naturally occurring amino acid
MPNLSLCHHGQFAHVPTVSALGYFVICLGHCPLSLTLPEGEPLMLMLKVTFAGSPLLIPKMRPPDNPRATVCTWAKQATFCADWGERFQEHSAIVLGREFQHSIVSMAVSGFGRGKCPRGDSQAVSYGQGPALIFACSGLAQGRERSRKSEPWKRQSGGNVHARGWARKERTLPRRLREGAPRITSRTPRKLKCTVCGLLIELSSLCALXXXXXXXXGGGGGAEQGQALFNGDMEPEAGAAASSAADPAIPEEVWNIKQMIKLTQEHIEALLDKFGGEHNPPSIYLEAYEEYTSKLDALQQREQQLLESLGNGTDFSVSSSASTDTVTSSSSSSLSVLPSSLSVFQNPTDVSRSNPKSPQKPIVRVFLPNKQRTVVPARCGVTVRDSLKKALMMRGLIPECCAVYRIQDGEKKPIGWDTDISWLTGEELHVEVLENVPLTTHNFVCTENVFTLAFCDFCRKLLFQGFRCQTCGYKFHQRCSTEVPLMCVNYDQLDLLFVSKFFEHHPIPQEEASIAETALTSGSSPSAPPSDSTGPQILTSPSPSKSIPIPQPFRPADEDHRNQFGQRDRSSSAPNVHINTIEPVNIDDLIRDQGFRSDGGSTTGLSATPPASLPGSLTNVKALQKSPGPQRERKSSSSSEDRNRMKTLGRRDSSDDWEIPDGQITVGQRIGSGSFGTVYKGKWHGDVAVKMLNVTAPTPQQLQAFKNEVGVLRKTRHVNILLFMGYSTKPQLAIVTQWCEGSSLYHHLHIIETKFEMIKLIDIARQTAQGMDYLHAKSIIHRDLKSNNIFLHEDLTVKIGDFGLATVKSRWSGSHQFEQLSGSILWMAPEVIRMQDKNPYSFQSDVYAFGIVLYELMTGQLPYSNINNRDQIIFMVGRGYLSPDLSKVRSNCPKAMKRLMAECLKKKRDERPLFPQILASIELLARSLPKIHRSASEPSLNRAGFQTEDFSLYACASPKTPIQAGGYGAFPVH

SEQ ID NO: 17 - DNA, 3853 bp, Bos taurus
ctcagctgcgccgggtctcacaagacggttcccgaggtggcccaggcgccgtcccaccgccgacgccgcccgggccgcccgggccgtccctccccgctgccccccgtcctccgcctccgcctccccccgccctcagcctcccttccccctccccgcccagcagcggtcgctcgggcccggctctcggttataagatggcggcgctgagtggcggcggcggcggcggcggcggtggcgcggagcagggccaggctctgttcaacggggacatggagcccgaggccggcgccgcggcctcttcggctgcggaccccgccattcccgaggaggtgtggaatatcaaacaaatgattaagttgacacaggagcatatagaggccctattggacaaatttggtggggagcataatccaccatcaatatatctggaggcctatgaagaatacaccagcaagctagatgccctccaacaaagagaacaacagttattggaatccctggggaatggaactgatttttctgtttctagctctgcatcaacggacaccgttacatcttcttcctcttctagcctttcagtgctgccttcatctctttcagtttttcaaaatcccacagatgtgtcacggagcaaccccaagtcaccacaaaaacctatcgttagagtcttcctgcccaataaacagaggacagtggtacctgcacggtgtggagtcacagtccgggacagcctgaagaaggcactgatgatgagaggtctaatcccagagtgctgtgctgtttacagaattcaggatggggagaagaaaccaattggctgggacactgatatttcctggcttactggagaggagttgcatgtagaagtgttggagaatgttccacttacaacacacaactttgtacggaaaacttttttcaccttagcattttgtgacttctgtagaaagctgcttttccagggattccgctgtcaaacatgtggttataaatttcaccagcgttgtagtacagaggttccactgatgtgtgttaattatgaccaactagatttgctgtttgtctccaagttctttgaacaccacccaataccacaggaggaggcctccttagcagagactacccttccatgtggctcatccccttctgcacccccctccgattctattgggcccccaattctcaccagtccatctccttcaaaatccattccaattccacagcctttccgaccagcagatgaagatcatcgaaatcagtttggacaacgagaccggtcctcatcagctccaaatgtgcatataaacacaatagaacccgtcaatattgatgacttgattagagaccaagggtttcgtagtgatggaggatcaaccacaggtttatccgccacaccccctgcctcattacctggctcactctctaatgtgaaagcattgcagaaatctccaggacctcagcgagaaagaaagtcctcttcatcctcagaagacaggaatcgaatgaaaacgcttggtagacgggattcaagtgacgattgggagattcctgatggacagatcacagtgggacaaagaattggatcagggtcatttgggacagtctacaagggaaagtggcatggtgatgtggcagtgaaaatgttgaatgtgacagcacccacacctcagcagttacaggccttcaaaaatgaagtaggagtactcaggaaaacgcgacatgtgaatatcctcctcttcatgggttattcaacaaagccacaactggctattgttacccagtggtgtgagggctccagtttatatcatcatctccacatcattgagaccaaattcgagatgatcaaacttatagatattgcacggcagactgcacagggcatggattacttacacgccaagtcaatcatccacagagacctcaagagtaataatatttttcttcatgaagacctcacagtaaaaataggtgattttggtctagccacagtgaaatctcgatggagtgggtcccatcagtttgaacagttgtctggatccattttgtggatggcaccagaagtaatcagaatgcaagataaaaacccatatagctttcagtcagatgtatatgcatttgggattgttctgtatgaattgatgaccggacagttaccttattcaaatatcaacaacagggaccagataatttttatggtgggacgaggatatctgtctccagatctcagtaaggtacggagtaactgtccaaaagccatgaagagattaatggcagagtgcctaaaaaagaaaagagatgaaagaccactctttccccaaattctcgcctctattgagctgctggcccgctcattgccaaaaattcaccgcagtgcatcagaaccctccttgaatcgggctggcttccaaacagaggattttagtctatatgcttgtgcttctccaaaaacacccattcaggcagggggatatggtacgtttcctgttcactgaaacaaaccgagtgagtgacagcatgtaggagggtagggacaaaagaaagtgaacaaatgtttgcttatatatttgttaaattgaataggattttctttttctttaaaggtgaacaagagaacatgtgtgtttttaaagtttggatatagttttcttcccagtctaaaacccatagttagcattacattttcaacatcgaatttttttttaattcatagacattgctgaaaatttataataccttttccagaggctttacttcccattccaagtttgttttgtttacttggttagtctaatcattaaactttaaactttccccacctaccttttgctgttagctatcccgcatccattaggggctccaagaacagcactgtctgcgtgtgtgtgttggcaggtgggaagctgatggtaagttaggctgtgttagtgaaggtaaactgaccaggtctaattaggagtcactagaattgaataagcttatttttattaatattttttcttataactatttctttttgtaataatttagaaaatataattgttctttattcccttacagcagtataaattattggtgcaggtaaccaaagatattactgaggagtggcatgtttgacatgagtgacatggtttaactttggatttttagttaatatttctttatatattaaggatgtcttacacattatagaagtcaaatttactgacaaaggtattgcctcctcttcctccccaaaaacacagcaaaattctctgggaactcgtagcattgttggttttcttttggatgactatggttgccaaacaaccaagtaattgattttttttaaattattattgctttagattatactcacctctcatgatgcctgttagcaatcacctttatccatgtgtcttgtaaaatatctttcctccttatattctttgcccaacaagagtctacttgttatgaatgagtactattttctttttttgattccccagtataattagtatgtttagtgctttctaggacttccactttcttatgttaaaaaaaaaaacaaactaatgtggcagtcagtatattcttactgtgaatcagagtctttactgggaatcaaagtgaaagaagcagctgttctgacttcagagtcagcctagggaccaaaaccagcctcttaaatacaccttcatttattcagtttggatttgtgatgattttcattatagctgacagttcaaggttattcagtggcacacagatagcatctgcataaatgcctttcttcttgaaaataaaggagaaaattgggaagactttacaccaatagtttagtctttaagtaccacagataacacacaccataaat

SEQ ID NO: 18 - protein, 764 aa, Bos taurus
AALSGGGGGGGGGAEQGQALFNGDMEPEAGAAASSAADPAIPEEVWNIKQMIKLTQEHIEALLDKFGGEHNPPSIYLEAYEEYTSKLDALQQREQQLLESLGNGTDFSVSSSASTDTVTSSSSSSLSVLPSSLSVFQNPTDVSRSNPKSPQKPIVRVFLPNKQRTVVPARCGVTVRDSLKKALMMRGLIPECCAVYRIQDGEKKPIGWDTDISWLTGEELHVEVLENVPLTTHNFVRKTFFTLAFCDFCRKLLFQGFRCQTCGYKFHQRCSTEVPLMCVNYDQLDLLFVSKFFEHHPIPQEEASLAETTLPCGSSPSAPPSDSIGPPILTSPSPSKSIPIPQPFRPADEDHRNQFGQRDRSSSAPNVHINTIEPVNIDDLIRDQGFRSDGGSTTGLSATPPASLPGSLSNVKALQKSPGPQRERKSSSSSEDRNRMKTLGRRDSSDDWEIPDGQITVGQRIGSGSFGTVYKGKWHGDVAVKMLNVTAPTPQQLQAFKNEVGVLRKTRHVNILLFMGYSTKPQLAIVTQWCEGSSLYHHLHIIETKFEMIKLIDIARQTAQGMDYLHAKSIIHRDLKSNNIFLHEDLTVKIGDFGLATVKSRWSGSHQFEQLSGSILWMAPEVIRMQDKNPYSFQSDVYAFGIVLYELMTGQLPYSNINNRDQIIFMVGRGYLSPDLSKVRSNCPKAMKRLMAECLKKKRDERPLFPQILASIELLARSLPKIHRSASEPSLNRAGFQTEDFSLYACASPKTPIQAGGYGTFPVH

SEQ ID NO: 19 - DNA, 4936 bp, Bos taurus
ctcagctgcgccgggtctcacaagacggttcccgaggtggcccaggcgccgtcccaccgccgacgccgcccgggccgcccgggccgtccctccccgctgccccccgtcctccgcctccgcctccccccgccctcagcctcccttccccctccccgcccagcagcggtcgctcgggcccggctctcggttataagatggcggcgctgagtggcggcggcggcggcggcggcggtggcgcggagcagggccaggctctgttcaacggggacatggagcccgaggccggcgccgcggcctcttcggctgcggaccccgccattcccgaggaggtgtggaatatcaaacaaatgattaagttgacacaggagcatatagaggccctattggacaaatttggtggggagcataatccaccatcaatatatctggaggcctatgaagaatacaccagcaagctagatgccctccaacaaagagaacaacagttattggaatccctggggaatggaactgatttttctgtttctagctctgcatcaacggacaccgttacatcttcttcctcttctagcctttcagtgctgccttcatctctttcagtttttcaaaatcccacagatgtgtcacggagcaaccccaagtcaccacaaaaacctatcgttagagtcttcctgcccaataaacagaggacagtggtacctgcacggtgtggagtcacagtccgggacagcctgaagaaggcactgatgatgagaggtctaatcccagagtgctgtgctgtttacagaattcaggatggggagaagaaaccaattggctgggacactgatatttcctggcttactggagaggagttgcatgtagaagtgttggagaatgttccacttacaacacacaactttgtacggaaaacttttttcaccttagcattttgtgacttctgtagaaagctgcttttccagggattccgctgtcaaacatgtggttataaatttcaccagcgttgtagtacagaggttccactgatgtgtgttaattatgaccaactagatttgctgtttgtctccaagttctttgaacaccacccaataccacaggaggaggcctccttagcagagactacccttccatgtggctcatccccttctgcacccccctccgattctattgggcccccaattctcaccagtccatctccttcaaaatccattccaattccacagcctttccgaccagcagatgaagatcatcgaaatcagtttggacaacgagaccggtcctcatcagctccaaatgtgcatataaacacaatagaacccgtcaatattgatgacttgattagagaccaagggtttcgtagtgatggaggatcaaccacaggtttatccgccacaccccctgcctcattacctggctcactctctaatgtgaaagcattgcagaaatctccaggacctcagcgagaaagaaagtcctcttcatcctcagaagacaggaatcgaatgaaaacgcttggtagacgggattcaagtgacgattgggagattcctgatggacagatcacagtgggacaaagaattggatcagggtcatttgggacagtctacaagggaaagtggcatggtgatgtggcagtgaaaatgttgaatgtgacagcacccacacctcagcagttacaggccttcaaaaatgaagtaggagtactcaggaaaacgcgacatgtgaatatcctcctcttcatgggttattcaacaaagccacaactggctattgttacccagtggtgtgagggctccagtttatatcatcatctccacatcattgagaccaaattcgagatgatcaaacttatagatattgcacggcagactgcacagggcatggattacttacacgccaagtcaatcatccacagagacctcaagagtaataatatttttcttcatgaagacctcacagtaaaaataggtgattttggtctagccacagtgaaatctcgatggagtgggtcccatcagtttgaacagttgtctggatccattttgtggatggcaccagaagtaatcagaatgcaagataaaaacccatatagctttcagtcagatgtatatgcatttgggattgttctgtatgaattgatgaccggacagttaccttattcaaatatcaacaacagggaccagataatttttatggtgggacgaggatatctgtctccagatctcagtaaggtacggagtaactgtccaaaagccatgaagagattaatggcagagtgcctaaaaaagaaaagagatgaaagaccactctttccccaagtaggaaagactctcctaagcaagagacaaaattcagaagttatcagggaaaaagataagcagattctcgcctctattgagctgctggcccgctcattgccaaaaattcaccgcagtgcatcagaaccctccttgaatcgggctggcttccaaacagaggattttagtctatatgcttgtgcttctccaaaaacacccattcaggcagggggatatgaagcagatttggctcttacatcaaataaaaatagagtagaagttgggatttagagatttcctgacatgcaagaaggaataagcaagaaaaaaaggtttgttttccccaaatcatatctattgtcttttacttctattttttcttaaattttttgtgatttcagagacatgtagagttttattgatacctaaactatgagttcttttttttttttttttttcattattttgatttttttggccaagaggcatatgggatcttagcttgagaaagcaacaattttcttgatgtcattttgggtgagggcacatattgctgtgaacagtgtggtgatagccaccagggaccaaactcacacccgctgcattgaaaggtgaagtcttaaacactggaccagcagagaaattcctactctatgagttctttttgtcatcccctccccgcaccctccacccccaacctaaagtctgatgatgaaatcaacaactattccattagaagcagtagattctggtagcatgatctttagtttgttagtaagattttgtgctttgtggggttgtgtcgttttaaggctaatatttaagtttgtcaaatagaatgctgttcagattgtaaaaatgagtaataaacatctgaagttttttttaagttatttttaacatggtatatacagttgagcttagagtttatcattttctgatattctcttacttagtagatgaattctagccattttttataaagatttctgttaagcaaatcctgttttcacatgggcttcctttaagggattttagattctgctggatatggtgactgctcataagactgttgaaaattacttttaagatgtattagaatacttctgaaaaaaaatagcaaccttaaaaccataagcaaaagtagtaagggtgtttatacatttctagagtccctgtttaggtaatagcctcctatgattgtactttaaatgttttgctctccaaggttttagtaacttggctttttttctaatcagtgccaaactcccccagtttttttaactttaaatatgaggtaataaatcttttacccttccttgatcttttgacttataataccttggtcagttgtttcttaaaaggaatccttaaatggaaagagacaatatcactgtctgcagttctgattagtagttttattcagaatggaaaaacagattattcatttttgaaaattgttcaggggtatgttcattgttaggaccttggactttggagtcagtgcctagctatgcattccaggtctgccattttctggctgtgaaattttggacaagttacttaaccactttaaaccccagctttaagaagtaaattaaccccagtaaattaagaagtaatagcagccacttcgtagagttgttatgaggctcagatgcagtgcaaatgtgtataaagtattcagggagtcacctggtatactataatagacactagaatagttgccaatattatcagcatacaatctgaggattctgtcagccaatcattagcaatctgttgtttgttgggacatgccagtgttctccagttgaaatcagtagcaatctaaaaatggatagattattcctcatttaaatagtgtgttcatataagtgattgcttggatccttatcagaagttgctgttactgaaaaatgataaggctgactaaattgtgatagttgtcagttactaaccaactcccagaaatgaataagaggaacctatctctagttcctagtagaaggtatggacaaaatagtaggtgaaaaataatgtcttgaacccccaaattaagtaagctttaaagagtacaatacctcaaagggtctttgcggtttaaaatttgtatgctgagaatgatgttcattgacatgtgcctatatgtaattttttgatagtttaaaaggtgaaatgaactacagatgggagaggtctgaattttcttgccttcagtcaaatgtgtaatgtggacatattatttgacctgtgaattttatcttttaaaaaagattaattcctgcttcttccttcctaatagttgcattataataatgaaaatgagttgataatttggggggaaagtattctacaaatcaaccttattattttaccattggtttctgagaaattttgttcatttgaaccgtttatagcttgattagaatcatagcatgtaaaacccaactgagggattatctgcagacttaatgtagtattatgtaagttgtcttctttcatttcgaccttttttgcttttgttgttgctagatctgtagtatgtagctagtcacctttcagcgaggtttcagcgaggcttttctgtgtctctaggttatttgagataacttttttaaaattagctcttgtcctcc

SEQ ID NO: 20 - protein, 797 aa, Bos taurus
MAALSGGGGGGGGGAEQGQALFNGDMEPEAGAAASSAADPAIPEEVWNIKQMIKLTQEHIEALLDKFGGEHNPPSIYLEAYEEYTSKLDALQQREQQLLESLGNGTDFSVSSSASTDTVTSSSSSSLSVLPSSLSVFQNPTDVSRSNPKSPQKPIVRVFLPNKQRTVVPARCGVTVRDSLKKALMMRGLIPECCAVYRIQDGEKKPIGWDTDISWLTGEELHVEVLENVPLTTHNFVRKTFFTLAFCDFCRKLLFQGFRCQTCGYKFHQRCSTEVPLMCVNYDQLDLLFVSKFFEHHPIPQEEASLAETTLPCGSSPSAPPSDSIGPPILTSPSPSKSIPIPQPFRPADEDHRNQFGQRDRSSSAPNVHINTIEPVNIDDLIRDQGFRSDGGSTTGLSATPPASLPGSLSNVKALQKSPGPQRERKSSSSSEDRNRMKTLGRRDSSDDWEIPDGQITVGQRIGSGSFGTVYKGKWHGDVAVKMLNVTAPTPQQLQAFKNEVGVLRKTRHVNILLFMGYSTKPQLAIVTQWCEGSSLYHHLHIIETKFEMIKLIDIARQTAQGMDYLHAKSIIHRDLKSNNIFLHEDLTVKIGDFGLATVKSRWSGSHQFEQLSGSILWMAPEVIRMQDKNPYSFQSDVYAFGIVLYELMTGQLPYSNINNRDQIIFMVGRGYLSPDLSKVRSNCPKAMKRLMAECLKKKRDERPLFPQVGKTLLSKRQNSEVIREKDKQILASIELLARSLPKIHRSASEPSLNRAGFQTEDFSLYACASPKTPIQAGGYEADLALTSNKNRVEVGI

SEQ ID NO: 21 - DNA, 4154 bp, Bos taurus
ctcagctgcgccgggtctcacaagacggttcccgaggtggcccaggcgccgtcccaccgccgacgccgcccgggccgcccgggccgtccctccccgctgccccccgtcctccgcctccgcctccccccgccctcagcctcccttccccctccccgcccagcagcggtcgctcgggcccggctctcggttataagatggcggcgctgagtggcggcggcggcggcggcggcggtggcgcggagcagggccaggctctgttcaacggggacatggagcccgaggccggcgccgcggcctcttcggctgcggaccccgccattcccgaggaggtgtggaatatcaaacaaatgattaagttgacacaggagcatatagaggccctattggacaaatttggtggggagcataatccaccatcaatatatctggaggcctatgaagaatacaccagcaagctagatgccctccaacaaagagaacaacagttattggaatccctggggaatggaactgatttttctgtttctagctctgcatcaacggacaccgttacatcttcttcctcttctagcctttcagtgctgccttcatctctttcagtttttcaaaatcccacagatgtgtcacggagcaaccccaagtcaccacaaaaacctatcgttagagtcttcctgcccaataaacagaggacagtggtacctgcacggtgtggagtcacagtccgggacagcctgaagaaggcactgatgatgagaggtctaatcccagagtgctgtgctgtttacagaattcaggatggggagaagaaaccaattggctgggacactgatatttcctggcttactggagaggagttgcatgtagaagtgttggagaatgttccacttacaacacacaactttgtacggaaaacttttttcaccttagcattttgtgacttctgtagaaagctgcttttccagggattccgctgtcaaacatgtggttataaatttcaccagcgttgtagtacagaggttccactgatgtgtgttaattatgaccaactagatttgctgtttgtctccaagttctttgaacaccacccaataccacaggaggaggcctccttagcagagactacccttccatgtggctcatccccttctgcacccccctccgattctattgggcccccaattctcaccagtccatctccttcaaaatccattccaattccacagcctttccgaccagcagatgaagatcatcgaaatcagtttggacaacgagaccggtcctcatcagctccaaatgtgcatataaacacaatagaacccgtcaatattgatgacttgattagagaccaagggtttcgtagtgatggaggatcaaccacaggtttatccgccacaccccctgcctcattacctggctcactctctaatgtgaaagcattgcagaaatctccaggacctcagcgagaaagaaagtcctcttcatcctcagaagacaggaatcgaatgaaaacgcttggtagacgggattcaagtgacgattgggagattcctgatggacagatcacagtgggacaaagaattggatcagggtcatttgggacagtctacaagggaaagtggcatggtgatgtggcagtgaaaatgttgaatgtgacagcacccacacctcagcagttacaggccttcaaaaatgaagtaggagtactcaggaaaacgcgacatgtgaatatcctcctcttcatgggttattcaacaaagccacaactggctattgttacccagtggtgtgagggctccagtttatatcatcatctccacatcattgagaccaaattcgagatgatcaaacttatagatattgcacggcagactgcacagggcatggattacttacacgccaagtcaatcatccacagagacctcaagagtaataatatttttcttcatgaagacctcacagtaaaaataggtgattttggtctagccacagtgaaatctcgatggagtgggtcccatcagtttgaacagttgtctggatccattttgtggatggcaccagaagtaatcagaatgcaagataaaaacccatatagctttcagtcagatgtatatgcatttgggattgttctgtatgaattgatgaccggacagttaccttattcaaatatcaacaacagggaccagataatttttatggtgggacgaggatatctgtctccagatctcagtaaggtacggagtaactgtccaaaagccatgaagagattaatggcagagtgcctaaaaaagaaaagagatgaaagaccactctttccccaagtaggaaagactctcctaagcaagagacaaaattcagaagttatcagggaaaaagataagcagattctcgcctctattgagctgctggcccgctcattgccaaaaattcaccgcagtgcatcagaaccctccttgaatcgggctggcttccaaacagaggattttagtctatatgcttgtgcttctccaaaaacacccattcaggcagggggatatggctgagcacattgtccatcacccacaagtggctggttctcatcgcagaatctacgtagggaatcgggcgtgaaattcacttaagagatagagcagaggaagtgttctgtttacaggaatggagatgagagttatgagtaagttgcttagtcagttggctttgttttgaaaattattgtgttatatttgtgttaacctacttgtgttttgacagtatatgtcacataggaagaaacctcagactagcataataacaaagctcagactaggcacagatgtacacagaatggaccaaaatgggatgggggaaggtatgggaataagtctaggggtagggaaaaattgatgtgagggtgggaaataaactgtaattacctgaaataaaatgtaagagtgcaataagtgtgctttttattctaagctgtgaatgggttttttaaaaaaagcattccttcccaatgcatttgcctatgttccatagctgattaaaaccagctatataaacatatgcctttttattcatgttaattaccaatataaatggctaacctttacgtcttatttatcttcatgttatgttagtttacatacagggatgtgtgtgtgtgtgtatgctataaattttccctccttcgtttaaaaacgcgtttgttggatcctctctgtttccttaggccatgccacagctcatagtctcagcttggccttcctgtcacctgatctgaaggactatcacagtgacgtagctcgttcattggttgtacacactctaacccttttccttgctcagcaattactgtgtcttctaaaacaggagtgtacaaccatgagattgcaattaattgtttgacatatgtccctttgaattctatttattagttatgattgattgctctttggtttggaccaagaaaaacgaaatcccacctccccaccttttcacttatttcttactttgaggacaattctgtaagagagaggaaagggaactccttcatgttttaactgcagcaagttaatggccctggtttacaccaaacattatggtgattcacattcacattcctctcctctcttgctgccagaggtttgggttttgttcagttctgctcaagcactgaaaaagttttcatggagtctggagagtgcccagtgaaaagatggtttttaattgtccacagacctttctgttcctgctttgcaaaaattacaaaggagtaactatttttaaagcttatttttcaattcataaaaaagacatttattttcagtcagatgatgtctccttgtcccttaatcctcaatgtttgcttgaatcttttttttttttctgattttctcccatccccacttcttgatacttcttgagttctctttcctgctcaggtcctttcatttgtactttggagttttttctcatgtaaatttgtacaatggaaaatattgttcagtttggatagaacgcatggagaattaaataaaaaagatagctgaaattcagattgaaatttatttgtgtaaagttatttaaaaactctgtactatataaaaggcaaaaaaagttctatgtacttgatgtgaatatgcgaatactgctataataaagattgactgcatgga

SEQ ID NO: 22 - protein, 781 aa, Bos taurus
MAALSGGGGGGGGGAEQGQALFNGDMEPEAGAAASSAADPAIPEEVWNIKQMIKLTQEHIEALLDKFGGEHNPPSIYLEAYEEYTSKLDALQQREQQLLESLGNGTDFSVSSSASTDTVTSSSSSSLSVLPSSLSVFQNPTDVSRSNPKSPQKPIVRVFLPNKQRTVVPARCGVTVRDSLKKALMMRGLIPECCAVYRIQDGEKKPIGWDTDISWLTGEELHVEVLENVPLTTHNFVRKTFFTLAFCDFCRKLLFQGFRCQTCGYKFHQRCSTEVPLMCVNYDQLDLLFVSKFFEHHPIPQEEASLAETTLPCGSSPSAPPSDSIGPPILTSPSPSKSIPIPQPFRPADEDHRNQFGQRDRSSSAPNVHINTIEPVNIDDLIRDQGFRSDGGSTTGLSATPPASLPGSLSNVKALQKSPGPQRERKSSSSSEDRNRMKTLGRRDSSDDWEIPDGQITVGQRIGSGSFGTVYKGKWHGDVAVKMLNVTAPTPQQLQAFKNEVGVLRKTRHVNILLFMGYSTKPQLAIVTQWCEGSSLYHHLHIIETKFEMIKLIDIARQTAQGMDYLHAKSIIHRDLKSNNIFLHEDLTVKIGDFGLATVKSRWSGSHQFEQLSGSILWMAPEVIRMQDKNPYSFQSDVYAFGIVLYELMTGQLPYSNINNRDQIIFMVGRGYLSPDLSKVRSNCPKAMKRLMAECLKKKRDERPLFPQVGKTLLSKRQNSEVIREKDKQILASIELLARSLPKIHRSASEPSLNRAGFQTEDFSLYACASPKTPIQAGGYG

SEQ ID NO: 23 - DNA, 7914 bp, Bos taurus
ctcagctgcgccgggtctcacaagacggttcccgaggtggcccaggcgccgtcccaccgccgacgccgcccgggccgcccgggccgtccctccccgctgccccccgtcctccgcctccgcctccccccgccctcagcctcccttccccctccccgcccagcagcggtcgctcgggcccggctctcggttataagatggcggcgctgagtggcggcggcggcggcggcggcggtggcgcggagcagggccaggctctgttcaacggggacatggagcccgaggccggcgccgcggcctcttcggctgcggaccccgccattcccgaggaggtgtggaatatcaaacaaatgattaagttgacacaggagcatatagaggccctattggacaaatttggtggggagcataatccaccatcaatatatctggaggcctatgaagaatacaccagcaagctagatgccctccaacaaagagaacaacagttattggaatccctggggaatggaactgatttttctgtttctagctctgcatcaacggacaccgttacatcttcttcctcttctagcctttcagtgctgccttcatctctttcagtttttcaaaatcccacagatgtgtcacggagcaaccccaagtcaccacaaaaacctatcgttagagtcttcctgcccaataaacagaggacagtggtacctgcacggtgtggagtcacagtccgggacagcctgaagaaggcactgatgatgagaggtctaatcccagagtgctgtgctgtttacagaattcaggatggggagaagaaaccaattggctgggacactgatatttcctggcttactggagaggagttgcatgtagaagtgttggagaatgttccacttacaacacacaactttgtacggaaaacttttttcaccttagcattttgtgacttctgtagaaagctgcttttccagggattccgctgtcaaacatgtggttataaatttcaccagcgttgtagtacagaggttccactgatgtgtgttaattatgaccaactagatttgctgtttgtctccaagttctttgaacaccacccaataccacaggaggaggcctccttagcagagactacccttccatgtggctcatccccttctgcacccccctccgattctattgggcccccaattctcaccagtccatctccttcaaaatccattccaattccacagcctttccgaccagcagatgaagatcatcgaaatcagtttggacaacgagaccggtcctcatcagctccaaatgtgcatataaacacaatagaacccgtcaatattgatgacttgattagagaccaagggtttcgtagtgatggaggatcaaccacaggtttatccgccacaccccctgcctcattacctggctcactctctaatgtgaaagcattgcagaaatctccaggacctcagcgagaaagaaagtcctcttcatcctcagaagacaggaatcgaatgaaaacgcttggtagacgggattcaagtgacgattgggagattcctgatggacagatcacagtgggacaaagaattggatcagggtcatttgggacagtctacaagggaaagtggcatggtgatgtggcagtgaaaatgttgaatgtgacagcacccacacctcagcagttacaggccttcaaaaatgaagtaggagtactcaggaaaacgcgacatgtgaatatcctcctcttcatgggttattcaacaaagccacaactggctattgttacccagtggtgtgagggctccagtttatatcatcatctccacatcattgagaccaaattcgagatgatcaaacttatagatattgcacggcagactgcacagggcatggattacttacacgccaagtcaatcatccacagagacctcaagagtaataatatttttcttcatgaagacctcacagtaaaaataggtgattttggtctagccacagtgaaatctcgatggagtgggtcccatcagtttgaacagttgtctggatccattttgtggatggcaccagaagtaatcagaatgcaagataaaaacccatatagctttcagtcagatgtatatgcatttgggattgttctgtatgaattgatgaccggacagttaccttattcaaatatcaacaacagggaccagataatttttatggtgggacgaggatatctgtctccagatctcagtaaggtacggagtaactgtccaaaagccatgaagagattaatggcagagtgcctaaaaaagaaaagagatgaaagaccactctttccccaaattctcgcctctattgagctgctggcccgctcattgccaaaaattcaccgcagtgcatcagaaccctccttgaatcgggctggcttccaaacagaggattttagtctatatgcttgtgcttctccaaaaacacccattcaggcagggggatatggagaatttgcagccttcaagtagccacaccatcatgacagcatctactcttatttcttaagtcttgtgttcgtacaatttgttaacatcaaaacacagttctgttcctcaactctttttaaagttaaaatttttcagtgcataagctggtgtggaacagaaggaaatttcccatccaacaaaagagggaagaatgttttaggaaccagaattctctgctgccagtgtttcttcttcaacacaaatatcacaagtctgcccactcccaggaagaaagaggagagaccctgagttctgaccttttgatggtcaggcatgatggaaagaaactgctgctacagcttgggagatttgctctgggaagtctgccagtcaactttgcccttctaaccaccagatcaatatgtggctgatcatctgatggggcagttgcaatcaccaagccttgttctctttcctgttctgggattgtgttgtggaacccttttccctagccaccaccagttcatttctgagggatggaacaaaaatgcagcatgcccttcctgtgtggtgcatgttcagtccttgacaaatttttaccaaaatgaagctactttatttaaaaggagggtgagaggtgaggaggtcactttgggtgtggcggaaagggaatgctgcatctttttcctgggctgctggggctctggccttggcttgccagccggaagcgctggcacgcatcgccttcttttcccattgggtccagcaatgaagacgagtgtttggggttttttttttctccaccatgtagcaagttctcaggaaaatacaattgatatcttcctcctaagctcttccaatcagtcaccaagtacttatgtggttactttgtccagggcacaaaatgcctgtatctaattaaaagcctacaaaactgcttgataacagttttgaatgtgagacatttatgtaatttaaatgtaaggtacaagttttaatttctgagtttcttctattatatttttattaaaaaaagaaaataattttcagattgaattggagtaaaataatattacttcccactagaattatatatcctggaaaattgtatttttgttacataagcagcttttaaagaaagatcattacccttttctctacataaatatatggggagtcttagcctaatgacaaatatttataatttttaaattaatggtacttgctggatccatactaacatctttactaatacctcattgtttcttccaacttactcctacactacatcctacatcttcttcctagtcttttatctagaatatgcaacctcaaataaaaatggtggtgtcctcattcattctcctccttccttttttcccaagcctgatcttcaaaaggttggttaatttggcagctgagttcctccccaggcagagaatagaccaattttaggtgtattgggactgagggaggatgtgtaaagattaacatcagtaaagaaccgctgtggagtaattaagaactttgttctttataactggagaatataacctaaccctaacatccctcagcctttactaaagtgtggcgtaaatcacagtagtagcaaagaaagtgactctggatgtgttcctggccagtacctcccttatcatgaatgtagactctctcatcaagatttaggaatataaatcaaatcaaatgtgcccagccaagctatgtagtaagggacttgaacaatattaggcagaacctataaaataaatcagggaattagaaattatttaaagttttcaaattgtaaattgccccggtgtctttcagcctactgccattatttttgctacaatacctacatttcagaggagggcctactgaaaattccatgcaagtggaaaataatcctcaagttattaatgagtttgaaaagcaatgagttcttaagtctttgtgagtagagcaagatcctacaaaattcagaaatagtaaaaatggattcatgctgatttgaagagcatctgtgtgcataatataatgctgcatctcttttaaaagcagtctatttttctttttaaatttgtccccatagatgcttttgaacatgaacatgcttatgttaccttttccgaggttgggaagagccaggagctctcaggcagggccccctccctcagctgggcaggagctgctcaggaggagctagttatagaggaagcttagcgttggcattttcaaaattcaaggtgataacgctttcttcttcctttctgttttagaatagattgctgtctgatttgaaaaagggaaatagatttgatctcaaatgaatctgtgcccagaagccaggctcagggtattcagagatttgtatagtgccctcaaaaaataacaaaattttagctttccttttttcttcttttctccatcaaattcttttttctctagtttacaaatgacatggaaaaggaatttcccctgagttttgtatgcctttttttttttggcttagactatagataggcgtgttgagctcctaagaaaatacaaggaggaactctttgttgtgcagagcactttatgagtagtttgtgtggataatatgtgactgcttccctgacgagcttgtgaggctgtacttatgtctttcctgtaaggcagcttcagtgccttctgtagtgtatataaggaaagattacgccttctgaaaaatctcagagcaaccataagattattttaaaatatgtagtatgactgatggactttttcatcattaaattagtctagcatctaaacttttaccactgaaataatattgaccaaaaagcaatttataaaaggtatttgtgaatagaaaatacaatgtgatcatttgtacttatgtgcaccttaaaagaggaattctgtctagctgtcaaattctggttccttaacatccagtccttgattgtgattgagatctggtaggacgtgctggggcacgctagcagataaaatcccgtatactttaggatagatgttacatttatgtcagtgttggcaaagagcattgtgtagtaataaagaattcaagacttcagcaatgtcaacctgaaactttgtaaatatttcctagattgttatttgatgcagtcacagctctttatcacacaatgttgtctttccctcatcaggcaattttagaactgctgcacacccctcctcagatctcacctgcccctcctgtacattcacctctccagccttgtgcacacctcatttagctttagtttgaaacacattgcagggttcaggtgacctcttcaaaaactacctcctcagaatgaggtaatgaatagttatttattttaaaatatgaaaagtcaggagctctagaatatgaagatgatctaagattttaacttttatgtatacttgttgagcactctccttttgtcctaaagggcattatacatttaagcagtaatactgaaaaatgtagctcagagtaactgaatgttgttgaaagtggtgccagaatctgttttaggggtacgtatcagaatcttaatcttaaatcggttacatgaaattaaatagttaatggtaacacttgactaacagatataattttaattttcggtaggcttttagcaagacagtaagtacatcttcataatgagttagccacagcttcatcacatgcacagattttcctgttgagagactgcccagttaagagggtagaatgatgaaccatttttcaggattctcttctttgtccaaactggcattgtgagtgctagaatatcagcactttcaaactagtgattccaactattaggctattaaaaagcaaaacaaaccaaacaaaccatagccagacatgggaagtttactatgagtataaacagcaaatagcttacaggtcatacattgaaatggtgtaggtaaggcgttagaaaaataccttgacaatttgccaaatgatcttactgtgccttcatgatgcaataaaaaaaaaaaaaatttagcataaatcagtgatttgtgaagagagcagccaccctggtctaactcagctgtgttaatattttttagcgtgcaatttagactgcaaagataaatgcactaaagagtttatagccaaaatcacatttaaaaaatgagagaaaacacaggtaaattttcagtgaacaaaattatttttttaaagtacataatccctagtatagtcagatatatttatcacatagagcaaataggttgaaatcacaattcagtgacatttctagagaaactttttctactcccataggttcttcaaagcatggaacttttatataacagaaatgtgtgacggtcattttaaattgctgtagtttggggctgaagtactgtgtgctgggcagcaatcacatgtattaactagtgagaaaggagaaattaagatataggacagaatttgattttcttgttcccagattactgctgccaacctagacactgagtttccagaggctgaaacgtaaacttgcagctcagcaactgttttgcaaagttagtgggactgtcctgcttatgctgttcaaaaatgctctgagggccaggtggggcctccaggggctcctctctgaggggacatcagactagctaacgacctggcgggcggatgtgaaccggacacactccatggtgtgcttcttgtatcggtccctcgccaccctcaagaaaggcttcagcgggttctctagacgtctccactaaggtgtgttactaacagccatgggttgttgagcacccgaggagtgcaatagcatctctgcatgattgtatattggcccgaagagaatgaagtggccagtgtactcatgttccatgttgctagctctggtaaactgaaaatactggtaagatttttgttttatcagtacactagagagtaagctttgttttgttgtttttagataatgttttcacttccatttggaaagacatttaaattgagtttcagtcctaaattttgccagtcatggtaattagcagtttctatcaggtatttttaaggtagaagaggatagaaacataagttctaaaagcttaaggtaaccgtggtttattttaaaatgtttaggggtggttagtctctacctcaaaaaaagtgagtgaatcttttatttcagcattcacaagttcggctgttgtttttgtaatacattttttttttaaccttttgacccccctttacctaagtgtcaatgtagttttattaattactaagtcagtttcattaaaatgtttatttagcagttttgactaattgcaatgattaatatagccagttgtgcatgaggacacagccagtgagtatatctgggttttttttgtgatgctttttttcttaagacttctgtagatttatgaagtactcattgaaaacaactaaaatacgtttattcgtgttaatatggaaaaaaaaaaa

SEQ ID NO: 24 - protein, 766 aa, Bos taurus
MAALSGGGGGGGGGAEQGQALFNGDMEPEAGAAASSAADPAIPEEVWNIKQMIKLTQEHIEALLDKFGGEHNPPSIYLEAYEEYTSKLDALQQREQQLLESLGNGTDFSVSSSASTDTVTSSSSSSLSVLPSSLSVFQNPTDVSRSNPKSPQKPIVRVFLPNKQRTVVPARCGVTVRDSLKKALMMRGLIPECCAVYRIQDGEKKPIGWDTDISWLTGEELHVEVLENVPLTTHNFVRKTFFTLAFCDFCRKLLFQGFRCQTCGYKFHQRCSTEVPLMCVNYDQLDLLFVSKFFEHHPIPQEEASLAETTLPCGSSPSAPPSDSIGPPILTSPSPSKSIPIPQPFRPADEDHRNQFGQRDRSSSAPNVHINTIEPVNIDDLIRDQGFRSDGGSTTGLSATPPASLPGSLSNVKALQKSPGPQRERKSSSSSEDRNRMKTLGRRDSSDDWEIPDGQITVGQRIGSGSFGTVYKGKWHGDVAVKMLNVTAPTPQQLQAFKNEVGVLRKTRHVNILLFMGYSTKPQLAIVTQWCEGSSLYHHLHIIETKFEMIKLIDIARQTAQGMDYLHAKSIIHRDLKSNNIFLHEDLTVKIGDFGLATVKSRWSGSHQFEQLSGSILWMAPEVIRMQDKNPYSFQSDVYAFGIVLYELMTGQLPYSNINNRDQIIFMVGRGYLSPDLSKVRSNCPKAMKRLMAECLKKKRDERPLFPQILASIELLARSLPKIHRSASEPSLNRAGFQTEDFSLYACASPKTPIQAGGYGEFAAFK

SEQ ID NO: 25 - DNA, 4670 bp, Bos taurus
ggtgtgtcatagtgcagcagattgaatgcagaagatatgaaaattcagatgtcttctgttaaggtgtggaatatcaaacaaatgattaagttgacacaggagcatatagaggccctattggacaaatttggtggggagcataatccaccatcaatatatctggaggcctatgaagaatacaccagcaagctagatgccctccaacaaagagaacaacagttattggaatccctggggaatggaactgatttttctgtttctagctctgcatcaacggacaccgttacatcttcttcctcttctagcctttcagtgctgccttcatctctttcagtttttcaaaatcccacagatgtgtcacggagcaaccccaagtcaccacaaaaacctatcgttagagtcttcctgcccaataaacagaggacagtggtacctgcacggtgtggagtcacagtccgggacagcctgaagaaggcactgatgatgagaggtctaatcccagagtgctgtgctgtttacagaattcaggatggggagaagaaaccaattggctgggacactgatatttcctggcttactggagaggagttgcatgtagaagtgttggagaatgttccacttacaacacacaactttgtacggaaaacttttttcaccttagcattttgtgacttctgtagaaagctgcttttccagggattccgctgtcaaacatgtggttataaatttcaccagcgttgtagtacagaggttccactgatgtgtgttaattatgaccaactagatttgctgtttgtctccaagttctttgaacaccacccaataccacaggaggaggcctccttagcagagactacccttccatgtggctcatccccttctgcacccccctccgattctattgggcccccaattctcaccagtccatctccttcaaaatccattccaattccacagcctttccgaccagcagatgaagatcatcgaaatcagtttggacaacgagaccggtcctcatcagctccaaatgtgcatataaacacaatagaacccgtcaatattgatgacttgattagagaccaagggtttcgtagtgatggaggatcaaccacaggtttatccgccacaccccctgcctcattacctggctcactctctaatgtgaaagcattgcagaaatctccaggacctcagcgagaaagaaagtcctcttcatcctcagaagacaggaatcgaatgaaaacgcttggtagacgggattcaagtgacgattgggagattcctgatggacagatcacagtgggacaaagaattggatcagggtcatttgggacagtctacaagggaaagtggcatggtgatgtggcagtgaaaatgttgaatgtgacagcacccacacctcagcagttacaggccttcaaaaatgaagtaggagtactcaggaaaacgcgacatgtgaatatcctcctcttcatgggttattcaacaaagccacaactggctattgttacccagtggtgtgagggctccagtttatatcatcatctccacatcattgagaccaaattcgagatgatcaaacttatagatattgcacggcagactgcacagggcatggattacttacacgccaagtcaatcatccacagagacctcaagagtaataatatttttcttcatgaagacctcacagtaaaaataggtgattttggtctagccacagtgaaatctcgatggagtgggtcccatcagtttgaacagttgtctggatccattttgtggatggcaccagaagtaatcagaatgcaagataaaaacccatatagctttcagtcagatgtatatgcatttgggattgttctgtatgaattgatgaccggacagttaccttattcaaatatcaacaacagggaccagataatttttatggtgggacgaggatatctgtctccagatctcagtaaggtacggagtaactgtccaaaagccatgaagagattaatggcagagtgcctaaaaaagaaaagagatgaaagaccactctttccccaagtaggaaagactctcctaagcaagagacaaaattcagaagttatcagggaaaaagataagcagattctcgcctctattgagctgctggcccgctcattgccaaaaattcaccgcagtgcatcagaaccctccttgaatcgggctggcttccaaacagaggattttagtctatatgcttgtgcttctccaaaaacacccattcaggcagggggatatgaagcagatttggctcttacatcaaataaaaatagagtagaagttgggatttagagatttcctgacatgcaagaaggaataagcaagaaaaaaaggtttgttttccccaaatcatatctattgtcttttacttctattttttcttaaattttttgtgatttcagagacatgtagagttttattgatacctaaactatgagttcttttttttttttttttttcattattttgatttttttggccaagaggcatatgggatcttagcttgagaaagcaacaattttcttgatgtcattttgggtgagggcacatattgctgtgaacagtgtggtgatagccaccagggaccaaactcacacccgctgcattgaaaggtgaagtcttaaacactggaccagcagagaaattcctactctatgagttctttttgtcatcccctccccgcaccctccacccccaacctaaagtctgatgatgaaatcaacaactattccattagaagcagtagattctggtagcatgatctttagtttgttagtaagattttgtgctttgtggggttgtgtcgttttaaggctaatatttaagtttgtcaaatagaatgctgttcagattgtaaaaatgagtaataaacatctgaagttttttttaagttatttttaacatggtatatacagttgagcttagagtttatcattttctgatattctcttacttagtagatgaattctagccattttttataaagatttctgttaagcaaatcctgttttcacatgggcttcctttaagggattttagattctgctggatatggtgactgctcataagactgttgaaaattacttttaagatgtattagaatacttctgaaaaaaaatagcaaccttaaaaccataagcaaaagtagtaagggtgtttatacatttctagagtccctgtttaggtaatagcctcctatgattgtactttaaatgttttgctctccaaggttttagtaacttggctttttttctaatcagtgccaaactcccccagtttttttaactttaaatatgaggtaataaatcttttacccttccttgatcttttgacttataataccttggtcagttgtttcttaaaaggaatccttaaatggaaagagacaatatcactgtctgcagttctgattagtagttttattcagaatggaaaaacagattattcatttttgaaaattgttcaggggtatgttcattgttaggaccttggactttggagtcagtgcctagctatgcattccaggtctgccattttctggctgtgaaattttggacaagttacttaaccactttaaaccccagctttaagaagtaaattaaccccagtaaattaagaagtaatagcagccacttcgtagagttgttatgaggctcagatgcagtgcaaatgtgtataaagtattcagggagtcacctggtatactataatagacactagaatagttgccaatattatcagcatacaatctgaggattctgtcagccaatcattagcaatctgttgtttgttgggacatgccagtgttctccagttgaaatcagtagcaatctaaaaatggatagattattcctcatttaaatagtgtgttcatataagtgattgcttggatccttatcagaagttgctgttactgaaaaatgataaggctgactaaattgtgatagttgtcagttactaaccaactcccagaaatgaataagaggaacctatctctagttcctagtagaaggtatggacaaaatagtaggtgaaaaataatgtcttgaacccccaaattaagtaagctttaaagagtacaatacctcaaagggtctttgcggtttaaaatttgtatgctgagaatgatgttcattgacatgtgcctatatgtaattttttgatagtttaaaaggtgaaatgaactacagatgggagaggtctgaattttcttgccttcagtcaaatgtgtaatgtggacatattatttgacctgtgaattttatcttttaaaaaagattaattcctgcttcttccttcctaatagttgcattataataatgaaaatgagttgataatttggggggaaagtattctacaaatcaaccttattattttaccattggtttctgagaaattttgttcatttgaaccgtttatagcttgattagaatcatagcatgtaaaacccaactgagggattatctgcagacttaatgtagtattatgtaagttgtcttctttcatttcgaccttttttgcttttgttgttgctagatctgtagtatgtagctagtcacctttcagcgaggtttcagcgaggcttttctgtgtctctaggttatttgagataacttttttaaaattagctcttgtcctcc

SEQ ID NO: 26 - protein, 761 aa, Bos taurus
MKIQMSSVKVWNIKQMIKLTQEHIEALLDKFGGEHNPPSIYLEAYEEYTSKLDALQQREQQLLESLGNGTDFSVSSSASTDTVTSSSSSSLSVLPSSLSVFQNPTDVSRSNPKSPQKPIVRVFLPNKQRTVVPARCGVTVRDSLKKALMMRGLIPECCAVYRIQDGEKKPIGWDTDISWLTGEELHVEVLENVPLTTHNFVRKTFFTLAFCDFCRKLLFQGFRCQTCGYKFHQRCSTEVPLMCVNYDQLDLLFVSKFFEHHPIPQEEASLAETTLPCGSSPSAPPSDSIGPPILTSPSPSKSIPIPQPFRPADEDHRNQFGQRDRSSSAPNVHINTIEPVNIDDLIRDQGFRSDGGSTTGLSATPPASLPGSLSNVKALQKSPGPQRERKSSSSSEDRNRMKTLGRRDSSDDWEIPDGQITVGQRIGSGSFGTVYKGKWHGDVAVKMLNVTAPTPQQLQAFKNEVGVLRKTRHVNILLFMGYSTKPQLAIVTQWCEGSSLYHHLHIIETKFEMIKLIDIARQTAQGMDYLHAKSIIHRDLKSNNIFLHEDLTVKIGDFGLATVKSRWSGSHQFEQLSGSILWMAPEVIRMQDKNPYSFQSDVYAFGIVLYELMTGQLPYSNINNRDQIIFMVGRGYLSPDLSKVRSNCPKAMKRLMAECLKKKRDERPLFPQVGKTLLSKRQNSEVIREKDKQILASIELLARSLPKIHRSASEPSLNRAGFQTEDFSLYACASPKTPIQAGGYEADLALTSNKNRVEVGI

SEQ ID NO: 27 - DNA, 4816 bp, Bos taurus
ctcagctgcgccgggtctcacaagacggttcccgaggtggcccaggcgccgtcccaccgccgacgccgcccgggccgcccgggccgtccctccccgctgccccccgtcctccgcctccgcctccccccgccctcagcctcccttccccctccccgcccagcagcggtcgctcgggcccggctctcggttataagatggcggcgctgagtggcggcggcggcggcggcggcggtggcgcggagcagggccaggctctgttcaacggggacatggagcccgaggccggcgccgcggcctcttcggctgcggaccccgccattcccgaggaggtgtggaatatcaaacaaatgattaagttgacacaggagcatatagaggccctattggacaaatttggtggggagcataatccaccatcaatatatctggaggcctatgaagaatacaccagcaagctagatgccctccaacaaagagaacaacagttattggaatccctggggaatggaactgatttttctgtttctagctctgcatcaacggacaccgttacatcttcttcctcttctagcctttcagtgctgccttcatctctttcagtttttcaaaatcccacagatgtgtcacggagcaaccccaagtcaccacaaaaacctatcgttagagtcttcctgcccaataaacagaggacagtggtacctgcacggtgtggagtcacagtccgggacagcctgaagaaggcactgatgatgagaggtctaatcccagagtgctgtgctgtttacagaattcaggatggggagaagaaaccaattggctgggacactgatatttcctggcttactggagaggagttgcatgtagaagtgttggagaatgttccacttacaacacacaactttgtacggaaaacttttttcaccttagcattttgtgacttctgtagaaagctgcttttccagggattccgctgtcaaacatgtggttataaatttcaccagcgttgtagtacagaggttccactgatgtgtgttaattatgaccaactagagcccccaattctcaccagtccatctccttcaaaatccattccaattccacagcctttccgaccagcagatgaagatcatcgaaatcagtttggacaacgagaccggtcctcatcagctccaaatgtgcatataaacacaatagaacccgtcaatattgatgacttgattagagaccaagggtttcgtagtgatggaggatcaaccacaggtttatccgccacaccccctgcctcattacctggctcactctctaatgtgaaagcattgcagaaatctccaggacctcagcgagaaagaaagtcctcttcatcctcagaagacaggaatcgaatgaaaacgcttggtagacgggattcaagtgacgattgggagattcctgatggacagatcacagtgggacaaagaattggatcagggtcatttgggacagtctacaagggaaagtggcatggtgatgtggcagtgaaaatgttgaatgtgacagcacccacacctcagcagttacaggccttcaaaaatgaagtaggagtactcaggaaaacgcgacatgtgaatatcctcctcttcatgggttattcaacaaagccacaactggctattgttacccagtggtgtgagggctccagtttatatcatcatctccacatcattgagaccaaattcgagatgatcaaacttatagatattgcacggcagactgcacagggcatggattacttacacgccaagtcaatcatccacagagacctcaagagtaataatatttttcttcatgaagacctcacagtaaaaataggtgattttggtctagccacagtgaaatctcgatggagtgggtcccatcagtttgaacagttgtctggatccattttgtggatggcaccagaagtaatcagaatgcaagataaaaacccatatagctttcagtcagatgtatatgcatttgggattgttctgtatgaattgatgaccggacagttaccttattcaaatatcaacaacagggaccagataatttttatggtgggacgaggatatctgtctccagatctcagtaaggtacggagtaactgtccaaaagccatgaagagattaatggcagagtgcctaaaaaagaaaagagatgaaagaccactctttccccaagtaggaaagactctcctaagcaagagacaaaattcagaagttatcagggaaaaagataagcagattctcgcctctattgagctgctggcccgctcattgccaaaaattcaccgcagtgcatcagaaccctccttgaatcgggctggcttccaaacagaggattttagtctatatgcttgtgcttctccaaaaacacccattcaggcagggggatatgaagcagatttggctcttacatcaaataaaaatagagtagaagttgggatttagagatttcctgacatgcaagaaggaataagcaagaaaaaaaggtttgttttccccaaatcatatctattgtcttttacttctattttttcttaaattttttgtgatttcagagacatgtagagttttattgatacctaaactatgagttcttttttttttttttttttcattattttgatttttttggccaagaggcatatgggatcttagcttgagaaagcaacaattttcttgatgtcattttgggtgagggcacatattgctgtgaacagtgtggtgatagccaccagggaccaaactcacacccgctgcattgaaaggtgaagtcttaaacactggaccagcagagaaattcctactctatgagttctttttgtcatcccctccccgcaccctccacccccaacctaaagtctgatgatgaaatcaacaactattccattagaagcagtagattctggtagcatgatctttagtttgttagtaagattttgtgctttgtggggttgtgtcgttttaaggctaatatttaagtttgtcaaatagaatgctgttcagattgtaaaaatgagtaataaacatctgaagttttttttaagttatttttaacatggtatatacagttgagcttagagtttatcattttctgatattctcttacttagtagatgaattctagccattttttataaagatttctgttaagcaaatcctgttttcacatgggcttcctttaagggattttagattctgctggatatggtgactgctcataagactgttgaaaattacttttaagatgtattagaatacttctgaaaaaaaatagcaaccttaaaaccataagcaaaagtagtaagggtgtttatacatttctagagtccctgtttaggtaatagcctcctatgattgtactttaaatgttttgctctccaaggttttagtaacttggctttttttctaatcagtgccaaactcccccagtttttttaactttaaatatgaggtaataaatcttttacccttccttgatcttttgacttataataccttggtcagttgtttcttaaaaggaatccttaaatggaaagagacaatatcactgtctgcagttctgattagtagttttattcagaatggaaaaacagattattcatttttgaaaattgttcaggggtatgttcattgttaggaccttggactttggagtcagtgcctagctatgcattccaggtctgccattttctggctgtgaaattttggacaagttacttaaccactttaaaccccagctttaagaagtaaattaaccccagtaaattaagaagtaatagcagccacttcgtagagttgttatgaggctcagatgcagtgcaaatgtgtataaagtattcagggagtcacctggtatactataatagacactagaatagttgccaatattatcagcatacaatctgaggattctgtcagccaatcattagcaatctgttgtttgttgggacatgccagtgttctccagttgaaatcagtagcaatctaaaaatggatagattattcctcatttaaatagtgtgttcatataagtgattgcttggatccttatcagaagttgctgttactgaaaaatgataaggctgactaaattgtgatagttgtcagttactaaccaactcccagaaatgaataagaggaacctatctctagttcctagtagaaggtatggacaaaatagtaggtgaaaaataatgtcttgaacccccaaattaagtaagctttaaagagtacaatacctcaaagggtctttgcggtttaaaatttgtatgctgagaatgatgttcattgacatgtgcctatatgtaattttttgatagtttaaaaggtgaaatgaactacagatgggagaggtctgaattttcttgccttcagtcaaatgtgtaatgtggacatattatttgacctgtgaattttatcttttaaaaaagattaattcctgcttcttccttcctaatagttgcattataataatgaaaatgagttgataatttggggggaaagtattctacaaatcaaccttattattttaccattggtttctgagaaattttgttcatttgaaccgtttatagcttgattagaatcatagcatgtaaaacccaactgagggattatctgcagacttaatgtagtattatgtaagttgtcttctttcatttcgaccttttttgcttttgttgttgctagatctgtagtatgtagctagtcacctttcagcgaggtttcagcgaggcttttctgtgtctctaggttatttgagataacttttttaaaattagctcttgtcctcc

SEQ ID NO: 28 - protein, 757 aa, Bos taurus
MAALSGGGGGGGGGAEQGQALFNGDMEPEAGAAASSAADPAIPEEVWNIKQMIKLTQEHIEALLDKFGGEHNPPSIYLEAYEEYTSKLDALQQREQQLLESLGNGTDFSVSSSASTDTVTSSSSSSLSVLPSSLSVFQNPTDVSRSNPKSPQKPIVRVFLPNKQRTVVPARCGVTVRDSLKKALMMRGLIPECCAVYRIQDGEKKPIGWDTDISWLTGEELHVEVLENVPLTTHNFVRKTFFTLAFCDFCRKLLFQGFRCQTCGYKFHQRCSTEVPLMCVNYDQLEPPILTSPSPSKSIPIPQPFRPADEDHRNQFGQRDRSSSAPNVHINTIEPVNIDDLIRDQGFRSDGGSTTGLSATPPASLPGSLSNVKALQKSPGPQRERKSSSSSEDRNRMKTLGRRDSSDDWEIPDGQITVGQRIGSGSFGTVYKGKWHGDVAVKMLNVTAPTPQQLQAFKNEVGVLRKTRHVNILLFMGYSTKPQLAIVTQWCEGSSLYHHLHIIETKFEMIKLIDIARQTAQGMDYLHAKSIIHRDLKSNNIFLHEDLTVKIGDFGLATVKSRWSGSHQFEQLSGSILWMAPEVIRMQDKNPYSFQSDVYAFGIVLYELMTGQLPYSNINNRDQIIFMVGRGYLSPDLSKVRSNCPKAMKRLMAECLKKKRDERPLFPQVGKTLLSKRQNSEVIREKDKQILASIELLARSLPKIHRSASEPSLNRAGFQTEDFSLYACASPKTPIQAGGYEADLALTSNKNRVEVGI

SEQ ID NO: 29 - DNA, 2499 bp, Bos taurus
ctcagctgcgccgggtctcacaagacggttcccgaggtggcccaggcgccgtcccaccgccgacgccgcccgggccgcccgggccgtccctccccgctgccccccgtcctccgcctccgcctccccccgccctcagcctcccttccccctccccgcccagcagcggtcgctcgggcccggctctcggttataagatggcggcgctgagtggcggcggcggcggcggcggcggtggcgcggagcagggccaggctctgttcaacggggacatggagcccgaggccggcgccgcggcctcttcggctgcggaccccgccattcccgaggaggtgtggaatatcaaacaaatgattaagttgacacaggagcatatagaggccctattggacaaatttggtggggagcataatccaccatcaatatatctggaggcctatgaagaatacaccagcaagctagatgccctccaacaaagagaacaacagttattggaatccctggggaatggaactgatttttctgtttctagctctgcatcaacggacaccgttacatcttcttcctcttctagcctttcagtgctgccttcatctctttcagtttttcaaaatcccacagatgtgtcacggagcaaccccaagtcaccacaaaaacctatcgttagagtcttcctgcccaataaacagaggacagtggtacctgcacggtgtggagtcacagtccgggacagcctgaagaaggcactgatgatgagaggtctaatcccagagtgctgtgctgtttacagaattcaggatggggagaagaaaccaattggctgggacactgatatttcctggcttactggagaggagttgcatgtagaagtgttggagaatgttccacttacaacacacaactttgtacggaaaacttttttcaccttagcattttgtgacttctgtagaaagctgcttttccagggattccgctgtcaaacatgtggttataaatttcaccagcgttgtagtacagaggttccactgatgtgtgttaattatgaccaactagatttgctgtttgtctccaagttctttgaacaccacccaataccacaggaggaggcctccttagcagagactacccttccatgtggctcatccccttctgcacccccctccgattctattgggcccccaattctcaccagtccatctccttcaaaatccattccaattccacagcctttccgaccagcagatgaagatcatcgaaatcagtttggacaacgagaccggtcctcatcagctccaaatgtgcatataaacacaatagaacccgtcaatattgatgacttgattagagaccaagggtttcgtagtgatggaggatcaaccacaggtttatccgccacaccccctgcctcattacctggctcactctctaatgtgaaagcattgcagaaatctccaggacctcagcgagaaagaaagtcctcttcatcctcagaagacaggaatcgaatgaaaacgcttggtagacgggattcaagtgacgattgggagattcctgatggacagatcacagtgggacaaagaattggatcagggtcatttgggacagtctacaagggaaagtggcatggtgatgtggcagtgaaaatgttgaatgtgacagcacccacacctcagcagttacaggccttcaaaaatgaagtaggagtactcaggaaaacgcgacatgtgaatatcctcctcttcatgggttattcaacaaagccacaactggctattgttacccagtggtgtgagggctccagtttatatcatcatctccacatcattgagaccaaattcgagatgatcaaacttatagatattgcacggcagactgcacagggcatggattacttacacgccaagtcaatcatccacagagacctcaagagtaataatatttttcttcatgaagacctcacagtaaaaataggtgattttggtctagccacagtgaaatctcgatggagtgggtcccatcagtttgaacagttgtctggatccattttgtggatggcaccagaagtaatcagaatgcaagataaaaacccatatagctttcagtcagatgtatatgcatttgggattgttctgtatgaattgatgaccggacagttaccttattcaaatatcaacaacagggaccagataatttttatggtgggacgaggatatctgtctccagatctcagtaaggtacggagtaactgtccaaaagccatgaagagattaatggcagagtgcctaaaaaagaaaagagatgaaagaccactctttccccaagtaggaaagactctcctaagcaagagacaaaattcagaagttatcagggaaaaagataagcaggaaaagtatgtttctttagtacattccaggcatttgggattacagtaaaaacaatattctcgcctctattgagctgctggcccgctcattgccaaaaattcaccgcagtgcatcagaa

SEQ ID NO: 30 - protein, 744 aa, Bos taurus
MAALSGGGGGGGGGAEQGQALFNGDMEPEAGAAASSAADPAIPEEVWNIKQMIKLTQEHIEALLDKFGGEHNPPSIYLEAYEEYTSKLDALQQREQQLLESLGNGTDFSVSSSASTDTVTSSSSSSLSVLPSSLSVFQNPTDVSRSNPKSPQKPIVRVFLPNKQRTVVPARCGVTVRDSLKKALMMRGLIPECCAVYRIQDGEKKPIGWDTDISWLTGEELHVEVLENVPLTTHNFVRKTFFTLAFCDFCRKLLFQGFRCQTCGYKFHQRCSTEVPLMCVNYDQLDLLFVSKFFEHHPIPQEEASLAETTLPCGSSPSAPPSDSIGPPILTSPSPSKSIPIPQPFRPADEDHRNQFGQRDRSSSAPNVHINTIEPVNIDDLIRDQGFRSDGGSTTGLSATPPASLPGSLSNVKALQKSPGPQRERKSSSSSEDRNRMKTLGRRDSSDDWEIPDGQITVGQRIGSGSFGTVYKGKWHGDVAVKMLNVTAPTPQQLQAFKNEVGVLRKTRHVNILLFMGYSTKPQLAIVTQWCEGSSLYHHLHIIETKFEMIKLIDIARQTAQGMDYLHAKSIIHRDLKSNNIFLHEDLTVKIGDFGLATVKSRWSGSHQFEQLSGSILWMAPEVIRMQDKNPYSFQSDVYAFGIVLYELMTGQLPYSNINNRDQIIFMVGRGYLSPDLSKVRSNCPKAMKRLMAECLKKKRDERPLFPQVGKTLLSKRQNSEVIREKDKQEKYVSLVHSRHLGLQ

SEQ ID NO: 31 - DNA, 2404 bp, Bos taurus
ctcagctgcgccgggtctcacaagacggttcccgaggtggcccaggcgccgtcccaccgccgacgccgcccgggccgcccgggccgtccctccccgctgccccccgtcctccgcctccgcctccccccgccctcagcctcccttccccctccccgcccagcagcggtcgctcgggcccggctctcggttataagatggcggcgctgagtggcggcggcggcggcggcggcggtggcgcggagcagggccaggctctgttcaacggggacatggagcccgaggccggcgccgcggcctcttcggctgcggaccccgccattcccgaggaggtgtggaatatcaaacaaatgattaagttgacacaggagcatatagaggccctattggacaaatttggtggggagcataatccaccatcaatatatctggaggcctatgaagaatacaccagcaagctagatgccctccaacaaagagaacaacagttattggaatccctggggaatggaactgatttttctgtttctagctctgcatcaacggacaccgttacatcttcttcctcttctagcctttcagtgctgccttcatctctttcagtttttcaaaatcccacagatgtgtcacggagcaaccccaagtcaccacaaaaacctatcgttagagtcttcctgcccaataaacagaggacagtggtacctgcacggtgtggagtcacagtccgggacagcctgaagaaggcactgatgatgagaggtctaatcccagagtgctgtgctgtttacagaattcaggatggggagaagaaaccaattggctgggacactgatatttcctggcttactggagaggagttgcatgtagaagtgttggagaatgttccacttacaacacacaactttgtacggaaaacttttttcaccttagcattttgtgacttctgtagaaagctgcttttccagggattccgctgtcaaacatgtggttataaatttcaccagcgttgtagtacagaggttccactgatgtgtgttaattatgaccaactagatttgctgtttgtctccaagttctttgaacaccacccaataccacaggaggaggcctccttagcagagactacccttccatgtggctcatccccttctgcacccccctccgattctattgggcccccaattctcaccagtccatctccttcaaaatccattccaattccacagcctttccgaccagcagatgaagatcatcgaaatcagtttggacaacgagaccggtcctcatcagctccaaatgtgcatataaacacaatagaacccgtcaatattgatgacttgattagagaccaagggtttcgtagtgatggaggatcaaccacaggtttatccgccacaccccctgcctcattacctggctcactctctaatgtgaaagcattgcagaaatctccaggacctcagcgagaaagaaagtcctcttcatcctcagaagacaggaatcgaatgaaaacgcttggtagacgggattcaagtgacgattgggagattcctgatggacagatcacagtgggacaaagaattggatcagggtcatttgggacagtctacaagggaaagtggcatggtgatgtggcagtgaaaatgttgaatgtgacagcacccacacctcagcagttacaggccttcaaaaatgaagtaggagtactcaggaaaacgcgacatgtgaatatcctcctcttcatgggttattcaacaaagccacaactggctattgttacccagtggtgtgagggctccagtttatatcatcatctccacatcattgagaccaaattcgagatgatcaaacttatagatattgcacggcagactgcacagggcatggattacttacacgccaagtcaatcatccacagagacctcaagagtaataatatttttcttcatgaagacctcacagtaaaaataggtgattttggtctagccacagtgaaatctcgatggagtgggtcccatcagtttgaacagttgtctggatccattttgtggatggcaccagaagtaatcagaatgcaagataaaaacccatatagctttcagtcagatgtatatgcatttgggattgttctgtatgaattgatgaccggacagttaccttattcaaatatcaacaacagggaccagataatttttatggtgggacgaggatatctgtctccagatctcagtaaggtacggagtaactgtccaaaagccatgaagagattaatggcagagtgcctaaaaaagaaaagagatgaaagaccactctttccccaagatctctcttcccaccatagacacaaaaatttcagatggctacaggtttacatgtaaaaaacagaattataacaaatgatttttat

SEQ ID NO: 32 - protein, 726 aa, Bos taurus
MAALSGGGGGGGGGAEQGQALFNGDMEPEAGAAASSAADPAIPEEVWNIKQMIKLTQEHIEALLDKFGGEHNPPSIYLEAYEEYTSKLDALQQREQQLLESLGNGTDFSVSSSASTDTVTSSSSSSLSVLPSSLSVFQNPTDVSRSNPKSPQKPIVRVFLPNKQRTVVPARCGVTVRDSLKKALMMRGLIPECCAVYRIQDGEKKPIGWDTDISWLTGEELHVEVLENVPLTTHNFVRKTFFTLAFCDFCRKLLFQGFRCQTCGYKFHQRCSTEVPLMCVNYDQLDLLFVSKFFEHHPIPQEEASLAETTLPCGSSPSAPPSDSIGPPILTSPSPSKSIPIPQPFRPADEDHRNQFGQRDRSSSAPNVHINTIEPVNIDDLIRDQGFRSDGGSTTGLSATPPASLPGSLSNVKALQKSPGPQRERKSSSSSEDRNRMKTLGRRDSSDDWEIPDGQITVGQRIGSGSFGTVYKGKWHGDVAVKMLNVTAPTPQQLQAFKNEVGVLRKTRHVNILLFMGYSTKPQLAIVTQWCEGSSLYHHLHIIETKFEMIKLIDIARQTAQGMDYLHAKSIIHRDLKSNNIFLHEDLTVKIGDFGLATVKSRWSGSHQFEQLSGSILWMAPEVIRMQDKNPYSFQSDVYAFGIVLYELMTGQLPYSNINNRDQIIFMVGRGYLSPDLSKVRSNCPKAMKRLMAECLKKKRDERPLFPQDLSSHHRHKNFRWLQVYM

SEQ ID NO: 33 - DNA, 2331 bp, Bos taurus
ctcagctgcgccgggtctcacaagacggttcccgaggtggcccaggcgccgtcccaccgccgacgccgcccgggccgcccgggccgtccctccccgctgccccccgtcctccgcctccgcctccccccgccctcagcctcccttccccctccccgcccagcagcggtcgctcgggcccggctctcggttataagatggcggcgctgagtggcggcggcggcggcggcggcggtggcgcggagcagggccaggctctgttcaacggggacatggagcccgaggccggcgccgcggcctcttcggctgcggaccccgccattcccgaggaggtgtggaatatcaaacaaatgattaagttgacacaggagcatatagaggccctattggacaaatttggtggggagcataatccaccatcaatatatctggaggcctatgaagaatacaccagcaagctagatgccctccaacaaagagaacaacagttattggaatccctggggaatggaactgatttttctgtttctagctctgcatcaacggacaccgttacatcttcttcctcttctagcctttcagtgctgccttcatctctttcagtttttcaaaatcccacagatgtgtcacggagcaaccccaagtcaccacaaaaacctatcgttagagtcttcctgcccaataaacagaggacagtggtacctgcacggtgtggagtcacagtccgggacagcctgaagaaggcactgatgatgagaggtctaatcccagagtgctgtgctgtttacagaattcaggatggggagaagaaaccaattggctgggacactgatatttcctggcttactggagaggagttgcatgtagaagtgttggagaatgttccacttacaacacacaactttgtacggaaaacttttttcaccttagcattttgtgacttctgtagaaagctgcttttccagggattccgctgtcaaacatgtggttataaatttcaccagcgttgtagtacagaggttccactgatgtgtgttaattatgaccaactagatttgctgtttgtctccaagttctttgaacaccacccaataccacaggaggaggcctccttagcagagactacccttccatgtggctcatccccttctgcacccccctccgattctattgggcccccaattctcaccagtccatctccttcaaaatccattccaattccacagcctttccgaccagcagatgaagatcatcgaaatcagtttggacaacgagaccggtcctcatcagctccaaatgtgcatataaacacaatagaacccgtcaatattgatgacttgattagagaccaagggtttcgtagtgatggaggatcaaccacaggtttatccgccacaccccctgcctcattacctggctcactctctaatgtgaaagcattgcagaaatctccaggacctcagcgagaaagaaagtcctcttcatcctcagaagacaggaatcgaatgaaaacgcttggtagacgggattcaagtgacgattgggagattcctgatggacagatcacagtgggacaaagaattggatcagggtcatttgggacagtctacaagggaaagtggcatggtgatgtggcagtgaaaatgttgaatgtgacagcacccacacctcagcagttacaggccttcaaaaatgaagtaggagtactcaggaaaacgcgacatgtgaatatcctcctcttcatgggttattcaacaaagccacaactggctattgttacccagtggtgtgagggctccagtttatatcatcatctccacatcattgagaccaaattcgagatgatcaaacttatagatattgcacggcagactgcacagggcatggattacttacacgccaagtcaatcatccacagagacctcaagagtaataatatttttcttcatgaagacctcacagtaaaaataggtgattttggtctagccacagtgaaatctcgatggagtgggtcccatcagtttgaacagttgtctggatccattttgtggatggcaccagaagtaatcagaatgcaagataaaaacccatatagctttcagtcagatgtatatgcatttgggattgttctgtatgaattgatgaccggacagttaccttattcaaatatcaacaacagggaccaggtgctttgtcctccatgggagtgtaataaatgctgtgcaagggcttacttcccatgagagaagtgagtgaccaacagaaggataatttttatggtgggacgaggatatctgtctccagatctcagtaaggtacggagtaactgtccaa

SEQ ID NO: 34 - protein, 681 aa, Bos taurus
MAALSGGGGGGGGGAEQGQALFNGDMEPEAGAAASSAADPAIPEEVWNIKQMIKLTQEHIEALLDKFGGEHNPPSIYLEAYEEYTSKLDALQQREQQLLESLGNGTDFSVSSSASTDTVTSSSSSSLSVLPSSLSVFQNPTDVSRSNPKSPQKPIVRVFLPNKQRTVVPARCGVTVRDSLKKALMMRGLIPECCAVYRIQDGEKKPIGWDTDISWLTGEELHVEVLENVPLTTHNFVRKTFFTLAFCDFCRKLLFQGFRCQTCGYKFHQRCSTEVPLMCVNYDQLDLLFVSKFFEHHPIPQEEASLAETTLPCGSSPSAPPSDSIGPPILTSPSPSKSIPIPQPFRPADEDHRNQFGQRDRSSSAPNVHINTIEPVNIDDLIRDQGFRSDGGSTTGLSATPPASLPGSLSNVKALQKSPGPQRERKSSSSSEDRNRMKTLGRRDSSDDWEIPDGQITVGQRIGSGSFGTVYKGKWHGDVAVKMLNVTAPTPQQLQAFKNEVGVLRKTRHVNILLFMGYSTKPQLAIVTQWCEGSSLYHHLHIIETKFEMIKLIDIARQTAQGMDYLHAKSIIHRDLKSNNIFLHEDLTVKIGDFGLATVKSRWSGSHQFEQLSGSILWMAPEVIRMQDKNPYSFQSDVYAFGIVLYELMTGQLPYSNINNRDQVLCPPWECNKCCARAYFP

SEQ ID NO: 35 - DNA, 2319 bp, Bos taurus
ctcagctgcgccgggtctcacaagacggttcccgaggtggcccaggcgccgtcccaccgccgacgccgcccgggccgcccgggccgtccctccccgctgccccccgtcctccgcctccgcctccccccgccctcagcctcccttccccctccccgcccagcagcggtcgctcgggcccggctctcggttataagatggcggcgctgagtggcggcggcggcggcggcggcggtggcgcggagcagggccaggctctgttcaacggggacatggagcccgaggccggcgccgcggcctcttcggctgcggaccccgccattcccgaggaggtgtggaatatcaaacaaatgattaagttgacacaggagcatatagaggccctattggacaaatttggtggggagcataatccaccatcaatatatctggaggcctatgaagaatacaccagcaagctagatgccctccaacaaagagaacaacagttattggaatccctggggaatggaactgatttttctgtttctagctctgcatcaacggacaccgttacatcttcttcctcttctagcctttcagtgctgccttcatctctttcagtttttcaaaatcccacagatgtgtcacggagcaaccccaagtcaccacaaaaacctatcgttagagtcttcctgcccaataaacagaggacagtggtacctgcacggtgtggagtcacagtccgggacagcctgaagaaggcactgatgatgagaggtctaatcccagagtgctgtgctgtttacagaattcaggatggggagaagaaaccaattggctgggacactgatatttcctggcttactggagaggagttgcatgtagaagtgttggagaatgttccacttacaacacacaactttgtacggaaaacttttttcaccttagcattttgtgacttctgtagaaagctgcttttccagggattccgctgtcaaacatgtggttataaatttcaccagcgttgtagtacagaggttccactgatgtgtgttaattatgaccaactagatttgctgtttgtctccaagttctttgaacaccacccaataccacaggaggaggcctccttagcagagactacccttccatgtggctcatccccttctgcacccccctccgattctattgggcccccaattctcaccagtccatctccttcaaaatccattccaattccacagcctttccgaccagcagatgaagatcatcgaaatcagtttggacaacgagaccggtcctcatcagctccaaatgtgcatataaacacaatagaacccgtcaatattgatgacttgattagagaccaagggtttcgtagtgatggaggatcaaccacaggtttatccgccacaccccctgcctcattacctggctcactctctaatgtgaaagcattgcagaaatctccaggacctcagcgagaaagaaagtcctcttcatcctcagaagacaggaatcgaatgaaaacgcttggtagacgggattcaagtgacgattgggagattcctgatggacagatcacagtgggacaaagaattggatcagggtcatttgggacagtctacaagggaaagtggcatggtgatgtggcagtgaaaatgttgaatgtgacagcacccacacctcagcagttacaggccttcaaaaatgaagtaggagtactcaggaaaacgcgacatgtgaatatcctcctcttcatgggttattcaacaaagccacaactggctattgttacccagtggtgtgagggctccagtttatatcatcatctccacatcattgagaccaaattcgagatgatcaaacttatagatattgcacggcagactgcacagggcatggattacttacacgccaagtcaatcatccacagagacctcaagagtaataatatttttcttcatgaagacctcacagtaaaaataggtgattttggtctagccacagtgaaatctcgatggagtgggtcccatcagtttgaacagttgtctggatccattttgtggatggcaccagaagtaatcagaatgcaagataaaaacccatatagctttcagtcagatgtatatgcatttgggattgttctgtatgaattgatgaccggacagttaccttattcaaatatcaacaacagggaccaggtgctttgtcctccatgggagtgtaataaatgctgtgcaagggcttacttcccatgagagaagtgagtgaccaacagaaggtctgtgcaaggaaaagagacaaagccacggatcagaagcacatggccataactga

SEQ ID NO: 36 - protein, 681 aa, Bos taurus; identical to SEQ ID NO: 34

SEQ ID NO: 37 - DNA, 2661 bp, Bos taurus
tcagctgcgccgggtctcacaagacggttcccgaggtggcccaggcgccgtcccaccgccgacgccgcccgggccgcccgggccgtccctccccgctgccccccgtcctccgcctccgcctccccccgccctcagcctcccttccccctccccgcccagcagcggtcgctcgggcccggctctcggttataagatggcggcgctgagtggcggcggcggcggcggcggcggtggcgcggagcagggccaggctctgttcaacggggacatggagcccgaggccggcgccgcggcctcttcggctgcggaccccgccattcccgaggaggtgtggaatatcaaacaaatgattaagttgacacaggagcatatagaggccctattggacaaatttggtggggagcataatccaccatcaatatatctggaggcctatgaagaatacaccagcaagctagatgccctccaacaaagagaacaacagttattggaatccctggggaatggaactgatttttctgtttctagctctgcatcaacggacaccgttacatcttcttcctcttctagcctttcagtgctgccttcatctctttcagtttttcaaaatcccacagatgtgtcacggagcaaccccaagtcaccacaaaaacctatcgttagagtcttcctgcccaataaacagaggacagtggtacctgcacggtgtggagtcacagtccgggacagcctgaagaaggcactgatgatgagaggtctaatcccagagtgctgtgctgtttacagaattcaggatggggagaagaaaccaattggctgggacactgatatttcctggcttactggagaggagttgcatgtagaagtgttggagaatgttccacttacaacacacaactttgtacggaaaacttttttcaccttagcattttgtgacttctgtagaaagctgcttttccagggattccgctgtcaaacatgtggttataaatttcaccagcgttgtagtacagaggttccactgatgtgtgttaattatgaccaactagatttgctgtttgtctccaagttctttgaacaccacccaataccacaggaggaggcctccttagcagagactacccttccatgtggctcatccccttctgcacccccctccgattctattgggcccccaattctcaccagtccatctccttcaaaatccattccaattccacagcctttccgaccagcagatgaagatcatcgaaatcagtttggacaacgagaccggtcctcatcagctccaaatgtgcatataaacacaatagaacccgtcaatattgatgacttgattagagaccaagggtttcgtagtgatggaggatcaaccacaggtttatccgccacaccccctgcctcattacctggctcactctctaatgtgaaagcattgcagaaatctccaggacctcagcgagaaagaaagtcctcttcatcctcagaagacaggaatcgaatgaaaacgcttggtagacgggattcaagtgacgattgggagattcctgatggacagatcacagtgggacaaagaattggatcagggtcatttgggacagtctacaagggaaagtggcatggtgatgtggcagtgaaaatgttgaatgtgacagcacccacacctcagcagttacaggccttcaaaaatgaagtaggagtactcaggaaaacgcgacatgtgaatatcctcctcttcatgggttattcaacaaagccacaactggctattgttacccagtggtgtgagggctccagtttatatcatcatctccacatcattgagaccaaattcgagatgatcaaacttatagatattgcacggcagactgcacagggcatggattacttacacgccaagtcaatcatccacagagacctcaagagtaataatatttttcttcatgaagacctcacagtaaaaataggtgattttggtctagccacagtgaaatctcgatggagtgggtcccatcagtttgaacagttgtctggatccattttgtggatggcaccagaagtaatcagaatgcaagataaaaacccatatagctttcagtcagatgtatatgcatttgggattgttctgtatgaattgatgaccggacagttaccttattcaaatatcaacaacagggaccagtctgtgcaaggaaaagagacaaagccacggatcagaagcacatggccataactgaagattttgtgaactctcacaaggaaaaaatttgctctttgaacaataagaaggaactcactaaaatgtaactgagaactgttcaacaggttgaaagctgaaagatgccattggaactgacaaaatgtttcttaaacataaatgatgaaacagtgaaactacataatatctcctctggctgaaacattcaagaagtttaaaatgcttaagttaaaaataaaatcctagtaaacaatggacttactgtgcaacatagagaatatcttacgataacctgtaatggaaaagaatctgaaaaagaatgtatataactgaatcactttgctgtaaactagaatctgacacaacactgtaaatcactacacttttctgttgcatgccaaagattatttaataacgtcattaaaaaattattttaataatta

SEQ ID NO: 38 - protein, 679 aa, Bos taurus
MAALSGGGGGGGGGAEQGQALFNGDMEPEAGAAASSAADPAIPEEVWNIKQMIKLTQEHIEALLDKFGGEHNPPSIYLEAYEEYTSKLDALQQREQQLLESLGNGTDFSVSSSASTDTVTSSSSSSLSVLPSSLSVFQNPTDVSRSNPKSPQKPIVRVFLPNKQRTVVPARCGVTVRDSLKKALMMRGLIPECCAVYRIQDGEKKPIGWDTDISWLTGEELHVEVLENVPLTTHNFVRKTFFTLAFCDFCRKLLFQGFRCQTCGYKFHQRCSTEVPLMCVNYDQLDLLFVSKFFEHHPIPQEEASLAETTLPCGSSPSAPPSDSIGPPILTSPSPSKSIPIPQPFRPADEDHRNQFGQRDRSSSAPNVHINTIEPVNIDDLIRDQGFRSDGGSTTGLSATPPASLPGSLSNVKALQKSPGPQRERKSSSSSEDRNRMKTLGRRDSSDDWEIPDGQITVGQRIGSGSFGTVYKGKWHGDVAVKMLNVTAPTPQQLQAFKNEVGVLRKTRHVNILLFMGYSTKPQLAIVTQWCEGSSLYHHLHIIETKFEMIKLIDIARQTAQGMDYLHAKSIIHRDLKSNNIFLHEDLTVKIGDFGLATVKSRWSGSHQFEQLSGSILWMAPEVIRMQDKNPYSFQSDVYAFGIVLYELMTGQLPYSNINNRDQSVQGKETKPRIRSTWP

SEQ ID NO: 39 - DNA, 7434 bp, Bos taurus
acaccgttacatcttcttcctcttctagcctttcagtgctgccttcatctctttcagtttttcaaaatcccacagatgtgtcacggagcaaccccaagtcaccacaaaaacctatcgttagagtcttcctgcccaataaacagaggacagtggtacctgcacggtgtggagtcacagtccgggacagcctgaagaaggcactgatgatgagaggtctaatcccagagtgctgtgctgtttacagaattcaggatggggagaagaaaccaattggctgggacactgatatttcctggcttactggagaggagttgcatgtagaagtgttggagaatgttccacttacaacacacaactttgtacggaaaacttttttcaccttagcattttgtgacttctgtagaaagctgcttttccagggattccgctgtcaaacatgtggttataaatttcaccagcgttgtagtacagaggttccactgatgtgtgttaattatgaccaactagatttgctgtttgtctccaagttctttgaacaccacccaataccacaggaggaggcctccttagcagagactacccttccatgtggctcatccccttctgcacccccctccgattctattgggcccccaattctcaccagtccatctccttcaaaatccattccaattccacagcctttccgaccagcagatgaagatcatcgaaatcagtttggacaacgagaccggtcctcatcagctccaaatgtgcatataaacacaatagaacccgtcaatattgatgacttgattagagaccaagggtttcgtagtgatggaggatcaaccacaggtttatccgccacaccccctgcctcattacctggctcactctctaatgtgaaagcattgcagaaatctccaggacctcagcgagaaagaaagtcctcttcatcctcagaagacaggaatcgaatgaaaacgcttggtagacgggattcaagtgacgattgggagattcctgatggacagatcacagtgggacaaagaattggatcagggtcatttgggacagtctacaagggaaagtggcatggtgatgtggcagtgaaaatgttgaatgtgacagcacccacacctcagcagttacaggccttcaaaaatgaagtaggagtactcaggaaaacgcgacatgtgaatatcctcctcttcatgggttattcaacaaagccacaactggctattgttacccagtggtgtgagggctccagtttatatcatcatctccacatcattgagaccaaattcgagatgatcaaacttatagatattgcacggcagactgcacagggcatggattacttacacgccaagtcaatcatccacagagacctcaagagtaataatatttttcttcatgaagacctcacagtaaaaataggtgattttggtctagccacagtgaaatctcgatggagtgggtcccatcagtttgaacagttgtctggatccattttgtggatggcaccagaagtaatcagaatgcaagataaaaacccatatagctttcagtcagatgtatatgcatttgggattgttctgtatgaattgatgaccggacagttaccttattcaaatatcaacaacagggaccagataatttttatggtgggacgaggatatctgtctccagatctcagtaaggtacggagtaactgtccaaaagccatgaagagattaatggcagagtgcctaaaaaagaaaagagatgaaagaccactctttccccaagtaggaaagactctcctaagcaagagacaaaattcagaagttatcagggaaaaagataagcagattctcgcctctattgagctgctggcccgctcattgccaaaaattcaccgcagtgcatcagaaccctccttgaatcgggctggcttccaaacagaggattttagtctatatgcttgtgcttctccaaaaacacccattcaggcagggggatatggagaatttgcagccttcaagtagccacaccatcatgacagcatctactcttatttcttaagtcttgtgttcgtacaatttgttaacatcaaaacacagttctgttcctcaactctttttaaagttaaaatttttcagtgcataagctggtgtggaacagaaggaaatttcccatccaacaaaagagggaagaatgttttaggaaccagaattctctgctgccagtgtttcttcttcaacacaaatatcacaagtctgcccactcccaggaagaaagaggagagaccctgagttctgaccttttgatggtcaggcatgatggaaagaaactgctgctacagcttgggagatttgctctgggaagtctgccagtcaactttgcccttctaaccaccagatcaatatgtggctgatcatctgatggggcagttgcaatcaccaagccttgttctctttcctgttctgggattgtgttgtggaacccttttccctagccaccaccagttcatttctgagggatggaacaaaaatgcagcatgcccttcctgtgtggtgcatgttcagtccttgacaaatttttaccaaaatgaagctactttatttaaaaggagggtgagaggtgaggaggtcactttgggtgtggcggaaagggaatgctgcatctttttcctgggctgctggggctctggccttggcttgccagccggaagcgctggcacgcatcgccttcttttcccattgggtccagcaatgaagacgagtgtttggggttttttttttctccaccatgtagcaagttctcaggaaaatacaattgatatcttcctcctaagctcttccaatcagtcaccaagtacttatgtggttactttgtccagggcacaaaatgcctgtatctaattaaaagcctacaaaactgcttgataacagttttgaatgtgagacatttatgtaatttaaatgtaaggtacaagttttaatttctgagtttcttctattatatttttattaaaaaaagaaaataattttcagattgaattggagtaaaataatattacttcccactagaattatatatcctggaaaattgtatttttgttacataagcagcttttaaagaaagatcattacccttttctctacataaatatatggggagtcttagcctaatgacaaatatttataatttttaaattaatggtacttgctggatccatactaacatctttactaatacctcattgtttcttccaacttactcctacactacatcctacatcttcttcctagtcttttatctagaatatgcaacctcaaataaaaatggtggtgtcctcattcattctcctccttccttttttcccaagcctgatcttcaaaaggttggttaatttggcagctgagttcctccccaggcagagaatagaccaattttaggtgtattgggactgagggaggatgtgtaaagattaacatcagtaaagaaccgctgtggagtaattaagaactttgttctttataactggagaatataacctaaccctaacatccctcagcctttactaaagtgtggcgtaaatcacagtagtagcaaagaaagtgactctggatgtgttcctggccagtacctcccttatcatgaatgtagactctctcatcaagatttaggaatataaatcaaatcaaatgtgcccagccaagctatgtagtaagggacttgaacaatattaggcagaacctataaaataaatcagggaattagaaattatttaaagttttcaaattgtaaattgccccggtgtctttcagcctactgccattatttttgctacaatacctacatttcagaggagggcctactgaaaattccatgcaagtggaaaataatcctcaagttattaatgagtttgaaaagcaatgagttcttaagtctttgtgagtagagcaagatcctacaaaattcagaaatagtaaaaatggattcatgctgatttgaagagcatctgtgtgcataatataatgctgcatctcttttaaaagcagtctatttttctttttaaatttgtccccatagatgcttttgaacatgaacatgcttatgttaccttttccgaggttgggaagagccaggagctctcaggcagggccccctccctcagctgggcaggagctgctcaggaggagctagttatagaggaagcttagcgttggcattttcaaaattcaaggtgataacgctttcttcttcctttctgttttagaatagattgctgtctgatttgaaaaagggaaatagatttgatctcaaatgaatctgtgcccagaagccaggctcagggtattcagagatttgtatagtgccctcaaaaaataacaaaattttagctttccttttttcttcttttctccatcaaattcttttttctctagtttacaaatgacatggaaaaggaatttcccctgagttttgtatgcctttttttttttggcttagactatagataggcgtgttgagctcctaagaaaatacaaggaggaactctttgttgtgcagagcactttatgagtagtttgtgtggataatatgtgactgcttccctgacgagcttgtgaggctgtacttatgtctttcctgtaaggcagcttcagtgccttctgtagtgtatataaggaaagattacgccttctgaaaaatctcagagcaaccataagattattttaaaatatgtagtatgactgatggactttttcatcattaaattagtctagcatctaaacttttaccactgaaataatattgaccaaaaagcaatttataaaaggtatttgtgaatagaaaatacaatgtgatcatttgtacttatgtgcaccttaaaagaggaattctgtctagctgtcaaattctggttccttaacatccagtccttgattgtgattgagatctggtaggacgtgctggggcacgctagcagataaaatcccgtatactttaggatagatgttacatttatgtcagtgttggcaaagagcattgtgtagtaataaagaattcaagacttcagcaatgtcaacctgaaactttgtaaatatttcctagattgttatttgatgcagtcacagctctttatcacacaatgttgtctttccctcatcaggcaattttagaactgctgcacacccctcctcagatctcacctgcccctcctgtacattcacctctccagccttgtgcacacctcatttagctttagtttgaaacacattgcagggttcaggtgacctcttcaaaaactacctcctcagaatgaggtaatgaatagttatttattttaaaatatgaaaagtcaggagctctagaatatgaagatgatctaagattttaacttttatgtatacttgttgagcactctccttttgtcctaaagggcattatacatttaagcagtaatactgaaaaatgtagctcagagtaactgaatgttgttgaaagtggtgccagaatctgttttaggggtacgtatcagaatcttaatcttaaatcggttacatgaaattaaatagttaatggtaacacttgactaacagatataattttaattttcggtaggcttttagcaagacagtaagtacatcttcataatgagttagccacagcttcatcacatgcacagattttcctgttgagagactgcccagttaagagggtagaatgatgaaccatttttcaggattctcttctttgtccaaactggcattgtgagtgctagaatatcagcactttcaaactagtgattccaactattaggctattaaaaagcaaaacaaaccaaacaaaccatagccagacatgggaagtttactatgagtataaacagcaaatagcttacaggtcatacattgaaatggtgtaggtaaggcgttagaaaaataccttgacaatttgccaaatgatcttactgtgccttcatgatgcaataaaaaaaaaaaaaatttagcataaatcagtgatttgtgaagagagcagccaccctggtctaactcagctgtgttaatattttttagcgtgcaatttagactgcaaagataaatgcactaaagagtttatagccaaaatcacatttaaaaaatgagagaaaacacaggtaaattttcagtgaacaaaattatttttttaaagtacataatccctagtatagtcagatatatttatcacatagagcaaataggttgaaatcacaattcagtgacatttctagagaaactttttctactcccataggttcttcaaagcatggaacttttatataacagaaatgtgtgacggtcattttaaattgctgtagtttggggctgaagtactgtgtgctgggcagcaatcacatgtattaactagtgagaaaggagaaattaagatataggacagaatttgattttcttgttcccagattactgctgccaacctagacactgagtttccagaggctgaaacgtaaacttgcagctcagcaactgttttgcaaagttagtgggactgtcctgcttatgctgttcaaaaatgctctgagggccaggtggggcctccaggggctcctctctgaggggacatcagactagctaacgacctggcgggcggatgtgaaccggacacactccatggtgtgcttcttgtatcggtccctcgccaccctcaagaaaggcttcagcgggttctctagacgtctccactaaggtgtgttactaacagccatgggttgttgagcacccgaggagtgcaatagcatctctgcatgattgtatattggcccgaagagaatgaagtggccagtgtactcatgttccatgttgctagctctggtaaactgaaaatactggtaagatttttgttttatcagtacactagagagtaagctttgttttgttgtttttagataatgttttcacttccatttggaaagacatttaaattgagtttcagtcctaaattttgccagtcatggtaattagcagtttctatcaggtatttttaaggtagaagaggatagaaacataagttctaaaagcttaaggtaaccgtggtttattttaaaatgtttaggggtggttagtctctacctcaaaaaaagtgagtgaatcttttatttcagcattcacaagttcggctgttgtttttgtaatacattttttttttaaccttttgacccccctttacctaagtgtcaatgtagttttattaattactaagtcagtttcattaaaatgtttatttagcagttttgactaattgcaatgattaatatagccagttgtgcatgaggacacagccagtgagtatatctgggttttttttgtgatgctttttttcttaagacttctgtagatttatgaagtactcattgaaaacaactaaaatacgtttattcgtgttaatatggaaaaaaaaaaa

SEQ ID NO: 40 - protein, 603 aa, Bos taurus
MMRGLIPECCAVYRIQDGEKKPIGWDTDISWLTGEELHVEVLENVPLTTHNFVRKTFFTLAFCDFCRKLLFQGFRCQTCGYKFHQRCSTEVPLMCVNYDQLDLLFVSKFFEHHPIPQEEASLAETTLPCGSSPSAPPSDSIGPPILTSPSPSKSIPIPQPFRPADEDHRNQFGQRDRSSSAPNVHINTIEPVNIDDLIRDQGFRSDGGSTTGLSATPPASLPGSLSNVKALQKSPGPQRERKSSSSSEDRNRMKTLGRRDSSDDWEIPDGQITVGQRIGSGSFGTVYKGKWHGDVAVKMLNVTAPTPQQLQAFKNEVGVLRKTRHVNILLFMGYSTKPQLAIVTQWCEGSSLYHHLHIIETKFEMIKLIDIARQTAQGMDYLHAKSIIHRDLKSNNIFLHEDLTVKIGDFGLATVKSRWSGSHQFEQLSGSILWMAPEVIRMQDKNPYSFQSDVYAFGIVLYELMTGQLPYSNINNRDQIIFMVGRGYLSPDLSKVRSNCPKAMKRLMAECLKKKRDERPLFPQVGKTLLSKRQNSEVIREKDKQILASIELLARSLPKIHRSASEPSLNRAGFQTEDFSLYACASPKTPIQAGGYGEFAAFK

SEQ ID NO: 41 - DNA, 2295 bp, Equus caballus
  misc_feature (79)..(79): n is a, c, g, or t
atgaagacgctgagcggcggcggcggcggcgcggagcagggccaggctctgttcaacggggacatggaacccggaggcnccgcgccggcgcccgcggcctcgtcggccgcggaccctgccattcccgaggaggtatggaatatcaaacaaatgattaaattgacacaggaacatatagaggccctattggacaaatttggtggggagcataatccaccatcaatatatctggaggcctatgaagaatacaccagcaagctagatgccctccaacaaagagaacaacagttattggaatccctggggaatggaactgatttttctgtttctagttctgcatcaacggacaccgttacatcttcttcctcttctagcctttcagtgctaccttcatctctttcagtttttcaaaatcccacagatgtgtcacggagcaaccctaagtcaccacaaaaacctatcgttagagtcttcctgcccaacaaacagaggacagtggtacctgcaaggtgtggcgttacagtccgggacagtctaaagaaagcactgatgatgagaggtctaatcccagagtgctgtgctgtttacagaattcaggatggagagaagaaaccaattggctgggacactgatatttcctggctcactggagaggaattgcatgtagaagtgttggagaatgttccacttacaacacacaactttgtacggaaaacttttttcaccttagcattttgtgacttttgtcgaaagctgcttttccagggtttccgctgtcaaacatgtggttataaatttcaccagcgttgtagtacagaggttccactgatgtgtgttaattatgaccaacttgatttgctgtttgtctccaagttctttgaacaccacccagtatcacaggaggaggcctccttagcagagactgcccttacatctggatcatccccttctgcacccccctccgattccattgggccccaaattctcaccagtccatctccttcaaaatccattccaattccacagcctttccgaccagcagatgaagatcatcgaaatcagtttggacaacgagaccggtcctcatcagctccaaatgtacatataaacacaatagaacctgtcaatattgatgacttgattagagaccaagggtttcgtagtgatggaggatcaaccacaggtttatctgccaccccccctgcctcattacctggctcactcactaatgtgaaggcattacagaaatctccaggacctcaacgggaaaggaaatcatcttcatcctcagaagacaggaatcgaatgaaaactcttggtagacgggattcaagtgacgattgggagattcctgatgggcagatcacagtgggacaaagaattggatctgggtcatttgggacagtctacaagggaaagtggcatggtgatgtggcagtgaaaatgttgaatgtgacagcacccacacctcagcagttacaggccttcaaaaatgaagtaggagtactcaggaaaactcgacatgtgaatatcctactcttcatgggctattcaacaaagccacaactggctattgttacccagtggtgtgagggctccagcttatatcaccatctccacatcattgagaccaaatttgagatgatcaaacttatagatattgctcggcaaactgcacagggcatggattacttacacgccaagtcaatcatccacagagacctcaagagtaataatatttttcttcatgaagacctcacagtaaaaataggtgattttggtctagccacagtgaaatctcgatggagtgggtcccatcagtttgaacagttgtctggatccattttgtggatggcaccagaagtaatcagaatgcaagataaaaacccgtatagctttcaatcagatgtatatgcctttgggattgttctgtatgaattgatgactggacagttaccttattcaaacatcaacaacagggaccagataatttttatggtgggaagaggatatctatctccagatctcagtaaggtacggagtaactgtccaaaagccatgaagagattaatggcagagtgcctaaaaaagaaaagagacgagagaccactcttcccccaaattctcgcctctattgagctgctggcccgctcattgccaaaaattcaccgcagtgcatcagagccctccttgaatcgggctggcttccagacagaggattttagtctatatgcttgtgcttctccgaaaacacccatccaggcagggggatatggtgcgtttcctgtccactga

SEQ ID NO: 42 - protein, 764 aa, Equus caballus
  misc_feature (27)..(27): Xaa can be any naturally occurring amino acid
MKTLSGGGGGAEQGQALFNGDMEPGGXAPAPAASSAADPAIPEEVWNIKQMIKLTQEHIEALLDKFGGEHNPPSIYLEAYEEYTSKLDALQQREQQLLESLGNGTDFSVSSSASTDTVTSSSSSSLSVLPSSLSVFQNPTDVSRSNPKSPQKPIVRVFLPNKQRTVVPARCGVTVRDSLKKALMMRGLIPECCAVYRIQDGEKKPIGWDTDISWLTGEELHVEVLENVPLTTHNFVRKTFFTLAFCDFCRKLLFQGFRCQTCGYKFHQRCSTEVPLMCVNYDQLDLLFVSKFFEHHPVSQEEASLAETALTSGSSPSAPPSDSIGPQILTSPSPSKSIPIPQPFRPADEDHRNQFGQRDRSSSAPNVHINTIEPVNIDDLIRDQGFRSDGGSTTGLSATPPASLPGSLTNVKALQKSPGPQRERKSSSSSEDRNRMKTLGRRDSSDDWEIPDGQITVGQRIGSGSFGTVYKGKWHGDVAVKMLNVTAPTPQQLQAFKNEVGVLRKTRHVNILLFMGYSTKPQLAIVTQWCEGSSLYHHLHIIETKFEMIKLIDIARQTAQGMDYLHAKSIIHRDLKSNNIFLHEDLTVKIGDFGLATVKSRWSGSHQFEQLSGSILWMAPEVIRMQDKNPYSFQSDVYAFGIVLYELMTGQLPYSNINNRDQIIFMVGRGYLSPDLSKVRSNCPKAMKRLMAECLKKKRDERPLFPQILASIELLARSLPKIHRSASEPSLNRAGFQTEDFSLYACASPKTPIQAGGYGAFPVH

SEQ ID NO: 43 - DNA, 2678 bp, Gallus gallus
tccccctccctcgccccagcgcttcgatccaagatggcggcgctgagcagcggcagcagcgccgagggggcctcgctcttcaacggggacatggagcccgagccgccgccgcccgtgctgggcgcctgctacgccgggagcggcggcggcgacccggccatcccggaggaggtgtggaatatcaaacagatgattaaattaacacaagaacatatagaagcgctgttagacaagtttggaggagagcataacccaccatcaatatatttagaggcctatgaggagtacaccagcaaactagatgctctacagcagagagaacagcagttattggaatccatgggaaatggaactgatttctctgtttccagttcagcttcaacggacacagttgcatcatcttcctcctctagcctctctgtagcaccttcatccctttcagtttatcaaaatcctactgatatgtcgcggaataaccctaagtctccacagaagcctattgttagagtcttcctgcccaacaagcaaaggactgtggttccggcaagatgtggggtgacagtccgagacagcctgaagaaagctctgatgatgagaggtcttattccagaatgctgtgctgtttacagaatacaggatggagagaagaagccaattggctgggacactgacatttcctggctaaccggagaggagttacacgtggaggtcttggagaatgtgccactcacaacacacaattttgtacgaaaaacattcttcacgttagcgttctgcgacttctgtcgaaagctgcttttccagggattccgatgccagacatgtggctacaaatttcaccagcgctgtagcacagaagtgccactgatgtgtgttaactacgaccaactcgatttgctgtttgtctccaagttctttgaacatcaccccatatcgcaggaggagaccaccttaggagagaccaccccggcatcgggatcgtacccctcagtgcccccatcagattctgttggaccaccaattctccctagtccttctccttcaaaatccattccaatcccacagcccttccgaccagcagatgaagaccatcggaatcagtttgggcaacgcgaccgatcctcttcagctcccaatgttcacatcaatacaattgagccagtcaatattgatgacttgattagagaccagggtgtacgaggagagggagcccctttgaaccagctgatgcgctgtcttcggaaataccaatcccggactcccagtcccctccttcattctgtccccagtgaaatagtgtttgattttgagcctggcccagtgttcagaggttcaactgcaggtttgtctgcaacacctcctgcatctttgcctgggtcacttaccaatgtgaaagcattacagaaatcaccaggcccccaacgggaaaggaaatcatcctcatcctcagaagacagaaataggatgaaaacccttggtcgacgagattcaagtgatgattgggaaataccagatgggcagatcacagttggacaaaggataggatctggatcatttggaacagtctacaaaggaaagtggcatggtgacgtggcagtgaaaatgttgaatgttacagcacccacacctcaacagttacaggctttcaaaaatgaagtaggagtgctcaggaaaacacggcatgtgaatatcctactttttatgggttattcaacaaaacctcagttggctattgttacacagtggtgtgaggggtccagcttatatcaccatctgcacataattgagaccaagtttgaaatgatcaaactaattgatattgcacgacagactgcacaaggcatggattatttgcatgccaagtcaatcatccacagagacctcaagagtaataatatttttcttcatgaagacctcacagtaaaaataggtgacttcggtctggctacagtgaaatcacgatggagtggatctcatcaatttgaacagttatctggatcaattctatggatggcaccggaagtgatcaggatgcaagacaaaaacccatatagctttcagtcagatgtgtatgcattcgggattgtgctttatgaactgatgactggacagttaccatactcaaacatcaacaacagggaccagataatttttatggtgggacgaggatatctatctccagacctcagtaaagtaagaagtaactgtccaaaagctatgaagagactaatggcagaatgcttgaaaaagaaaagagatgagagacctctttttccacagattcttgcctccattgagcttctggcccggtcgttgccaaaaattcaccgcagtgcatctgagccgtcactaaaccgggctggcttccagaccgaggatttcagtctgtatgcttgtgcttctccaaaaacgcccatccaagcagggggatacggtgggtttccagtacactgaaaagaaatgtgaaagcgtgtgcctgtttgctcatgtgctggtgtgttcctgtgtgtgcaacgcatacgtacgttctcagttcctaccagcgactttttaaggtttactgagggaatgaagactcatttcctaacatggggcattgaacgtcctgagcacaagtcagtgctggtaaggaatgtcttgggaacagctggcaagaagaattagaaggtacttaaagg

SEQ ID NO: 44 - protein, 806 aa, Gallus gallus
MAALSSGSSAEGASLFNGDMEPEPPPPVLGACYAGSGGGDPAIPEEVWNIKQMIKLTQEHIEALLDKFGGEHNPPSIYLEAYEEYTSKLDALQQREQQLLESMGNGTDFSVSSSASTDTVASSSSSSLSVAPSSLSVYQNPTDMSRNNPKSPQKPIVRVFLPNKQRTVVPARCGVTVRDSLKKALMMRGLIPECCAVYRIQDGEKKPIGWDTDISWLTGEELHVEVLENVPLTTHNFVRKTFFTLAFCDFCRKLLFQGFRCQTCGYKFHQRCSTEVPLMCVNYDQLDLLFVSKFFEHHPISQEETTLGETTPASGSYPSVPPSDSVGPPILPSPSPSKSIPIPQPFRPADEDHRNQFGQRDRSSSAPNVHINTIEPVNIDDLIRDQGVRGEGAPLNQLMRCLRKYQSRTPSPLLHSVPSEIVFDFEPGPVFRGSTAGLSATPPASLPGSLTNVKALQKSPGPQRERKSSSSSEDRNRMKTLGRRDSSDDWEIPDGQITVGQRIGSGSFGTVYKGKWHGDVAVKMLNVTAPTPQQLQAFKNEVGVLRKTRHVNILLFMGYSTKPQLAIVTQWCEGSSLYHHLHIIETKFEMIKLIDIARQTAQGMDYLHAKSIIHRDLKSNNIFLHEDLTVKIGDFGLATVKSRWSGSHQFEQLSGSILWMAPEVIRMQDKNPYSFQSDVYAFGIVLYELMTGQLPYSNINNRDQIIFMVGRGYLSPDLSKVRSNCPKAMKRLMAECLKKKRDERPLFPQILASIELLARSLPKIHRSASEPSLNRAGFQTEDFSLYACASPKTPIQAGGYGGFPVH

SEQ ID NO: 45 - DNA, 4454 bp, Homo sapiens
gaaacgtcccgtgtgggaggggcgggtctgggtgcggcctgccgcatgactcgtggttcggaggcccacgtggccggggcggggactcaggcgcctggggcgccgactgattacgtagcgggcggggccggaagtgccgctccttggtgggggctgttcatggcggttccggggtctccaacatttttcccggctgtggtcctaaatctgtccaaagcagaggcagtggagcttgaggttcttgctggtgtgaaatgactgagtacaaactggtggtggttggagcaggtggtgttgggaaaagcgcactgacaatccagctaatccagaaccactttgtagatgaatatgatcccaccatagaggattcttacagaaaacaagtggttatagatggtgaaacctgtttgttggacatactggatacagctggacaagaagagtacagtgccatgagagaccaatacatgaggacaggcgaaggcttcctctgtgtatttgccatcaataatagcaagtcatttgcggatattaacctctacagggagcagattaagcgagtaaaagactcggatgatgtacctatggtgctagtgggaaacaagtgtgatttgccaacaaggacagttgatacaaaacaagcccacgaactggccaagagttacgggattccattcattgaaacctcagccaagaccagacagggtgttgaagatgctttttacacactggtaagagaaatacgccagtaccgaatgaaaaaactcaacagcagtgatgatgggactcagggttgtatgggattgccatgtgtggtgatgtaacaagatacttttaaagttttgtcagaaaagagccactttcaagctgcactgacaccctggtcctgacttccctggaggagaagtattcctgttgctgtcttcagtctcacagagaagctcctgctacttccccagctctcagtagtttagtacaataatctctatttgagaagttctcagaataactacctcctcacttggctgtctgaccagagaatgcacctcttgttactccctgttatttttctgccctgggttcttccacagcacaaacacacctctgccaccccaggtttttcatctgaaaagcagttcatgtctgaaacagagaaccaaaccgcaaacgtgaaattctattgaaaacagtgtcttgagctctaaagtagcaactgctggtgattttttttttctttttactgttgaacttagaactatgctaatttttggagaaatgtcataaattactgttttgccaagaatatagttattattgctgtttggtttgtttataatgttatcggctctattctctaaactggcatctgctctagattcataaatacaaaaatgaatactgaattttgagtctatcctagtcttcacaactttgacgtaattaaatccaactttcacagtgaagtgcctttttcctagaagtggtttgtagacttcctttataatatttcagtggaatagatgtctcaaaaatccttatgcatgaaatgaatgtctgagatacgtctgtgacttatctaccattgaaggaaagctatatctatttgagagcagatgccattttgtacatgtatgaaattggttttccagaggcctgttttggggctttcccaggagaaagatgaaactgaaagcacatgaataatttcacttaataatttttacctaatctccacttttttcataggttactacctatacaatgtatgtaatttgtttcccctagcttactgataaacctaatattcaatgaacttccatttgtattcaaatttgtgtcataccagaaagctctacatttgcagatgttcaaatattgtaaaactttggtgcattgttatttaatagctgtgatcagtgattttcaaacctcaaatatagtatattaacaaattacattttcactgtatatcatggtatcttaatgatgtatataattgccttcaatccccttctcaccccaccctctacagcttcccccacagcaataggggcttgattatttcagttgagtaaagcatggtgctaatggaccagggtcacagtttcaaaacttgaacaatccagttagcatcacagagaaagaaattcttctgcatttgctcattgcaccagtaactccagctagtaattttgctaggtagctgcagttagccctgcaaggaaagaagaggtcagttagcacaaaccctttaccatgactggaaaactcagtatcacgtatttaaacatttttttttcttttagccatgtagaaactctaaattaagccaatattctcatttgagaatgaggatgtctcagctgagaaacgttttaaattctctttattcataatgttctttgaagggtttaaaacaagatgttgataaatctaagctgatgagtttgctcaaaacaggaagttgaaattgttgagacaggaatggaaaatataattaattgatacctatgaggatttggaggcttggcattttaatttgcagataataccctggtaattctcatgaaaaatagacttggataacttttgataaaagactaattccaaaatggccactttgttcctgtctttaatatctaaatacttactgaggtcctccatcttctatattatgaattttcatttattaagcaaatgtcatattaccttgaaattcagaagagaagaaacatatactgtgtccagagtataatgaacctgcagagttgtgcttcttactgctaattctgggagctttcacagtactgtcatcatttgtaaatggaaattctgcttttctgtttctgctccttctggagcagtgctactctgtaattttcctgaggcttatcacctcagtcatttcttttttaaatgtctgtgactggcagtgattctttttcttaaaaatctattaaatttgatgtcaaattagggagaaagatagttactcatcttgggctcttgtgccaatagcccttgtatgtatgtacttagagttttccaagtatgttctaagcacagaagtttctaaatggggccaaaattcagacttgagtatgttctttgaataccttaagaagttacaattagccgggcatggtggcccgtgcctgtagtcccagctacttgagaggctgaggcaggagaatcacttcaacccaggaggtggaggttacagtgagcagagatcgtgccactgcactccagcctgggtgacaagagagacttgtctccaaaaaaaaagttacacctaggtgtgaattttggcacaaaggagtgacaaacttatagttaaaagctgaataacttcagtgtggtataaaacgtggtttttaggctatgtttgtgattgctgaaaagaattctagtttacctcaaaatccttctctttccccaaattaagtgcctggccagctgtcataaattacatattccttttggtttttttaaaggttacatgttcaagagtgaaaataagatgttctgtctgaaggctaccatgccggatctgtaaatgaacctgttaaatgctgtatttgctccaacggcttactatagaatgttacttaatacaatatcatacttattacaatttttactataggagtgtaataggtaaaattaatctctattttagtgggcccatgtttagtctttcaccatcctttaaactgctgtgaatttttttgtcatgacttgaaagcaaggatagagaaacactttagagatatgtggggtttttttaccattccagagcttgtgagcataatcatatttgctttatatttatagtcatgaactcctaagttggcagctacaaccaagaaccaaaaaatggtgcgttctgcttcttgtaattcatctctgctaataaattataagaagcaaggaaaattagggaaaatattttatttggatggtttctataaacaagggactataattcttgtacattatttttcatctttgctgtttctttgagcagtctaatgtgccacacaattatctaaggtatttgttttctataagaattgttttaaaagtattcttgttaccagagtagttgtattatatttcaaaacgtaagatgatttttaaaagcctgagtactgacctaagatggaattgtatgaactctgctctggagggaggggaggatgtccgtggaagttgtaagacttttatttttttgtgccatcaaatataggtaaaaataattgtgcaattctgctgtttaaacaggaactattggcctccttggccctaaatggaagggccgatattttaagttgattattttattgtaaattaatccaacctagttctttttaatttggttgaatgttttttcttgttaaatgatgtttaaaaaataaaaactggaagttcttggcttagtcataattctt

SEQ ID NO: 46 - protein, 189 aa, Homo sapiens
MTEYKLVVVGAGGVGKSALTIQLIQNHFVDEYDPTIEDSYRKQVVIDGETCLLDILDTAGQEEYSAMRDQYMRTGEGFLCVFAINNSKSFADINLYREQIKRVKDSDDVPMVLVGNKCDLPTRTVDTKQAHELAKSYGIPFIETSAKTRQGVEDAFYTLVREIRQYRMKKLNSSDDGTQGCMGLPCVVM

SEQ ID NO: 47 - DNA, 1326 bp, Rattus norvegicus
gccgttcatggcggtttcggggtctccaacagcttctcaggttgaaatccaaaagcctcccgaggcggggtctgcggagtttgagatttttgcaggtgtgaaatgactgagtacaaactggtggtggttggagcaggtggcgttgggaaaagtgctttgacaatccagctaatccagaaccactttgtggatgaatatgatcccaccatagaggattcttaccgaaaacaagtggtgattgacggtgagacctgtctactggacatactggacacagctggacaagaggagtacagtgccatgagagaccaatacatgaggacaggcgaagggttcctctgtgtgtttgccatcaataatagcaaatcctttgcagatattaacctctacagggagcaaattaagcgcgtgaaagactctgatgatgtacccatggtgctggtagggaacaagtgtgacttgccaacaaggacagttgacacaaagcaagcccacgagctggccaagagttatggaattccattcattgaaacctcagccaagacccgacagggtgtggaggatgccttttacacgcttgtaagggagatacgccagtaccggatgaagaagctcaacagcagtgaggatggcactcaaggctgtatggggctgccctgtgtggtgatgtagtaagaccctttaaaagttctgtcatcagaaacgagccactttcaagcctcactgatgccctggttctgacatccctggaggagacgtgtttctgctgctctctgcatctcagagaagctcctgcttcctgcttccccaacttagttactgagcacagccatctaacctgagacctcttcagaataactacctcctcactcggctgtccgaccagagaaatgaacctgtttctccccagtagttctctgccctgggtttcccctagaaacaaacacacctgccagctggctttgtcctccgaaaagcagtttacattgatgcagagaaccaaactatagacaagcaattctgttgtcaacagtttcttaagctctaaggtaacaattgctggtgatttccccctttgcccccaactgttgaacttggccttgttagttttgggggaaatgtcaaaaattaatctcttcccgagaatagaattagtgttgctgattgcctgatttgcaatgtgatcagctatattctataagctggcgtctgctctgtattcataaatgcaaacatgagtactgacgtaagtgcatccctagtcttctcagctgcatgcaattaaatccaacgttcacaacaaaaaaaaaaaaaaaaaaaaaaaaa

SEQ ID NO: 48 - protein, 189 aa, Rattus norvegicus
MTEYKLVVVGAGGVGKSALTIQLIQNHFVDEYDPTIEDSYRKQVVIDGETCLLDILDTAGQEEYSAMRDQYMRTGEGFLCVFAINNSKSFADINLYREQIKRVKDSDDVPMVLVGNKCDLPTRTVDTKQAHELAKSYGIPFIETSAKTRQGVEDAFYTLVREIRQYRMKKLNSSEDGTQGCMGLPCVVM

SEQ ID NO: 49 - DNA, 4470 bp, Mus musculus
gggactggggcgccttgggcgcctagtgattacgtagcgggtggggccggaagtgccgctccctggcgggggctgttcatggcggtttcggggtctccaacagcttctcaggttgaagtccaaaagcctcccgaggcggggtctgcggagtttgaggtttttgctggtgtgaaatgactgagtacaaactggtggtggttggagcaggtggtgttgggaaaagcgccttgacgatccagctaatccagaaccactttgtggatgaatatgatcccaccatagaggattcttaccgaaagcaagtggtgattgatggtgagacctgcctgctggacatactggacacagctggacaagaggagtacagtgccatgagagaccagtacatgaggacaggcgaagggttcctctgtgtatttgccatcaataatagcaaatcatttgcagatattaacctctacagggagcaaattaagcgtgtgaaagattctgatgatgtccccatggtgctggtaggcaacaagtgtgacttgccaacaaggacagttgacacaaagcaagcccacgaactggccaagagttacggaattccattcattgagacctcagccaagacccgacagggtgtggaggatgccttttacacactggtaagggagatacgccagtaccgaatgaaaaagctcaacagcagtgacgatggcactcaaggttgtatggggctgccctgtgtgctgatgtagtaagacactttgaaagttctgtcatcagaaaagagccactttgaagctgcactgatgccctggttctgacatccctggaggagacctgttcctgctgctctctgcatctcagagaagctcctgcttcctgcttccccgactcagttactgagcacagccatctaacctgagacctcttcagaataactacctcctcactcggctgtctgaccagagaaatagacctgtctctcccggtcgttctctgccctgggttcccctagaaacagacacagcctccagctggctttgtcctctgaaaagcagtttacattgatgcagagaaccaaactagacatgccattctgttgacaacagtttcttatactctaaggtaacaactgctggtgattttcccctgcccccaactgttgaacttggccttgttggtttggggggaaaatgtcataaattactttcttcccaaaatataattagtgttgctgattgatttgtaatgtgatcagctatattccataaactggcatctgctctgtattcataaatgcaaacacgaatactctcaactgcatgcaattaaatccaacattcacaacaaagtgcctttttcctaaaagtgctctgtaggctccattacagtttgtaattggaatagatgtgtcaagaaccattgtataggaaagtgactctgagccatctacctttgagggaaaggtgtatgtacctgatggcagatgctttgtgtatgcacatgaagatagtttccctgtctgggattctcccaggagaaagatggaactgaaacaattacaagtaatttcatttaattctagctaatcttttttttttttttttttttttttggtagactatcacctataaatatttggaatatcttctagcttactgataatctaataattaatgagcttccattataatgaattggttcataccaggaagccctccatttatagtatagatactgtaaaaattggcatgttgttactttatagctgtgattaatgattcctcagaccttgctgagatatagttattagcagacaggttatatctttgctgcatagtttcttcatggaatatatatctatctgtatgtggagagaacgtggccctcagttcccttctcagcatccctcatctctcagcctagagaagttcgagcatcctagaggggcttgaacagttatctcggttaaaccatggtgctaatggaccgggtcatggtttcaaaacttgaacaagccagttagcatcacagagaaacagtccatccatatttgctccctgcctattattcctgcttacagacttttgcctgatgcctgctgttagtgctacaaggataaagcttgtgtggttctcaccaggactggaagtacctggtgagctctggggtaagcctagatatctttacattttcagacccttattcttagccacgtggaaactgaagccagagtccatacctccatctccttccccccccaaaaaaattagattaatgttctttatatagcttttttaaagtatttaaaacatgtctataagttaggctgccaactaacaaaagctgatgtgtttgttcaaataaagaggtatccttcgctactcgagagaagaatgtaaaatgccattgattgttgtcacttggaggcttgatgtttgccctgataattcattagtgggttttgtttgtcacatgatacctaagatgtaactcagctcagtaattctaatgaaaacataaattggataccttaattgaaaaaagcaaacctaattccaaaatggccattttctcttctgatcttgtaatacctaaaattctgaggtccttgggattcttttgtttataacaggatcttgctgtgtagtcctagctggcctcaaactcacaatactcttcctggatcaatctcccaagtgctgggattacaggcacattccaccacacacacctgactgagctcgttcctaatgagttttcattaagcaaattccccatcaccttgaaactaatcagaagggggaagaaacatttgctatgctcctgagtgctaacactgggatcattcacatggggtttgcattcctaggcaaactaaactgctgccttttacaacaaggctcagtcatcttcctgaagctgctgagaccagcacttggtcttgttttgttttaatatgtctatatgactggtggtggatccctaaatagtttattaattaaactccagttaaggagaaagttactcaccttgacccgtttgaccatatcccgtgtgtgtgtgtgtgtgtgtgtgtgtgtgtgtgtgtgtgtgtgtgtgcacgcgtatgtacgtacgtatgtatgtaggtatgtaggtggtttccagtataaacacagaaacaaatggagccaattcaggtttcagatgcccttactaacatatattcccacggggtgtgggttttggcacaacagtgacaaacttaaaagccaagtaagagccgggcgtggtggcgcacgcctttaatcccagcacttgggaggcagaggcaggcggatttctgagttctaggccatcctggtctacagtgagttccaggacagccagtgctacacagagaaaccctgtctcgaaaagccaaaaaaaaaaaaaaaaaaaaaaaaaaaaagccaagtaggtccagttggtatagtatcaaagtgtttttagagtaattagtgaaggtctgctttacctcaaagttgcagagcctctcttcctgagtttaagtgcctggccggcagtcacaaattaacatgttgctgtaaggcagttagttgaagctttgttcacacattggagagtatgaaaataaagtgttctaagagcgctgatactggatctgtgtaaacctggtaaatgccgtttgtccaggacttagcgtgtgtgagttggtagctcagtacgagtttactagttccgcagtgtgtacaatggaggcgggtttgttttagctggccacctgtagaatcagcctttaaactgctgtgaactttgtcatgacttgaatatgaagatagacaaaaactctgtaaagacaaatgtttgttttcccccttacagaacgtgtgagcttggttttatcttcctttgtatttagtcataacctctcaagctggcagctccgaccaaggatcagaagctgtgtgcgttccacctggtggaattagctcagctctatatgagaagtggagttaatggaaaacgtgttgactgggtggtttctatttaaaagagtgatgataattcttgaacagtagtttttattttgctatttctttaagctgactgatgtgccacaaaattattttaaggtatttgtgttttaagagtgttctcatgagattagttgtagatattttttaaaatacaactggtttttaaaatctgagtattgctctaagcaagtgtttagactcttacgggaaggtgggtggaagttgtttggcttccgtatttccatgcgtgccgtcagacataggtcagaacgccaactgtgcatcctgctgtttaaagacctcttggcctctgtgaccctcatgaaggggctgatattttaagttgactgtttgattgtaaattaatcctttctaatttttaaagacttgcttgactgttttccttgttaaataattttaaaaaaataaaaaactggaagttctttgcttaactgta

SEQ ID NO: 50 - protein, 189 aa, Mus musculus
MTEYKLVVVGAGGVGKSALTIQLIQNHFVDEYDPTIEDSYRKQVVIDGETCLLDILDTAGQEEYSAMRDQYMRTGEGFLCVFAINNSKSFADINLYREQIKRVKDSDDVPMVLVGNKCDLPTRTVDTKQAHELAKSYGIPFIETSAKTRQGVEDAFYTLVREIRQYRMKKLNSSDDGTQGCMGLPCVLM

SEQ ID NO: 51 - DNA, 570 bp, Cavia porcellus
atgactgagtataaactggtggtggttggagcaggtggtgtcgggaaaagtgcactgaccatccagctaattcagaaccactttgtcgatgaatatgatcccaccatagaggattcttaccgaaaacaggtggttatagatggtgaaacttgtctgttggatattctggatacagctggacaagaggagtacagtgccatgagagaccaatacatgaggacaggcgaaggcttcctctgtgtgtttgccatcaataatagcaaatcatttgcagatattaacctctacagggagcagattaaacgagtaaaagactcagatgatgtacctatggtgctggtagggaacaagtgtgatttgccaacaaggactgttgacacaaaacaagcccatgaactggccaagagttacgggattccattcattgaaacctcagccaagaccagacagggtgttgaagatgcattttacacactcgtaagagaaatacgccagtacagaatgaaaaaactcaacagcaatgatgatgggactcaaggttgtatggggttgccatgtgtggtgatgtaa

SEQ ID NO: 52 - protein, 189 aa, Cavia porcellus
MTEYKLVVVGAGGVGKSALTIQLIQNHFVDEYDPTIEDSYRKQVVIDGETCLLDILDTAGQEEYSAMRDQYMRTGEGFLCVFAINNSKSFADINLYREQIKRVKDSDDVPMVLVGNKCDLPTRTVDTKQAHELAKSYGIPFIETSAKTRQGVEDAFYTLVREIRQYRMKKLNSNDDGTQGCMGLPCVVM

SEQ ID NO: 53 - DNA, 1220 bp, Cavia porcellus
gttccggggtcctcaacgtttctcagggttgagattctatatccttttgaagctggggcggcagagcttgaggttcttgctggtgtgaaatgactgagtataaactggtggtggttggagcaggtggtgtcgggaaaagtgcactgaccatccagctaattcagaaccactttgtcgatgaatatgatcccaccatagaggattcttaccgaaaacaggtggttatagatggtgaaacttgtctgttggatattctggatacagctggacaagaggagtacagtgccatgagagaccaatacatgaggacaggcgaaggcttcctctgtgtgtttgccatcaataatagcaaatcatttgcagatattaacctctacagggagcagattaaacgagtaaaagactcagatgatgtacctatggtgctggtagggaacaagtgtgatttgccaacaaggactgttgacacaaaacaagcccatgaactggccaagagttacgggattccattcattgaaacctcagccaagaccagacagggtgttgaagatgcattttacacactcgtaagagaaatacgccagtacagaatgaaaaaactcaacagcaatgatgatgggactcaaggttgtatggggttgccatgtgtggtgatgtaacaagatatttaacaaagttctatcagaaaagagccactttcaagctgcactgataccctggtcctgacttccctggaggagaagtatccctgttgctctcttcatctcagagaagctcctgctgtttgtccacctctcagtgtatgagcacagtctctgcttgagaacttctcagaataactacctcctcacttggttgtctgaccagagaaatgcacctcttgttaattccccaataattttctgccctgggctctccccaacaaaaaacaaacacttctgccatccaaaaagcaacttggtctgaaacagaaccaaactgtagattgaaattctcttaaaaagtcttgagctctaaagttagcaaccgctggtgatttttattttcctttttatttttgaacttggaactgacctatgttagattttggagaaatgtcataaagtactgttgtgccaagaagataattatgttgctgaatggttgatttatagtgttatcagctatattttacaaactggcatctgctctgtattcataaatacaaaaatgaagccagg

SEQ ID NO: 54 - protein, 189 aa, Cavia porcellus; identical to SEQ ID NO: 52

SEQ ID NO: 55 - DNA, 1307 bp, Canis familiaris
tgattacgtagcgggcggggccggaagtgccgctccctagtgggggctgttcatggcggttccggggtctccaacctttctcctagttgtggtcctaaatacgtcggaagcggaggcggcgaagcttgaggttcttgctggtgtgaaatgactgagtacaaactggtggtggttggagcaggtggtgttgggaaaagcgcactgacaatccagctaatccagaaccactttgtagatgaatatgatcccaccatagaggattcttaccgaaaacaggtggttatagacggtgaaacctgtctgttggatatactggatacagctggtcaagaagagtacagtgccatgagagaccaatacatgaggacaggcgaaggcttcctctgtgtatttgccatcaataatagcaaatcatttgcagacattaacctctacagggaacagattaagcgagtaaaagattcagatgatgtacctatggtgctagtaggaaacaagtgtgatttgccaacaaggacagttgacacaaaacaagcccatgaactggccaagagttatgggattccattcattgaaacctcagccaagaccagacagggtgtcgaggatgccttttacacactggtaagagaaatacgtcagtaccgaatgaagaaactcaacagcagtgatgatgggactcaaggttgtatggggttaccatgtgtggtgatgtaacaagacacttttaaagttctagcatcagaaaagagccactgtcaagctgcactgacaccctggtcctgacttccctggaggagaagtattcctgttgctatcttcagtctcacaaagaagctcctgctacttccccaactctcagtagatcagtacaatgttctctatttgagaagttctccgaacaactacctcctcacttggttgtctgaccagagaaatgaacctcttgttccttcccgctgtttttccaccctgaattctcccccaacacacataaacaaacctctgccatcccaggtttttcatctgaaaaataattcatgctctgaaacagagaacaaaactgtagacatgaaattctgtaggaaacaaggtcttgagctcaaaagtagcaactgctggtgacctttttttcccccctttttactgttgaacttggaactatgttggtttttggagaaatgtcataagttactgttttgctgagaatatagttaagttgacatttggtttgtttgtaatatcattagctattttctataaattggcatctgctctgcattcataaatacacgagtgaattctga

SEQ ID NO: 56 - protein, 189 aa, Canis familiaris; identical to SEQ ID NO: 46

SEQ ID NO: 57 - DNA, 3104 bp, Felis catus
aaaaaataaataaatttaagaaaccattttaaaattatgcacagttgcagcctggaaaacttaaggtggcgccttatagtatcaatcttaggagctttatttggtgcatttaacgcaactggtaattgcaaaatccacttcgcctgtgtaagtgaaaaatatagactgttatcttgttggccctatgaaattctgcacttggtatttagcatatactctaccttcattactatctggcaagatgttctgccttagcactcagttgcattcttttccttttctttcctgttcattatgctttaattctgaggaccatatgagggtagaatatattaaaaattacaaaaattataaaaatttgtataggcaaaccatttccttaagttgatggccaaatgttaaaatgttatttttcatatcatttataatcttgtcacagtccacttaacgaagtttggttagatttcagtgaaaattatcttccagagtagtttttttttttttttcctgggattagggaggggggtaactttactgcaattagtatgtatggtgcagaatttcatgcaaatgaggtgtgccagcagtgtggtaatttaatcgtatttaaacaaaaacaaacaaaaaaaaaacgaatgcacaaacttgctgctgcttagatcactgcagcttctaggacccagtttcttttactgatttcaaaacaaaacaaaacaaaaaaataaaaaaagttgtgcctgaaatgaatcttgttttttttataagtagccgcctggttcctgtgtcctgtgaaatacaggcacttgacccttggtgtagcttctgttcgactttatatcacgggaatggattggtctgatttcttggccctcatcttgaattggccacatccagggtccctggccagtggactgaaggctttgtctaagaggacaagggcagctcaggggatgtgggggagggcgcttttatcttccccgttgtcgtttgaggttttgatcttctctgggtaaagaggccgtttatctttgtaaacacaaaacatttttgctttctccagttttctgttaatggcgaaagaatggaagcgaataaagttttactgatttttgagactctagcacctagcgctttcatttttgaaacgtcctgtgtgggaggggcgggtctgggtgcggcccgccgcgtgactcctgagtcgggggcccacgtggctggggcggggactcggacgccccgggcgccgactgattacgtagcgggcggggccggaagtgccgctccctagtgggggctgttcatggcggttccggggtctccatcctttttcccagttgttctaaatcagtcggaagcggaggcagcgaagtttgaggttctcgctggtgtgaaatgactgagtacaaactggtggtggttggagcaggtggtgttgggaaaagcgcactgacaatccagctaatccagaaccactttgtagatgaatatgatcccaccatagaggattcttaccgaaaacaggtggttatagacggtgaaacctgtctgttggacatactggatacagctggtcaagaagagtacagtgccatgagagaccaatacatgaggacaggcgaaggcttcctctgtgtatttgccatcaacaatagcaaatcatttgcagatattaacctttacagggaacagattaagcgagtaaaagactccgatgatgtacctatggtgctagtaggaaacaagtgtgatttgccaacaaggaccgtcgacacaaaacaagcccacgaactggccaagagttatgggattccattcattgaaacctcagccaagaccagacagggtgttgaagatgccttttacacactggtaagagaaatacgtcagtaccgaatgaagaaactcaacagcagtgatgacgggactcaaggttgtatggggttaccgtgtgtggtgatgtaacaagatacttttaaagttctagcatcagaaaagagccactgtcaagctgcactgacaccctggtcctgacttccctggaggagaagcgttcctgttgctattttcagtttcacaaagaagctcctgctatttccccaactctccgtagatcagtacattattctctgtttgagaagttctccgaataactacctcctcacttggttgtctgaccagagaaatgaacctcttgttactccccactgtttttccaccctggttctcccccagcacatataaacaaacctcccaggtttttcatctgaaaagtaattcatgctctgaaacagagaaccaaactgtagacatgaaattctgtaggaaacaatgtcttgagctctaaagtagcaactgctggtgactttttttttttttttttcctttttactgttgaacttggaactatgttggtttttggagaaatgtcgtaagttactgttttgctgagtatatagttaagtttaccattcggtttgtttgtaatgtcattggctatactctgtacctggcatctgctctgcattcataaatacaaaagtgaattctgacttttgagtctatcctagtgttctcaacttccacataattaaatctaacttttgcagcaaagtgcctttttcctagaagtggtttgtagatttgctttataatactttggtggaatagatgtctcaaaaaccattatacatgaaaatgaatgtctgagatacgtctatgatctgtctacctttgagggaaaaatataccgacataatagcagatgccatgtcttacgtgtatgaagttggatttccagagacctgatttgggtctcttccaagagaaagatgaaactggaaacaattatgaataacttcacttaatttttacctaatctctacttcggggtgggagggcagggagtaggttaccacttacaaaatatatgcaatttgtttcttctagcttactgataatgaacttccattcttatttaaatttaggtcatatcctaaagctttacatttgcaggtgttcgaaattgtaagtttaatgcagttttatttaatagctatgatcaatgattttcaagcctcagatgtattaacggacacattttcact

SEQ ID NO: 58 - protein, 189 aa, Felis catus; identical to SEQ ID NO: 46

SEQ ID NO: 59 - DNA, 4283 bp, Bos taurus
ggccgctccctagtgggggctgttcatggcggttccggggtctcccaacaattttcccggttgtggtcgtaatctatccgaagtggaggcagtggagctagaggttcttgctggtgtgaaatgactgagtacaaactggtggtggttggagcaggtggtgttgggaaaagtgcactgacaatccagctaatccagaaccactttgtagatgaatatgatcccaccatagaggattcctaccgaaaacaggtggttatagatggtgaaacctgtctgttggacatactggatacagctggacaagaggagtacagtgccatgagagaccaatacatgaggacaggcgaaggcttcctttgtgtgtttgccatcaataatagcaaatcatttgcagatattaacctctacagggaacagataaagcgtgtaaaggactcggatgatgtacctatggtgctagtaggaaacaagtgtgatttgccaacaaggacagttgacacaaaacaagcccatgaactggccaaaagttatgggattccattcattgaaacctcagccaagaccagacagggtgttgaagatgccttttacacactggtaagagaaatacgtcagtaccgaatgaaaaagctcaacagcagtgatgatggcactcaaggctgtatggggttgccgtgtgtggtgatgtaacaagatacttttaaagttctcacatcagaaaagagccactgtcaagctgcactgacaccctggtcctgacttccctggaggagaagtattcctgttgctatcttcagtttcaaaaagaagctcctgctatttccccaactctcagtagatcaatataatattctctatttgagaagttctcaagaataactacctcctcacttggttgtctgaccagagaattgaacctcttgttactcccagtatttttccaccctgggttctcccccagcacacacaaacgcacctctgccacccaggtttttcatctgaaaagcaattaatactctgaaacagagaaccaaactgtagaaacatgaaattctgtagaaaacaatgtcttgagctctaaagtagcaactgctggtgattttttttttttttttttcctttttattgttgaacttggaactatgttggtttgtggagaaatgtcataaattactgttttgctgagaatatagttaatgttgctctctggtttgtttgtaatgttatcagctatattctataaactggcatctactctgtatttagaaatacaaaaatgaatactgaccttttgagtctaccctcatcttctcgactttcttgtaattaaatgtaactttcacgatgaagtgccttttgcctgggagtgactcgtagacttcctttaaaatacttcagtggaatagatgtctcagaaactgttatacataagaataaatgtctgagatatgtctatgacccatctagctttgagggaaagatataccaatatgatagcagatgccatttcttacatctataacgttgattttctggagacctattttggggctctccgagagaaagatgagactataaatgattaggaataatttcacttaatttttacataacctccactttttgttttgtagtttactacctgcaaaacatataatttgattccttttagcttacagataatctaatgttaaatgaacttccattcatattttaatttggatcatatcaggaagtctacatttgcaggtgttcaaaaattgtaaaagtgtgatgcagttttatttaatagctgtgatcaatgattttcaagcctcaaatatgttaatagacacattttcactgtatatcatggtattaataattattgatgtatataattgtccttggtccccttctctgttcatcacctcatggcaatggcttgattaattatttcagctgagtaaagcatggtgctaatagaccagggtcacagtgtcaaaacttcagtgagccagtaagcatcacagagaaagaaattctttcacatttgctcaccattaactccagctaatagttttgccagatgtgtgtggttagtcctgcaaggaaaggagaagtcagttaatacaaattcttaaccaggactggaaaaacttgttttcctgagaagggtcagcttagaagtctttatctggactctatttttagccacatggaaatcaaattaagctgatcttttttctcaagtttttgagagtgaggatgcctcagatcaacatttttaaaatattctttattcttacgttcttttaagggtttaaaacaacgttgagtaattagtctgggcataccaggtaacaagctgataagtttgtgctgaacaagaagtagcctttggattgaaattgctgttttgagaagggatagaaaatataattaataattatgagacttgacttttctatttgcagataatatcctgataattctgatgaaaatagacttggataatttttgataaaagaatcgttccaaaatggccacttgctgttcttgtcttctaatgtgtaaatacttactgaggtcctcttctaatatgagttgtcatttattaagcaaattccacattgccttgaaatgaattcggaagagaagaaaaagtcatagtatacccagagaatgaaaaatccagagaattgtgctccttagtgttaattctgaagccttcgtagtccacacccatagacagaaactctctgccactttgcttctgctcctcttggagcattgcgctgtcatttccttgaggatagattgaggcttgtcaactcagttgtattgtcttcctcctcttcctcttgtctgtgtgactgacagtgtgactcttactaatgtcagatgcggggatgcggggaggtgggggggagtagctcattttaggctcttgcaccctttaccgttgtatgtgtgtgtcttttagttttctcaagaatgttctaagcacagaagtatctaaatggggccaaaattcagacttgaaaatgttcttttaatagcttcttaaaaagttacactttggtgtgaattttggcaggatagagtgacaaactcttaaacgctgaataacttcagttagtgtgttatagtttttagaatatgtttgtgattgctgaaaacaattatagtttacctcaaaatctgaaagtctctttccccaagttaagtgcctggccagctgtcaaagattacatattactttatgtttgtttgttttttaaaggttgcacattcaagattgtgaaaataaggtgttctgtctgaaagctaccatgcctgtctgtaaatgaatccactgagtgctgtacttgttccaacagcttactacagaatgctacttggtaatatcatactcgttacagttttcacttcaggagtgtactaggtagaatgatcctgtgtgtattgtagtgggctccatgtttagtcttttcagcatcctttaaactgctgtgaatttttgtcttgacttgaaagcaaggatagagaaacactttaaagagatactttgggtttttttccattccagaattggtgagcatagttagattttgctttacatttacagtcatgaactcttaagctggcagctacaaccaagaaccaaaagagggtgcattctgcttcttgtaattcatctttgctaataaattatgagaagcaaagataattaattagagaaactattttatttgggtggtttctataaacaagggactataattcttaaacattatttttcatttttgctgtttctttaagaaacctaatgtgccacaacattattttaaggtgtttcttaaaagaattgtttttaaaagtgttctcattttcagagtaattgtagatatatttcaaaatataactgataatttttaaaggcctgagtactgacctaagaagcagttgtatgaattctctggggggaagggaggagctcagtgaaagttgtatgacttttatatttctgtgccatcaaataaaggtaaaaatgtcttttgtgcagttttgctgttcaaacagaaactattggcctccttggccctaaatgaaagggctggtattttaagttgactattttattgtaaattaatccatcttaatttttttaaatttggttgaatgttctcttgttaaatgtttaaaaaataaaaactggaagttctttgcttagtcataaaaaaaaaaaaaaaaaaaaaaaaaaaaaaaaaaaaaaaaaaaaaaataaaaaaaaaaaaaaa

SEQ ID NO: 60 - protein, 189 aa, Bos taurus; identical to SEQ ID NO: 46

SEQ ID NO: 61 - DNA, 4825 bp, Gallus gallus
gcgccgggaccggaagccggaagctttgcagaagggtgttccgcgttcgcggtgcgggagcggtcagccggggtggcggggctggggccggccggggcaggcggctccgcgctccgcactgggccgctgggagggcgatgactgaatacaagctggtggtggtgggagctggcggcgtcgggaagagcgcgttgaccatccagctcatccagaaccacttcgtggacgagtacgaccccaccatcgaggattcgtacagaaagcaggttgtcatcgatggagagacgtgcttgttggacattctggacactgcaggacaggaagaatacagtgctatgcgtgatcagtacatgagaactggggaaggattcctttgtgtgtttgccattaacaacagtaaatcattcgctgatattaacctttacagagagcaaatcaagagagtgaaagattcagacgatgtgccaatggtgctggtggggaataagtgcgatttgccaacaaggacagtagacaccaaacaggctcaagagttagcaaaaagctacggcattcccttcatagagacatcagccaaaacgagacagggtgtggaagatgcgttttacacactggtgagggagattcggcagtaccggatgaaaaagctcaacagcaacgaagatgggaatcagggctgtatggggttgtcctgcattgtgatgtgataagatgccaggttcagatgtagctgctggacaagtctcgatgctactgtattgtgtctcatgctgatgccctgcagtattttggtgccagcgaccagactcttggtaccagttaattagctcaggatcctttcctgtgctccatctgaagaaaacatctctggtatctacctccttgctcagctcacagagcagtcatatctcttggtgtactgggattcttttctagctgtgttgtctgggtttgttcaagaagaaaaccagtcacaagaaaagtgaattacagagactaaatgctgtgaaaaagatcacactttacctccagagtaaaagctagaagtggcgtttgacccctttgcattggattcagatttgcggtgttgtcagaggagtggcagaagtaattttgccattacaaaggtttctgtcaccagtcggattggtatctgctgtctgtgcacccacacagtgtatctgcaacatctgcattgtgccagaagtatcacttaactgatgaactgatcctttatttttctgtaataaaaaggagatatctttgctaacttaagtgcctgtttgctcagaaggttggaggttgtatgctgttcccttgggctgaggagaaccccaaggatgaatttcttgggtgctcattgtcttgagcaggcaagttttgtgtgggtgatctcttttcatggcaggatattaaaatgggaatttgtagtctggaagatggagcagctgtttgtgagactcttgagttagggagagaaatgtataccacgtctgttctcgatccatcagaatggatccatccacctctttgtgtgtggaactgtgtatagtctgtattggttttctacagcacttggatctctttggaccaaattagcgagctgttcattttaacataactgccagtatttatagacaatttcttacggacagataatgaatttagaaactggaggttactttgggcagctgttcctcagctctgtctgtaacttgcaaattattctgagttattttctgcagaacctccttccttatcacgggaggagcctgggagttgaggttgactgtaattgggtcaatggttgtcacagacttaaggtgtccaggctgattggaggaggcactgagccctaacagagcactgagctgacttctaattgcagcatccttgcaaaatgaggaagggagttcagtgatgtctgcactgaagatgtatgatacactgatagcagttctgggtatgttgtaacagcttcaaagtagaaccgcagtactgcgtgagctgtgtgacttcttcctagaacacagcactgtcaccccatatggttgggacgtgcaggtgagaccaacacctaccaggttccctggcgtaccgtggccttctcagttcttgtgccagtgatactgggttctgttctgtggtgtcagacagcgtcctgtagcaaagctgaattcccacttagtctggtgagagaataaagagccatcagccaacagagggagcgttcattctgctggagcagtgcgagctgtaagcattacgagaggcgtagtttcagtttgttgcagtcaggttcctatattttcaaagctgaaatcagaaataagtaaatacggagaaaataagctgttgcttttaatgctctttcctccactaattgtactcttaattttcttcttgggaggccgaggatccatctgcataactttagctgtgatgctccagataagtgtttagaattcattttatctttgactgatgggactgataagaagttaacgcacaatatttttacatacaacatcgttttccagtgacctcctgagcggtgggaagcattatgggatagcaccggctgtgactcgagttcatttgaaggcgatctcttgcctgcaggttaaatgggacggagtcagaatcactgtgagccgtctgtaatcagcaaacagtctgtgggcttttcttactgtgttctctctgtttgccttagtttggtgcaggaagagttccttgtgacagcgtcctttgaggtgtgttgcaggagctgaccatttgctccttgagctgtgtgatgaactgttgtccacttaatggagttacagaagcagcttctgggagtcgcatctggtcgcatacattcagtgttttgggaagctgtcagtgtggtgtttgcactgtgtttgaatggtgttcatggtgggtctgttatgctcctggatgatttggggagatgtggggctgcttccgtggcagacaggatcagctcagggcgctgctgcctatggctgtgggaaacctcacagttggtgtttgaatagtggccaagtatgtcaattaaaaatacattttgaagggaggtttgtcatagctctgtactttggcatgctctgcttactgaaaacatactagctgtagctcaaaaaaagttgtgaatcctcagaataatacaggagctggcaattgtggctgctttctctttgtgttccttttctcttgggttggatgaagctttaaaaaggaaggagccctggtgagggttggtcagtgtgcatttcattcttggaaccagagaggaagttgcatcaactttcaggacgctgcagagctcacttgcacaggtggtgctccagtctatgtgatttttggggtcaaatcttgagatgatcttacaaaatcagattttgtacccatcatgagcatgaggtgagtggttgtgctcggtttctagctgcatgtatgtatacagacacgtgtatgcagacatgtctatgtgtgagtagttcgagtcagtcaaggttactggcagcacctaaagcgtatgcaccacataatgcatgcaggcaaaagtcctatcttaggagccatctcttcatgggtttgggtttatataggcagtatttttaaacagaatatccgaagcactttctggagttctgtggtaatgcagtgacacctatttggatgaaggaagatgtgtctgaggagcacgtaagcagatttgctgccctaacagagaggttttggtaaccgtggaaaaggttttctcctggatctgtgtgtgctcttggtgagctgcaatccatgacagggcacaaccagatgagaaggaaacccggccatcccatgcttgagcacagctctgactcagtagttccaccagatgtgccctttcagtcaaagtgttctgatctcttagagctttctgtagttcaagttaccactcactctccagcttgctcggttaatgtctgttggcggcgttgagttggacttgggaaaggtgtgtgtggtaggaacaagcagagtgtgatgtgcttctgttatcaggacttaagctagagtggttggcagataggaaatgcagctattccttgaaagcaagcagatcatggatggtcagccaaactgccctggctttggtgggagctgcactgcagaaggaccaaaccccaacaagatttggcacatttgtttagaagataagcacagatggttttgcacaaggcagctcctcataatggtggctttgtagatttagtccaaatgttcttatttagatctagcagcacatcactgtgtccgtgcccatctaacctcgctatcctaagtagagcagaccccaaacaaccttgttcaaaaactaccagtgcaaataactgaactaaatatttgttactgctgactgagaacagctgttcgagtgtagcattgtggcttgttaatgtgagtgccccaactctatggtcttattaaagaaacccaaacattgctcagattttgttcttattgtcatcataagacttgaatagtgatggtaatgcttacgtagacgtgtcttgtgagtgcacttcagtgatttagaaagaactggatttcaagcaactttggacctgtggggggagggagattaatgaaggtttgaatcacattctaattctatgtacagtccttcattactccacaagcctaaatcctatacagcctccaggatagctggaaactgttgagatctggactttttttttttaatccaagggctaacttgttgtaacttggtataattatctgctttcggaaatgcatctctgttggtttgaaa

SEQ ID NO: 62 - protein, 189 aa, Gallus gallus
MTEYKLVVVGAGGVGKSALTIQLIQNHFVDEYDPTIEDSYRKQVVIDGETCLLDILDTAGQEEYSAMRDQYMRTGEGFLCVFAINNSKSFADINLYREQIKRVKDSDDVPMVLVGNKCDLPTRTVDTKQAQELAKSYGIPFIETSAKTRQGVEDAFYTLVREIRQYRMKKLNSNEDGNQGCMGLSCIVM

SEQ ID NO: 63 - DNA, 2603 bp, Homo sapiens
aggcgaggcttccccttccccgcccctcccccggcctccagtccctcccagggccgcttcgcagagcggctaggagcacggcggcggcggcactttccccggcaggagctggagctgggctctggtgcgcgcgcggctgtgccgcccgagccggagggactggttggttgagagagagagaggaagggaatcccgggctgccgaaccgcacgttcagcccgctccgctcctgcagggcagcctttcggctctctgcgcgcgaagccgagtcccgggcgggtggggcgggggtccactgagaccgctaccggcccctcggcgctgacgggaccgcgcggggcgcacccgctgaaggcagccccggggcccgcggcccggacttggtcctgcgcagcgggcgcggggcagcgcagcgggaggaagcgagaggtgctgccctccccccggagttggaagcgcgttacccgggtccaaaatgcccaagaagaagccgacgcccatccagctgaacccggcccccgacggctctgcagttaacgggaccagctctgcggagaccaacttggaggccttgcagaagaagctggaggagctagagcttgatgagcagcagcgaaagcgccttgaggcctttcttacccagaagcagaaggtgggagaactgaaggatgacgactttgagaagatcagtgagctgggggctggcaatggcggtgtggtgttcaaggtctcccacaagccttctggcctggtcatggccagaaagctaattcatctggagatcaaacccgcaatccggaaccagatcataagggagctgcaggttctgcatgagtgcaactctccgtacatcgtgggcttctatggtgcgttctacagcgatggcgagatcagtatctgcatggagcacatggatggaggttctctggatcaagtcctgaagaaagctggaagaattcctgaacaaattttaggaaaagttagcattgctgtaataaaaggcctgacatatctgagggagaagcacaagatcatgcacagagatgtcaagccctccaacatcctagtcaactcccgtggggagatcaagctctgtgactttggggtcagcgggcagctcatcgactccatggccaactccttcgtgggcacaaggtcctacatgtcgccagaaagactccaggggactcattactctgtgcagtcagacatctggagcatgggactgtctctggtagagatggcggttgggaggtatcccatccctcctccagatgccaaggagctggagctgatgtttgggtgccaggtggaaggagatgcggctgagaccccacccaggccaaggacccccgggaggccccttagctcatacggaatggacagccgacctcccatggcaatttttgagttgttggattacatagtcaacgagcctcctccaaaactgcccagtggagtgttcagtctggaatttcaagattttgtgaataaatgcttaataaaaaaccccgcagagagagcagatttgaagcaactcatggttcatgcttttatcaagagatctgatgctgaggaagtggattttgcaggttggctctgctccaccatcggccttaaccagcccagcacaccaacccatgctgctggcgtctaagtgtttgggaagcaacaaagagcgagtcccctgcccggtggtttgccatgtcgcttttgggcctccttcccatgcctgtctctgttcagatgtgcatttcacctgtgacaaaggatgaagaacacagcatgtgccaagattctactcttgtcatttttaatattactgtctttattcttattactattattgttcccctaagtggattggctttgtgcttggggctatttgtgtgtatgctgatgatcaaaacctgtgccaggctgaattacagtgaaattttggtgaatgtgggtagtcattcttacaattgcactgctgttcctgctccatgactggctgtctgcctgtattttcgggattctttgacatttggtggtactttattcttgctgggcatactttctctctaggagggagccttgtgagatccttcacaggcagtgcatgtgaagcatgctttgctgctatgaaaatgagcatcagagagtgtacatcatgttattttattattattatttgcttttcatgtagaactcagcagttgacatccaaatctagccagagcccttcactgccatgatagctggggcttcaccagtctgtctactgtggtgatctgtagacttctggttgtatttctatatttattttcagtatactgtgtgggatacttagtggtatgtctctttaagttttgattaatgtttcttaaatggaattattttgaatgtcacaaattgatcaagatattaaaatgtcggatttatctttccccatatccaagtaccaatgctgttgtaaacaacgtgtatagtgcctaaaattgtatgaaaatccttttaaccattttaacctagatgtttaacaaatctaatctcttattctaataaatatactatgaaataaaaaaaaaaggatgaaagctaaaaaaaaaaaaaaaaaa

SEQ ID NO: 64 - protein, 393 aa, Homo sapiens [sequence omitted]

SEQ ID NO: 65 - DNA, 2151 bp, Rattus norvegicus
cggccgcgcgctccctgctgagttgcaggctgtttcccggctgcaagatgcccaagaagaagccgacgcccatccagctgaacccggcccccgatggctccgcggttaacgggaccagctcggccgagaccaacctggaggccttgcagaagaagctggaggagctggagctggacgagcagcagcggaagcgccttgaggcctttctgacgcagaagcagaaggtgggagagttgaaggatgatgactttgagaagatcagtgaactgggggctggcaatggtggagtggtgttcaaggtctcccacaagccatctggcctggttatggctaggaagctaattcacctggagatcaaacccgcaatccggaaccagatcatccgggagctgcaggtgctgcatgagtgcaactccccgtacatagtgggcttctacggggccttctacagtgacggcgagatcagcatctgcatggagcacatggatggtgggtccttggatcaagtgctgaagaaagctggaagaattcctgagcaaattttaggaaaagtcagcatcgctgtgataaaaggcctgacatatctacgagagaagcacaagattatgcacagagatgtcaagccttccaacattctagtgaactcacgtggggagatcaaactctgcgattttggggtcagcgggcagctaattgactccatggccaactccttcgtgggaacaaggtcctacatgtcgcctgagagactccaggggactcactactctgtgcagtcggacatctggagcatggggctctctctggtggagatggcagttggaagataccccattcctcctcctgatgccaaggagctggagctgctgtttggatgccaggtggaaggagacgcggccgaaacgccacccaggccaaggacccctgggaggcccctcagctcatatggaatggatagccgacctcccatggcaatttttgagttgttggattacatcgtcaatgagcctcctccaaaactgcccagtggagtattcagtctggaatttcaggattttgtgaataagtgcttaataaagaaccctgcagagagagcagatctgaagcagctcatggtacatgctttcatcaagagatctgatgccgaggaggtagacttcgcaggctggctctgctccaccattgggcttaaccagcccagcacaccaacccacgctgccagcatctgagcctttgggaagcagcagagaggaatcctctgcccagtggcatgccatgttgctttcaggcctctcccatgcttgtctatgttcagatgtgcatctcatctgtgacaaaggatgaagaacacagcatgtgccaaatcgtacttgtgtcatttttaatattgtctttatcgctatggttactcccctaagtggattggctttgtgcttggggctatttgtctgttcatcaaatacatgccaggttgaactacagtgaaaccctggtgacctgggtggtcttcttactgatgtttgcgctgctgttcatcgtgactcactagctggctgcctgtattgtcaggattctcggacccttggtacttcactcttgctggtgacctctcagtctgaggagagggggccttctgagacccttcacaggcagtgcatgcatgaaaagcatgctttgctgctactgaaatgagcaccagaacgtgtacatcatggtattttatttttgcttttggtatagaactcagcagttcccatttaaaaaaaaaatctaaccagagcccatcactgccatgatagctggggcttcagtctgtctactgtggtgatttttagacttctggttgtatttctatatttatttttaaatatactgtgtgggatacttagtggtatatgtctctgagtttggattagtgtttctaaattggtagttattttgaatgtcacaaatggattaaggaatcaacgtatcaagagttctatctttcttccagtctaagtaccaatgctattgtaaacgtgtatagtgcctacaaattgtatgaaaacccttttaaccactttactcaagatgtttatcaaatctaatctcttattctaataaaaatactatcaagttaaagtaaaaaaaaaaaaaaaaaaaaaaaaa

SEQ ID NO: 66 - protein, 393 aa, Rattus norvegicus
MPKKKPTPIQLNPAPDGSAVNGTSSAETNLEALQKKLEELELDEQQRKRLEAFLTQKQKVGELKDDDFEKISELGAGNGGVVFKVSHKPSGLVMARKLIHLEIKPAIRNQIIRELQVLHECNSPYIVGFYGAFYSDGEISICMEHMDGGSLDQVLKKAGRIPEQILGKVSIAVIKGLTYLREKHKIMHRDVKPSNILVNSRGEIKLCDFGVSGQLIDSMANSFVGTRSYMSPERLQGTHYSVQSDIWSMGLSLVEMAVGRYPIPPPDAKELELLFGCQVEGDAAETPPRPRTPGRPLSSYGMDSRPPMAIFELLDYIVNEPPPKLPSGVFSLEFQDFVNKCLIKNPAERADLKQLMVHAFIKRSDAEEVDFAGWLCSTIGLNQPSTPTHAASI

SEQ ID NO: 67 - DNA, 2387 bp, Mus musculus
agtccctcactgggacgtctgtgcgcggcgtctcggagcgccggagcagcggtggccgcactttctccaagctggggctgtagctgagctgtgggtagtgcgcagggagccgtccgagcccgaggaaccggtgtgctgaggcgagagttcccggccggcgagcgcgcgcagctggttctccgcgtgggttgggcggagggtcccaggagcgcggcgttgatcgagccgccccgactctgggcagagccgagggaggaagcgagaagcggccgcgcgctccctgctgagttgcaggctctttcccggctgcaagatgcccaagaagaagccgacgcccatccagctgaacccggcccccgatggctcggcggttaacgggaccagctcggccgagaccaacctggaggccttgcagaagaagctggaggagctggagcttgacgagcagcagcggaagcggctcgaggcctttctgacgcagaagcagaaggtgggggaactgaaggatgatgactttgagaagatcagcgaactgggagctggcaacggtggagtggtcttcaaggtctcccacaagccatctggcctggttatggctagaaagctgatccacctggagatcaaacccgcaatccggaaccagatcatccgggagctgcaggtactgcacgagtgcaactccccgtacatcgtgggcttctacggggccttctacagcgacggcgagatcagcatctgcatggagcacatggatggtgggtccttggatcaagttctgaagaaagctggaagaattcctgagcaaattttaggaaaagttagcattgctgtgataaaaggcctgacctatcttcgggagaagcacaagattatgcacagagatgtcaagccatccaacattctagtgaactcacgtggggagatcaaactctgtgattttggggtcagcgggcagctaattgactctatggccaactccttcgtgggcacgagatcctacatgtcgcctgagagactccaggggactcactactctgtgcagtcggacatctggagcatggggctctctctggtggagatggcagttgggagataccccattcctcctcctgatgccaaggagctggagctactgtttggatgccatgtggaaggagacgcagccgaaacaccacccaggccaaggacccctgggaggcctctcagctcatatggaatggacagccgacctcccatggcaatttttgagttgttggattacattgtcaatgagcctcctccaaaactgcccagtggagtattcagtctggagtttcaggattttgtgaataaatgcttaataaagaaccctgcagagagagcagatctgaagcagctcatggtacatgctttcatcaaaagatctgacgccgaggaggtagacttcgcaggctggctctgctccaccattgggcttaaccagcccagcacaccaacccacgctgccagcatctgagcctttaggaagcagcaaagaggaattctctgcccagtggcatgccatgttgctttcaggcctctcccatgcttgtctatgttcagacgtgcatctcatctgtgacaaaggatgaagaacacagcatgtgccaaattgtacttgtgtcatttttaatatcattgtctttatcactatggttactcccctaagtggattggctttgtgcttggggctatttgtctgttcatcaaacacatgccaggctgaactacagtgaaaccctagtgacctgggtggtcgttcttactgatgtttgcactgctgttcatcgtgactcactagctggctgcctgtattgtcaggattctcggaccttggtacttcactcttgctggtgacctctcagtctgagagggagccttgtgagacccttcacaggcagtgcatgcatggaaagcatgctttgctgctactgaaatgagcatcagaacgtgtacgtcatggtatttttattttttgcttttggtatagaactcagcaattcccatcaaaaaaacctaagcagagcccatcactgccatgatagctgggcttcagtctgtctactgtggtgatttttagacttctggttgtatttctatatttatttttaaatatacagtgtgggatacttagtggtgtgtgtctctaagtttggattagtgtttctaaattggtggttattttgaatgtcacaaatggattaaagcatcaatgtatcaagagttctatctttcttccagtctaagtaccaatgctattgtaaacaacgtgtatagtgcctacaaattgtatgaaaccccttttaaccactttaatcaagatgtttatcaaatctaatctcttattctaataaaaatactatcaagtt

SEQ ID NO: 68 - protein, 393 aa, Mus musculus
MPKKKPTPIQLNPAPDGSAVNGTSSAETNLEALQKKLEELELDEQQRKRLEAFLTQKQKVGELKDDDFEKISELGAGNGGVVFKVSHKPSGLVMARKLIHLEIKPAIRNQIIRELQVLHECNSPYIVGFYGAFYSDGEISICMEHMDGGSLDQVLKKAGRIPEQILGKVSIAVIKGLTYLREKHKIMHRDVKPSNILVNSRGEIKLCDFGVSGQLIDSMANSFVGTRSYMSPERLQGTHYSVQSDIWSMGLSLVEMAVGRYPIPPPDAKELELLFGCHVEGDAAETPPRPRTPGRPLSSYGMDSRPPMAIFELLDYIVNEPPPKLPSGVFSLEFQDFVNKCLIKNPAERADLKQLMVHAFIKRSDAEEVDFAGWLCSTIGLNQPSTPTHAASI

SEQ ID NO: 69 - DNA, 1182 bp, Oryctolagus cuniculus
atgccaaagaagaagcccacccccatccagctgaatcctgcccctgacggctcggcggtgaatggtaccagctcggcggagaccaacctggaggccttgcagaagaagctggaggagctggagcttgacgagcagcagcggaagcgcctggaggccttcctcacccagaagcagaaagtgggagagctgaaggacgatgacttcgagaagatcagtgagctgggagccggcaacggcggcgtggtgttcaaggtctcccacaagcccagtggcctggtgatggccagaaagcttattcacctggagatcaaacctgctatccggaaccagatcataagggagctgcaggttctgcacgagtgcaactccccgtacatcgtgggcttctacggggcattctacagcgatggcgagatcagcatctgcatggagcacatggacgggggttccttggatcaagtcctgaagaaagctggacggattcccgagcaaattttggggaaagttagcattgctgtgatcaagggcctgacgtatctgagggagaagcacaagatcatgcacagagatgtgaagccctccaacatcctggtcaactcccgcggggagatcaagctctgtgacttcggggtcagtgggcagctcatcgactccatggccaactccttcgtgggcaccaggtcttatatgtcgcccgagagactccaggggacacactactctgtgcagtcggacatctggagcatggggctgtccctggtggagatggcggtggggcggtaccccatcccgccccccgacgccaaggagctggagctgatgtttgggtgccaggtggagggcgatgcggccgagactccgcccaggcccaggacccctgggcggcccctcagctcgtatggaatggatagccggcctcccatggcgatttttgagctgctggattacatcgtcaatgagcctcctccgaaactccccagcgcagtcttcagcctggagtttcaagattttgtgaataaatgcttaataaaaaaccccgccgagagagcagacttgaagcagctcatggttcatgcttttatcaagaggtctgatgccgaggaggtggattttgctggttggctgtgctccaccatcggccttaaccagcccagcacgccgacgcacgcggccggtgtgtga

SEQ ID NO: 70 - protein, 393 aa, Oryctolagus cuniculus
MPKKKPTPIQLNPAPDGSAVNGTSSAETNLEALQKKLEELELDEQQRKRLEAFLTQKQKVGELKDDDFEKISELGAGNGGVVFKVSHKPSGLVMARKLIHLEIKPAIRNQIIRELQVLHECNSPYIVGFYGAFYSDGEISICMEHMDGGSLDQVLKKAGRIPEQILGKVSIAVIKGLTYLREKHKIMHRDVKPSNILVNSRGEIKLCDFGVSGQLIDSMANSFVGTRSYMSPERLQGTHYSVQSDIWSMGLSLVEMAVGRYPIPPPDAKELELMFGCQVEGDAAETPPRPRTPGRPLSSYGMDSRPPMAIFELLDYIVNEPPPKLPSAVFSLEFQDFVNKCLIKNPAERADLKQLMVHAFIKRSDAEEVDFAGWLCSTIGLNQPSTPTHAAGV

SEQ ID NO: 71 - DNA, 1872 bp, Cavia porcellus
cgtgtcttcgtcgggaccgccctcctccttgagtcctccccccaccgggacggccgagtggagaggccggacgaaggcggcggccccggcggcggcttttcctcggcttcgctgtgcagcgtgcgcggcgaggttgaccgcccgcgagcgcccgtgactgagggaacagggagagagctcgggcggccgagcgcgcagccctccgtgggcattgccgcctggacctcccggaaggcaccccgggccgcggccgccacccgtcccgccctcgttcggagctgagacgccgtcgccgcgcaagatgcccaagaagaagccgacgcccatccagctgaacccggcccccgacggctcggcggtgaacgggaccagctcggccgagaccaacctagaggctttgcagaagaagctggaggagctggagctggatgagcagcagcggaagcgcctcgaagctttcctgacacagaagcagaaggtgggcgagctgaaggacgatgactttgagaagatcagtgagctgggtgccggcaatggcggtgtggtgttcaaggtctcccacaagccatctggcctggtcatggcccgaaagcttatccacctggagatcaagccagccatccgcaatcagatcatccgtgagctgcaggttctgcacgagtgcaactcgccctacattgtgggcttctatggggccttctacagtgatggcgagatcagcatctgcatggagcacatggatggaggttccttggatcaagtcctgaagaaagctggaagaattcctgagcaaattttaggaaaagttagcattgctgtgatcaaaggcctgacatacctgagggagaagcacaagattatgcacagagatgtcaagccctccaacatcctggtcaactcccgcggggagatcaagctctgtgactttggggtcagcgggcagctcatcgattccatggccaactccttcgtgggcacccggtcctacatgtcgccagagagactgcagggcacacactactcagtgcagtcggacatctggagcatgggactgtcactggtggagatggcggttgggaggtaccccatcccccctccagatgccaaggagctggagctggtgttcgggtgccaggtggaaggagatgcagctgagatgccgcccaggcccaggacccccggaagacccctgagctcatatggaatggacagccggcctcccatggcgattttcgagctgttggattacatagtcaacgagccacctcccaaactgcccagtggagtcttcagtctggaattccaggactttgtaaataaatgcttaataaagaaccctgcggagagagcagacttgaagcagctcatggttcatgccttcatcaagcgctctgatgctgaggaggtggacttcgcaggttggctctgtgccaccatcggccttaaccagcccagtaccccgacccacgtggccagcatctgagctgcggcccggcccagacgtgctctgccagcagccgctatgctctggcctctccctcgcttctcttcagacgtgcgtttcacctccgaccagggtgcagacacagcatgtgccaagctgtatttgtgttccttttcagtctttattgccaccgtgtcacccgagtggatttgctttgtgcttagggctgtttgtgctgatgatcacacacacgctgagctgaacagtgacacttggtgatgtggttgtcactgttctcactccatgtggctggcctgttgcctccagtgtctccagacttggggatgtctggtggcacttcccctgccagggcatctcctcagcagagagggaggcctctgggcccttgtccttggcagtgcaagtga

SEQ ID NO: 72 - protein, 393 aa, Cavia porcellus
MPKKKPTPIQLNPAPDGSAVNGTSSAETNLEALQKKLEELELDEQQRKRLEAFLTQKQKVGELKDDDFEKISELGAGNGGVVFKVSHKPSGLVMARKLIHLEIKPAIRNQIIRELQVLHECNSPYIVGFYGAFYSDGEISICMEHMDGGSLDQVLKKAGRIPEQILGKVSIAVIKGLTYLREKHKIMHRDVKPSNILVNSRGEIKLCDFGVSGQLIDSMANSFVGTRSYMSPERLQGTHYSVQSDIWSMGLSLVEMAVGRYPIPPPDAKELELVFGCQVEGDAAEMPPRPRTPGRPLSSYGMDSRPPMAIFELLDYIVNEPPPKLPSGVFSLEFQDFVNKCLIKNPAERADLKQLMVHAFIKRSDAEEVDFAGWLCATIGLNQPSTPTHVASI

SEQ ID NO: 73 - DNA, 1257 bp, Canis familiaris
ggagagcgagacacgggccgctctccgctcggagccggacgcgccttcccgcgtccaaaatgcccaagaagaagccgacgcccatccagctgaacccggcccccgacggctcggcggtgaacgggaccagctcggcggagaccaacctggaggccttgcagaagaagctggaggagctggagcttgatgagcagcagcggaagcgccttgaggcctttctcacccagaagcagaaggtcggggaactgaaggatgacgacttcgagaagatcagtgagctgggtgctggcaacggtggcgtggtgttcaaggtctcccacaagccgtccggcctagtcatggccagaaagctaattcacctggagatcaaacctgcaatccggaaccagatcataagggagctacaggttctacatgagtgcaactccccgtacatcgtgggcttctatggtgcattctacagcgatggcgagatcagtatctgcatggagcacatggatgggggttccttggatcaagtcctgaagaaagctggaagaattcctgaacaaattctaggaaaagttagcatcgctgtaataaaaggtctgacatacctgagagagaagcacaagattatgcacagagatgtcaagccttccaacatcctcgtgaactcccgtggggagatcaagctctgtgactttggggtcagcgggcagctcattgactccatggccaactccttcgtgggcacaaggtcctacatgtcgccagaaagactccaggggactcattactccgtgcagtcggacatctggagcatggggctctctctggtggagatggcagttgggaggtatcccatccctcctccggatgccaaggagctggagctgatgtttgggtgccaagtggagggagacgtggctgagaccccacccagaccaaggaccccgggaagaccccttagctcttatggaatggacagccgaccgcccatggcaatttttgagctgttggattacatagtcaacgagccccctccaaaactgcccagtggagtattcagtctggaatttcaagattttgtgaataaatgcttaataaaaaacccagcagagagagcagatctgaagcaactcatggttcatgccttcatcaagagatctgacggtgaagaagtggattttgcaggttggctctgctccccccattggccttaaccagcccagcacgccgacccacgcagctggcgtctaactcgagtctagagat

SEQ ID NO: 74 - protein, 381 aa, Canis familiaris
MPKKKPTPIQLNPAPDGSAVNGTSSAETNLEALQKKLEELELDEQQRKRLEAFLTQKQKVGELKDDDFEKISELGAGNGGVVFKVSHKPSGLVMARKLIHLEIKPAIRNQIIRELQVLHECNSPYIVGFYGAFYSDGEISICMEHMDGGSLDQVLKKAGRIPEQILGKVSIAVIKGLTYLREKHKIMHRDVKPSNILVNSRGEIKLCDFGVSGQLIDSMANSFVGTRSYMSPERLQGTHYSVQSDIWSMGLSLVEMAVGRYPIPPPDAKELELMFGCQVEGDVAETPPRPRTPGRPLSSYGMDSRPPMAIFELLDYIVNEPPPKLPSGVFSLEFQDFVNKCLIKNPAERADLKQLMVHAFIKRSDGEEVDFAGWLCSPHWP

SEQ ID NO: 75 - DNA, 2095 bp, Felis catus
agccggcaaggagttgagcgtgcggggtgcataggcgcgggtcgtgggagatgaagctggagaggaccaacctggaggccttgcagaagaagctggaggagctggagctcgatgagcagcaacggaagcgcctggaggcctttcttacccagaagcagaaggtcggggaattgaaggatgacgacttcgagaagatcagcgagctgggcgctggcaacggtggtgtggtgttcaaggtctcccataagccgtctggcctggtcatggccagaaagctaattcacctggagatcaaacctgcaatccggaaccagatcataagggagctgcaggttctacatgagtgcaactccccatacatcgtgggcttctatggcgcgttctacagcgacggcgagatcagtatctgtatggagcacatggatgggggttccttggatcaagtcctgaagaaagctggaagaattcctgaacaaattttaggaaaagttagcattgctgtaataaaaggtctgacatacctgagggagaagcacaagattatgcacagagatgtcaagccttccaacatcctagtgaactctcgtggggagatcaagctctgtgactttggggtcagcgggcagctcatcgactccatggccaactccttcgtgggcacaaggtcctacatgtcgccagaaagactccaggggactcattactccgtgcagtcggacatctggagcatggggctatctctggttgagatggcagtcgggaggtatcccatccctcctcccgatgccaaggagctggagctgatgtttgggtgccaagtggagggagatgcggctgagacgccacccaggccgaggacccccggaaggcccctcagctcgtatggaatggacagccgacctcccatggcaatttttgagttgttggattacatagtcaacgagcctcctccaaagctgcccagtggagtattcagtctggaatttcaagattttgtgaataaatgcctcataaaaaacccagcagagagagcagatctgaaacaactcatggttcatgcctttatcaagagatctgatggtgaggaagtggattttgcaggttggctctgctccaccatcggccttaaccagcccagcacaccgacccacgcggccggcgtctaagtatctgggaagcagcaaagagcgagtcccctgcccagtggtgtgccattgtcgctttcaggcctctttgccatgcctgtctccgttcagacgtgcatttcgcctacgacaaaggatgaagaacacagcatgtgccaaaattctatttgtgtcttttttaatattactgtcatttattctgttatttccctaagtggattggctttgtgcttggggctatttttgtgtatgttgatccaaacatgcgcaacgttcagttacagtgaaaccttggtgactgtgggtagtcattcttactgaaaattgcactgctcttcccccaccgtgactggctagctgcctgtagttttgggattcttttgacacttggtggtactgcattcttgccgggcgcaccttccttctgttggggtaggagccttgtaagatccttcacaggcactgcatgtgaagcatgctttgctgctatgaaaaagaacatcagaaagtatagatcttgttattttattatatttttgcttttggtgtagaatgaagcaatttctgtcaaaatctagccagagcccttcactgccacgatagctggggcttcaccagtctgtctactgtgatgatttgtagacttctggttgtatttctatatttattttaaaatatattatgtgggatatttagtggtatgtgtctctttaagtttgaattagtgtttctaaaatgatggttactttgaatgttacaaatggatcaaggcattaaaatgtatgagatttatctttccccaaatccaagtaccgatgctattgtaaacaacagtgtgtatagtgcctaagaattgtatgaaaatccttttaaccatttcaacccagatgtttaacaaatctaatctcttattctaataaatatactatcaagttaaaaggatgaaaaaa

SEQ ID NO: 76 - protein, 371 aa, Felis catus
MKLERTNLEALQKKLEELELDEQQRKRLEAFLTQKQKVGELKDDDFEKISELGAGNGGVVFKVSHKPSGLVMARKLIHLEIKPAIRNQIIRELQVLHECNSPYIVGFYGAFYSDGEISICMEHMDGGSLDQVLKKAGRIPEQILGKVSIAVIKGLTYLREKHKIMHRDVKPSNILVNSRGEIKLCDFGVSGQLIDSMANSFVGTRSYMSPERLQGTHYSVQSDIWSMGLSLVEMAVGRYPIPPPDAKELELMFGCQVEGDAAETPPRPRTPGRPLSSYGMDSRPPMAIFELLDYIVNEPPPKLPSGVFSLEFQDFVNKCLIKNPAERADLKQLMVHAFIKRSDGEEVDFAGWLCSTIGLNQPSTPTHAAGV

SEQ ID NO: 77 - DNA, 2405 bp, Bos taurus
ccggttgactgagggagagtgggagggaatcccgggctgccgagctgcgccggcggggaagcccttcggttccctgtgcactgagcaagtgggccggggggttcccccagaccgccactggccctttggccctgacgggaccgcgcagggcgcgccccccgaaggcagccttcgggcttgcggcccagacttggccccgcgaggccggcgcggggcagctcagagggaggaagctagaggggccgccctcagagttgggagcgcctttcctgggtccaaaatgcccaagaagaagccgacgcccatccagctgaacccggccccggacggctccgcggttaacgggaccagctcggcggagaccaacctggaggccttgcagaagaagctggaggagctggagctcgatgaacagcagcggaagcgcctcgaggcctttctgacccagaagcagaaggtgggggaactgaaggatgatgactttgagaagatcagtgagctgggtgccggcaatggaggtgtggtgttcaaggtctcccacaagccgtccggacttgttatggccagaaagctaattcacctggagatcaaacctgccatccggaaccagatcataagggagctgcaggttctccatgagtgcaactcgccttatatcgtgggcttctacggggcgttctacagcgacggcgagatcagcatctgcatggagcacatggatgggggttccttggatcaagttctgaagaaagctggaagaattcctgaacaaattttaggaaaagttagcattgctgtaataaaaggcctgacatacctgagggagaagcacaagattatgcacagagatgtcaagccgtccaacatcctagtgaacagccgtggagagatcaagctctgtgactttggggtcagcgggcagctcatcgactccatggccaactccttcgtgggcaccaggtcctacatgtcgccagagcgactccaggggacccattactccgtgcagtcggacatctggagcatggggctctctctggttgagatggctgtcgggaggtatcccatccctcctccagatgccaaggagctggagctgatgtttgggtgccaggtggagggagatgcggctgagaccccgcccaggccaaggacccccgggaggcccctcagctcttatggaatggacagccgacctccaatggcaatttttgagttgttggattacatagtcaatgagcctcctccaaaactgcccagtggagtattcagtctggaatttcaagattttgtgaataaatgcttaataaaaaaccccgcagagagagcagatttgaagcaactcatggttcatgcttttatcaagagatctgatgctgaggaagtggattttgcaggttggctctgctccaccatcggccttaaccaacccagcacacccacccatgcggctggcgtctaagtggttgggaagcagcagtccctgcccaagggcatgcactgttgcttccgggcagccttcccatgcctgtctctgttcagacgtgcatttcacctatgacaaaggatgaagaacacagcatgtgccaaaattctatttgtgtcattttcaatattatcatctttactcttattactattgttattcccctaagtggattggctttgtgcttggggctatttttgtgtatattgatgatgaagacatgtgcaatgtagaattacagtgaaactctggtgactgtgggtagtcattcttactgaaaactgcactgctttcccacaccatgaactggctggtcgcctctattttcgggattctttgacacttggtggtacttcattcttgccaggcataccttctaactgagtaggaaggagccttgtaagatccttcacaggcagtgcatgtgaagcatgctttgctgctataaaaatgagcatcagaaagtgtgtatcatgttattttattatgttcttgcttttggtgtagaattcagcaaattttcatcaaaatctagccagagcccttcactgccatgatagctggggcttcaccagtctgtctactgtgatgatttgtagacttctggttgtatttctgtatttatttttaaatctaccgtgtggatatttagtgctatgtctctttaagtttggattagtgtttctaaaatggtggagttgctctgaatgttacaaatggatcaaggcattaaaatgaatgagatctacctttcaccaagtactgatgctattgtaaacaacagtgtgtatagtgcctaacaactgtatgaaaatccttttaccattttaatccagatgtttaacaagcctaatctcttactctaataaatatactatcaaattcaaaggaaaaaaaaaaaaaaaaaaaaaaaaaaaaa

SEQ ID NO: 78 - protein, 393 aa, Bos taurus [sequence omitted]

SEQ ID NO: 79 - DNA, 2146 bp, Equus caballus
caagtgggaaagcttgggatgcgtggaggagccagctactagtttagtgtgctgggtgcgtcggtgcaggtcgcaggagatgaagccggagaggaccaacctggaggccttgcagaagaagctggaggagctggagctcgatgaacagcagcgaaagcgccttgaggcctttcttactcagaagcagaaggttggggaactgaaggatgatgactttgagaagatcagtgagctgggtgctggcaatggtggtgtggtattcaaggttgcccacaaaccgtctggtttggtcatggccagaaagctaattcacctggagatcaagcctgcaatccggaaccagatcataagggagctgcaggttctacatgagtgcaactccccatatattgtgggcttctatggcgcattctacagcgatggtgagatcagcatctgcatggagcacatggatgggggttccttggatcaagtcctaaagaaagctggaagaattcctgagcaaattttaggaaaagttagcattgctgtaataaaaggcctgacgtatctgagggagaagcacaagattatgcacagagatgtcaagccctccaacatcctagtgaactcccgtggggagatcaagctgtgtgattttggggtcagcgggcagctcatcgactccatggccaactccttcgtgggcacaaggtcttacatgtcgccggaaagactccaggggactcattattcagtgcagtcggacatctggagcatggggctctctctggttgagatggcggtcgggaggtatcccatccctcctccagatgccaaggagctggagctgatgtttgggtgccaagtggagggagatgcggctgagactccgcctaggccaaggacccctggaagacccctcagctcttatggaatggacagccgacctcctatggcaatttttgagttactggattacatagtcaacgagcctcctcccaagctgcccagtggagtattcagtctggaatttcaggattttgtgaataaatgcttaatcaaaaaccctgcagagagagcagatttgaagcaactcatggttcacgcttttatcaagagatctgatgccgaggaagtggattttgcaggttggctctgctccaccattggccttaaccagcccagcacaccaacccacgcggctggcgtctaagcgtttgggaagcagcaaaaagcgagccccctgccgcgtggtgtgccatgttgctttcgggcctccttcccatgcctgtctgttcacacgtgcatttcacctgtgacaaaggatgaagaacacagcatgtgccaaaattctatttgtgtcatttttaatagtactgtctttattcttattactattgttattcccctaagtggattggctttgtgcttgggactattttgtgtatgttgatgatcaaaacatgcgcaatgttgaattaccgtgaaactggtgactgtgggtagtccttcttattgaaaattgcactgctcttccctccctgtcactggctggctgcctgtatttctggggttctttgacacttggtggtacttcattcttgcagggcatacctcctattcgagtaggaaggagcctttaagatccttcacaggcagtgcatgtgaagcatgctttgctgctatgaaaatgagcatcagaaagtgtatatcatgttattttattattattatgtttttgcttttggtgtagaattcagcaatttccatcaagatctagccagagcccttcactgccatgatagctggggcttcaccagtctgcctactgtgatgatttgtagacttctggttgtatttctatatttatttttaaatatactgtgtgggatatttagtggtatatgtctctctaagtttggagtggtgtttctaaaatggagttactttgaatgttatagatggatcaaggcataaaatgtatgagatttatttttccccaaatccaaatactgatgctattgtaaacaacaaacagtgtgtatagtgcctaaaaattgtatgaaagtccttttaaccattttaatccagatgtttaacaaatctaatctcttattctaataaatatactatcaagttaaacggacaaaagatttctactttc

SEQ ID NO: 80 - protein, 371 aa, Equus caballus
MKPERTNLEALQKKLEELELDEQQRKRLEAFLTQKQKVGELKDDDFEKISELGAGNGGVVFKVAHKPSGLVMARKLIHLEIKPAIRNQIIRELQVLHECNSPYIVGFYGAFYSDGEISICMEHMDGGSLDQVLKKAGRIPEQILGKVSIAVIKGLTYLREKHKIMHRDVKPSNILVNSRGEIKLCDFGVSGQLIDSMANSFVGTRSYMSPERLQGTHYSVQSDIWSMGLSLVEMAVGRYPIPPPDAKELELMFGCQVEGDAAETPPRPRTPGRPLSSYGMDSRPPMAIFELLDYIVNEPPPKLPSGVFSLEFQDFVNKCLIKNPAERADLKQLMVHAFIKRSDAEEVDFAGWLCSTIGLNQPSTPTHAAGV

SEQ ID NO: 81 - DNA, 2274 bp, Gallus gallus
ctaaccaggcgggagctgtcggtgcggagctcggtgtcgctccgccgggcaggccgggtcgacggccgcgctgtgccggagcggcagcgtcgcgggctcggctccttctcggggaggcggccgcgcgctgctccggcgctgaggggcggccccgaagtttgcttcgcgtcgggaagtccgtcggacctggccgaagtggggccgcggccgctccgtccgtcacgctctgcgctggccggggggcaacatgcccaagaagaagccagggccgatccagctcaaccccgctccggatggctccgccgtcaacgggaccagctctgccgagacaaacttggaagctcttcagaagaagctggaagagctagagctggatgaacagcaaaggaagcgccttgaagctttccttacccagaaacaaaaagttggggagctgaaggatgatgacttcgagaagatcagtgagctgggagcagggaatggcggggtggtgttcaaagtatctcacaagccttctggcctcatcatggcaagaaaattgattcatctagaaatcaagccagctattcgaaaccagatcatccgtgagctgcaggttctacatgagtgcaattcaccatacatagtgggcttttatggagctttttacagtgatggggaaatcagcatttgcatggaacacatggatggtggctcattggatcaagtgctgaaaaaggctggaagaattccagagcagatactgggcaaagtcagcattgcagtaataaaaggactcacatatctgagagaaaagcataaaataatgcacagagatgttaaaccatctaacatcttggtaaactctagaggtgagatcaagctttgtgattttggtgtcagtggacaactgatagattctatggcaaactcatttgttggcacgcgctcctacatgtctccggaaagactgcagggaactcattattcagtgcagtcagatatatggagtatggggctgtctctggtagaaatggccattggcagatacccgattcctcctcctgactctaaggagctcgagttgatgtttggctgcccggtagagggagattctccagtcacagagacctcacccaggcaaagaacacctggtcgaccaatgagctcctatggaccagacagcagacccccgatggcaatctttgaacttctggattacatcgtcaatgagccacctccaaaactgcccaatggtgtctttggttctgaatttcaagattttgttaacaaatgtttaattaaaaatcctgctgagagagctgatttgaagcagctgatgattcacgctttcattaagagatctgaagcagaggaggtggattttgcaggatggctttgctcaaccataggccttaaccaaccgagtacacccacgcatgctgctggagtctgaatgtggaagagcaaatcctgtcccgtacatctgttaacagcgctactttggtcctatttcctaagcttgtacctgttcaaacatgtatttcacctcttaaggaagaatgtctttatagcatgtgccaaattgttttcaattttgtcatcaactaattggtattgtactgggttacatttgtttgctgaccaaaatgtaaaatgtttaagttacagtgcttgctgattttaagtgattatggaattatggatattctttcttaatgaaaatatcactgggggggaatttacccctggattgtttgaactttatcaagactctttgtaaactgttggtacttcagtcatgcttacctaatctcccatgcaaaaaaaggggtagggatgctccaaaactgtatctgttgagcatgcttttgctgctgccaaactgtatcttggaagttaggcctaatggttccaatttggtgttgtgtagagatcactctttccaggtaaagaaggtaagagctctgcattccttgggatggacagggcagtatcctacttgtagacttgttcatatttctatatttatttttaaaatgtatcatcatacttggatttagtgatatatgtctttccaattgatttttaaaggttagctctcagaagcgtcctacagaatcatgacaaagatctgggctttcttttaaccttaagattcatgacagctgtgtttggtgtctaaaatgtatgaagatcctctattgttttattctctcagatgtttagcaatggtttctcttaataaatatattatcaagtaaaaaaaaaaaaaaaataaaaaaaaaaaaaaaa

SEQ ID NO: 82 - protein, 395 aa, Gallus gallus
MPKKKPGPIQLNPAPDGSAVNGTSSAETNLEALQKKLEELELDEQQRKRLEAFLTQKQKVGELKDDDFEKISELGAGNGGVVFKVSHKPSGLIMARKLIHLEIKPAIRNQIIRELQVLHECNSPYIVGFYGAFYSDGEISICMEHMDGGSLDQVLKKAGRIPEQILGKVSIAVIKGLTYLREKHKIMHRDVKPSNILVNSRGEIKLCDFGVSGQLIDSMANSFVGTRSYMSPERLQGTHYSVQSDIWSMGLSLVEMAIGRYPIPPPDSKELELMFGCPVEGDSPVTETSPRQRTPGRPMSSYGPDSRPPMAIFELLDYIVNEPPPKLPNGVFGSEFQDFVNKCLIKNPAERADLKQLMIHAFIKRSEAEEVDFAGWLCSTIGLNQPSTPTHAAGV